European Patent Application EP 4 170 029 A2, published April 26, 2023. Title: MODIFYING THE SPECIFICITY OF PLANT NON-CODING RNA MOLECULES FOR SILENCING GENE EXPRESSION. Applicant: Tropic Biosciences UK Limited MAORI, Eyal GALANTY, Yaron PIGNOCCHI, Cristina CHAPARRO GARCIA, Angela MEIR, Ofir. The sequence listing filed with the application follows.

SEQUENCE LISTING (417 sequences)

SEQ ID NO: 1 - DNA, 23 bp, Arabidopsis thaliana
ctatccatcctgagtttcattgg

SEQ ID NO: 2 - DNA, 23 bp, Arabidopsis thaliana
aagaatctgtaaagctcaggagg

SEQ ID NO: 3 - DNA, 23 bp, Arabidopsis thaliana
cttgcagagagaaatcacagtgg

SEQ ID NO: 4 - DNA, 23 bp, Arabidopsis thaliana
gcttacacagagaatcacagagg

SEQ ID NO: 5 - DNA, 400 bp, Artificial sequence
  Oligo-1: GEiGS_mir173_si-GFP_1
gcataaaaaagtcaacaaaacttaaagcggcggtctcatcgtaatctcagcccaataccctattttcctctcccctatataaatactttcttcttctactgatcttcttctcacaaataaacccaaatatatcaatctactgtgttggtgattaagtacttaagtcgtgctgcttcatgtggagtggtcaaaaaagttgtagttttcttaaagtctctttcctctccacataagcaggacgagttaagagcttgctccctaaacttatctctctgatgatttaatgttagagatcttcgtaaatctatgtgtttgatagatctgatgcgttttttgagttgatgatttgattatttttcactggaaagtatctcattagggtaacgataatgttttatgg

SEQ ID NO: 6 - DNA, 400 bp, Artificial sequence
  Oligo-2: GEiGS_mir173_si-GFP_2
gcataaaaaagtcaacaaaacttaaagcggcggtctcatcgtaatctcagcccaataccctattttcctctcccctatataaatactttcttcttctactgatcttcttctcacaaataaacccaaatatatcaatctactgtgttggtgattaagtacttagttgtactccagcttgtgccagtggtcaaaaaagttgtagttttcttaaagtctctttcctctggcaaagctgcagtacaactaagagcttgctccctaaacttatctctctgatgatttaatgttagagatcttcgtaaatctatgtgtttgatagatctgatgcgttttttgagttgatgatttgattatttttcactggaaagtatctcattagggtaacgataatgttttatgg

SEQ ID NO: 7 - DNA, 400 bp, Artificial sequence
  Oligo-3: GEiGS_mir173_si-PDS_1
gcataaaaaagtcaacaaaacttaaagcggcggtctcatcgtaatctcagcccaataccctattttcctctcccctatataaatactttcttcttctactgatcttcttctcacaaataaacccaaatatatcaatctactgtgttggtgattaagtactttatccacacaaactacctgcaagtggtcaaaaaagttgtagttttcttaaagtctctttcctcttgcagtagttagtgtggataaagagcttgctccctaaacttatctctctgatgatttaatgttagagatcttcgtaaatctatgtgtttgatagatctgatgcgttttttgagttgatgatttgattatttttcactggaaagtatctcattagggtaacgataatgttttatgg

SEQ ID NO: 8 - DNA, 400 bp, Artificial sequence
  Oligo-4: GEiGS_mir173_si-PDS_2
gcataaaaaagtcaacaaaacttaaagcggcggtctcatcgtaatctcagcccaataccctattttcctctcccctatataaatactttcttcttctactgatcttcttctcacaaataaacccaaatatatcaatctactgtgttggtgattaagtactttgacaatccagccaatccagcagtggtcaaaaaagttgtagttttcttaaagtctctttcctctgctgattggcaggattgtcaaagagcttgctccctaaacttatctctctgatgatttaatgttagagatcttcgtaaatctatgtgtttgatagatctgatgcgttttttgagttgatgatttgattatttttcactggaaagtatctcattagggtaacgataatgttttatgg

SEQ ID NO: 9 - DNA, 400 bp, Artificial sequence
  Oligo-5: GEiGS_mir390a_si-GFP_1
agaggagatgacgtgtgttccttcgaacccgagttttgttcgtctataaatagcaccttctcttctccttcttcctcacttccatctttttagcttcactatctctctataatcggttttatctttctctaagtcacaacccaaaaaaacaaagtagagaagaatctgtaaagtcgtgctgcttcatgtggatgatgatcacattcgttatctattttttccacatgaagaagcacgacttgattggctcttcttactacaatgaaaaaggccgaggcaaaacgcctaaaatcacttgagaatcaattctttttactgtccatttaagctatcttttataaacgtgtcttattttctatctcttttgtttaaactaagaaactatagtattttgtctaaa

SEQ ID NO: 10 - DNA, 400 bp, Artificial sequence
  Oligo-6: GEiGS_mir390a_si-GFP_2
agaggagatgacgtgtgttccttcgaacccgagttttgttcgtctataaatagcaccttctcttctccttcttcctcacttccatctttttagcttcactatctctctataatcggttttatctttctctaagtcacaacccaaaaaaacaaagtagagaagaatctgtaagttgtactccagcttgtgccatgatgatcacattcgttatctattttttggcacaagcttgagtacaactgattggctcttcttactacaatgaaaaaggccgaggcaaaacgcctaaaatcacttgagaatcaattctttttactgtccatttaagctatcttttataaacgtgtcttattttctatctcttttgtttaaactaagaaactatagtattttgtctaaa

SEQ ID NO: 11 - DNA, 400 bp, Artificial sequence
  Oligo-7: GEiGS_mir390a_si-PDS_1
agaggagatgacgtgtgttccttcgaacccgagttttgttcgtctataaatagcaccttctcttctccttcttcctcacttccatctttttagcttcactatctctctataatcggttttatctttctctaagtcacaacccaaaaaaacaaagtagagaagaatctgtatatccacacaaactacctgcaatgatgatcacattcgttatctatttttttgcaggtagtgtgtgtggatagattggctcttcttactacaatgaaaaaggccgaggcaaaacgcctaaaatcacttgagaatcaattctttttactgtccatttaagctatcttttataaacgtgtcttattttctatctcttttgtttaaactaagaaactatagtattttgtctaaa

SEQ ID NO: 12 - DNA, 400 bp, Artificial sequence
  Oligo-8: GEiGS_mir390a_si-PDS_2
agaggagatgacgtgtgttccttcgaacccgagttttgttcgtctataaatagcaccttctcttctccttcttcctcacttccatctttttagcttcactatctctctataatcggttttatctttctctaagtcacaacccaaaaaaacaaagtagagaagaatctgtatgacaatccagccaatccagcatgatgatcacattcgttatctattttttgctggattggatggattgtcagattggctcttcttactacaatgaaaaaggccgaggcaaaacgcctaaaatcacttgagaatcaattctttttactgtccatttaagctatcttttataaacgtgtcttattttctatctcttttgtttaaactaagaaactatagtattttgtctaaa

SEQ ID NO: 13 - DNA, 1005 bp, Artificial sequence
  CaMV-35S-promoter nucleic acid sequence
tttggagaggacaggcttcttgagatccttcaacaattaccaacaacaacaaacaacaaacaacattacaattactatttacaattacagtcgactctagaggatccatggtgagcaagggcgaggagctgttcaccggggtggtgcccatcctggtcgagctggacggcgacgtaaacggccacaagttcagcgtgagaggcgagggcgagggcgatgccaccaacggcaagctgaccctgaagttcatctgcaccaccggcaagctgcccgtgccctggcccaccctcgtgaccaccctgacctacggcgtgcagtgcttcagccgctaccccgaccacatgaagcagcacgacttcttcaagtccgccatgcccgaaggctacgtccaggagcgcaccatctctttcaaggacgacggcacttacaagacccgcgccgaggtgaagttcgagggcgacaccctggtgaaccgcatcgagctgaagggcatcgacttcaaggaggacggcaacatcctggggcacaagctggagtacaacttcaacagccacaacgtctatatcactgccgacaagcagaagaacggcatcaaggccaacttcaagatccgccacaacgttgaggacggcagcgtgcagctcgccgaccactaccagcagaacacccccatcggcgacggccccgtgctgctgcccgacaaccactacctgagcacccagtccgttctgagcaaagaccccaacgagaagcgcgatcacatggtcctgctggagttcgtgaccgccgccgggatcactctcggcatggacgagctgtacaagtaaagcggccgcccggctgcagatcgttcaaacatttggcaataaagtttcttaagattgaatcctgttgccggtcttgcgatgattatcatataatttctgttgaattacgttaagcatgtaataattaacatgtaatgcatgacgttatttatgagatgggtttttatgattagagtcc

SEQ ID NO: 14 - DNA, 855 bp, Artificial sequence
  NOS terminator nucleic acid sequence
gctcgtccatgccgagagtgatcccggcggcggtcacgaactccagcaggaccatgtgatcgcgcttctcgttggggtctttgctcagaacggactgggtgctcaggtagtggttgtcgggcagcagcacggggccgtcgccgatgggggtgttctgctggtagtggtcggcgagctgcacgctgccgtcctcaacgttgtggcggatcttgaagttggccttgatgccgttcttctgcttgtcggcagtgatatagacgttgtggctgttgaagttgtactccagcttgtgccccaggatgttgccgtcctccttgaagtcgatgcccttcagctcgatgcggttcaccagggtgtcgccctcgaacttcacctcggcgcgggtcttgtaagtgccgtcgtccttgaaagagatggtgcgctcctggacgtagccttcgggcatggcggacttgaagaagtcgtgctgcttcatgtggtcggggtagcggctgaagcactgcacgccgtaggtcagggtggtcacgagggtgggccagggcacgggcagcttgccggtggtgcagatgaacttcagggtcagcttgccgttggtggcatcgccctcgccctcgcctctcacgctgaacttgtggccgtttacgtcgccgtccagctcgaccaggatgggcaccaccccggtgaacagctcctcgcccttgctcaccatggatcctctagagtcgactgtaattgtaaatagtaattgtaatgttgtttgttgtttgttgttgttggtaattgttgaaggatctcaagaagcctgtcctctccaaatgaaatgaacttccttatatagaggaagggtcttgcgaa

SEQ ID NO: 15 - DNA, 215 bp, Artificial sequence
  CaMV-35S terminator nucleic acid sequence
cgctctgtcatcgttacaatcaacatgctaccctccgcgagatcatccgtgtttcaaacccggcagcttagttgccgttcttccgaatagcatcggtaacatgagcaaagtctgccgccttacaacggctctcccgctgacgccgtcccggactgatgggctgcctgtatcgagtggtgattttgtgccgagctgccggtcggggagctgttggc

SEQ ID NO: 16 - DNA, 216 bp, Artificial sequence
  G7-ter nucleic acid sequence
gatcccccgtcgacagctagctatatcatcaatttatgtattacacataatatcgcactcagtctttcatctacggcaatgtaccagctgatataatcagttattgaaatatttctgaatttaaacttgcatcaataaatttatgtttttgcttggactataatacctgacttgttattttatcaataaatatttaaactatatttctttcaagat

SEQ ID NO: 17 - DNA, 516 bp, Artificial sequence
  CsVMV promoter nucleic acid sequence
ccagaaggtaattatccaagatgtagcatcaagaatccaatgtttacgggaaaaactatggaagtattatgtaagctcagcaagaagcagatcaatatgcggcacatatgcaacctatgttcaaaaatgaagaatgtacagatacaagatcctatactgccagaatacgaagaagaatacgtagaaattgaaaaagaagaaccaggcgaagaaaagaatcttgatgacgtaagcactgacgacaacaatgaaaagaagaagataaggtcggtgattgtgaaagagacatagaggacacatgtaaggtggaaaatgtaagggcggaaagtaaccttatcacaaaggaatcttatcccccactacttatccttttatatttttccgtgtcatttttgcccttgagttttcctatataaggaaccaagttcggcatttgtgaaaacaagaaaaaatttggtgtaagctattttctttgaagtactgaggatacaacttcagagaaatttgtaagtttgt

SEQ ID NO: 18 - DNA, 636 bp, Arabidopsis thaliana
gtcgacgagtcagtaataaacggcgtcaaagtggttgcagccggcacacacgagtcgtgtttatcaactcaaagcacaaatacttttcctcaacctaaaaataaggcaattagccaaaaacaactttgcgtgtaaacaacgctcaatacacgtgtcattttattattagctattgcttcaccgccttagctttctcgtgacctagtcgtcctcgtcttttcttcttcttcttctataaaacaatacccaaagagctcttcttcttcacaattcagatttcaatttctcaaaatcttaaaaactttctctcaattctctctaccgtgatcaaggtaaatttctgtgttccttattctctcaaaatcttcgattttgttttcgttcgatcccaatttcgtatatgttctttggtttagattctgttaatcttagatcgaagacgattttctgggtttgatcgttagatatcatcttaattctcgattagggtttcatagatatcatccgatttgttcaaataatttgagttttgtcgaataattactcttcgatttgtgatttctatctagatctggtgttagtttctagtttgtgcgatcgaatttgtagattaatctgagtttttctgattaacag

SEQ ID NO: 19 - DNA, 4140 bp, Artificial sequence
  pco_Cas9_NLS  nucleic acid sequence
atggataagaagtactctatcggactcgatatcggaactaactctgtgggatgggctgtgatcaccgatgagtacaaggtgccatctaagaagttcaaggttctcggaaacaccgataggcactctatcaagaaaaaccttatcggtgctctcctcttcgattctggtgaaactgctgaggctaccagactcaagagaaccgctagaagaaggtacaccagaagaaagaacaggatctgctacctccaagagatcttctctaacgagatggctaaagtggatgattcattcttccacaggctcgaagagtcattcctcgtggaagaagataagaagcacgagaggcaccctatcttcggaaacatcgttgatgaggtggcataccacgagaagtaccctactatctaccacctcagaaagaagctcgttgattctactgataaggctgatctcaggctcatctacctcgctctcgctcacatgatcaagttcagaggacacttcctcatcgagggtgatctcaaccctgataactctgatgtggataagttgttcatccagctcgtgcagacctacaaccagcttttcgaagagaaccctatcaacgcttcaggtgtggatgctaaggctatcctctctgctaggctctctaagtcaagaaggcttgagaacctcattgctcagctccctggtgagaagaagaacggacttttcggaaacttgatcgctctctctctcggactcacccctaacttcaagtctaacttcgatctcgctgaggatgcaaagctccagctctcaaaggatacctacgatgatgatctcgataacctcctcgctcagatcggagatcagtacgctgatttgttcctcgctgctaagaacctctctgatgctatcctcctcagtgatatcctcagagtgaacaccgagatcaccaaggctccactctcagcttctatgatcaagagatacgatgagcaccaccaggatctcacacttctcaaggctcttgttagacagcagctcccagagaagtacaaagagattttcttcgatcagtctaagaacggatacgctggttacatcgatggtggtgcatctcaagaagagttctacaagttcatcaagcctatcctcgagaagatggatggaaccgaggaactcctcgtgaagctcaatagagaggatcttctcagaaagcagaggaccttcgataacggatctatccctcatcagatccacctcggagagttgcacgctatccttagaaggcaagaggatttctacccattcctcaaggataacagggaaaagattgagaagattctcaccttcagaatcccttactacgtgggacctctcgctagaggaaactcaagattcgcttggatgaccagaaagtctgaggaaaccatcaccccttggaacttcgaagaggtggtggataagggtgctagtgctcagtctttcatcgagaggatgaccaacttcgataagaaccttccaaacgagaaggtgctccctaagcactctttgctctacgagtacttcaccgtgtacaacgagttgaccaaggttaagtacgtgaccgagggaatgaggaagcctgcttttttgtcaggtgagcaaaagaaggctatcgttgatctcttgttcaagaccaacagaaaggtgaccgtgaagcagctcaaagaggattacttcaagaaaatcgagtgcttcgattcagttgagatttctggtgttgaggataggttcaacgcatctctcggaacctaccacgatctcctcaagatcattaaggataaggatttcttggataacgaggaaaacgaggatatcttggaggatatcgttcttaccctcaccctctttgaagatagagagatgattgaagaaaggctcaagacctacgctcatctcttcgatgataaggtgatgaagcagttgaagagaagaagatacactggttggggaaggctctcaagaaagctcattaacggaatcagggataagcagtctggaaagacaatccttgatttcctcaagtctgatggattcgctaacagaaacttcatgcagctcatccacgatgattctctcacctttaaagaggatatccagaaggctcaggtttcaggacagggtgatagtctccatgagcatatcgctaacctcgctggatctcctgcaatcaagaagggaatcctccagactgtgaaggttgtggatgagttggtgaaggtgatgggaaggcataagcctgagaacatcgtgatcgaaatggctagagagaaccagaccactcagaagggacagaagaactctagggaaaggatgaagaggatcgaggaaggtatcaaagagcttggatctcagatcctcaaagagcaccctgttgagaacactcagctccagaatgagaagctctacctctactacctccagaacggaagggatatgtatgtggatcaagagttggatatcaacaggctctctgattacgatgttgatcatatcgtgccacagtcattcttgaaggatgattctatcgataacaaggtgctcaccaggtctgataagaacaggggtaagagtgataacgtgccaagtgaagaggttgtgaagaaaatgaagaactattggaggcagctcctcaacgctaagctcatcactcagagaaagttcgataacttgactaaggctgagaggggaggactctctgaattggataaggcaggattcatcaagaggcagcttgtggaaaccaggcagatcactaagcacgttgcacagatcctcgattctaggatgaacaccaagtacgatgagaacgataagttgatcagggaagtgaaggttatcaccctcaagtcaaagctcgtgtctgatttcagaaaggatttccaattctacaaggtgagggaaatcaacaactaccaccacgctcacgatgcttaccttaacgctgttgttggaaccgctctcatcaagaagtatcctaagctcgagtcagagttcgtgtacggtgattacaaggtgtacgatgtgaggaagatgatcgctaagtctgagcaagagatcggaaaggctaccgctaagtatttcttctactctaacatcatgaatttcttcaagaccgagattaccctcgctaacggtgagatcagaaagaggccactcatcgagacaaacggtgaaacaggtgagatcgtgtgggataagggaagggatttcgctaccgttagaaaggtgctctctatgccacaggtgaacatcgttaagaaaaccgaggtgcagaccggtggattctctaaagagtctatcctccctaagaggaactctgataagctcattgctaggaagaaggattgggaccctaagaaatacggtggtttcgattctcctaccgtggcttactctgttctcgttgtggctaaggttgagaagggaaagagtaagaagctcaagtctgttaaggaacttctcggaatcactatcatggaaaggtcatctttcgagaagaacccaatcgatttcctcgaggctaagggatacaaagaggttaagaaggatctcatcatcaagctcccaaagtactcactcttcgaactcgagaacggtagaaagaggatgctcgcttctgctggtgagcttcaaaagggaaacgagcttgctctcccatctaagtacgttaactttctttacctcgcttctcactacgagaagttgaagggatctccagaagataacgagcagaagcaacttttcgttgagcagcacaagcactacttggatgagatcatcgagcagatctctgagttctctaaaagggtgatcctcgctgatgcaaacctcgataaggtgttgtctgcttacaacaagcacagagataagcctatcagggaacaggcagagaacatcatccatctcttcacccttaccaacctcggtgctcctgctgctttcaagtacttcgatacaaccatcgataggaagagatacacctctaccaaagaagtgctcgatgctaccctcatccatcagtctatcactggactctacgagactaggatcgatctctcacagctcggtggtgattcaagggctgatcctaagaagaagaggaaggtttga

SEQ ID NO: 20 - DNA, 263 bp, Artificial sequence
  AtuNos ter nucleic acid sequence
gtcaagcagatcgttcaaacatttggcaataaagtttcttaagattgaatcctgttgccggtcttgcgatgattatcatataatttctgttgaattacgttaagcatgtaataattaacatgtaatgcatgacgttatttatgagatgggtttttatgattagagtcccgcaattatacatttaatacgcgatagaaaacaaaatatagcgcgcaaactaggataaattatcgcgcgcggtgtcatctatgttactagatcga

SEQ ID NO: 21 - DNA, 1147 bp, Artificial sequence
  Synthetic construct clone eGFP-OsP5SM_E/R eGFP (eGFP) gene
atgtctagagtgagcaagggcgaggagctgttcaccggggtggtgcccatcctggtcgagctggacggcgacgtaaacggccacaagttcagcgtgtccggcgagggcgagggcgatgccacctacggcaagctgaccctgaagttcatctgcaccaccggcaagctgcccgtgccctggcccaccctcgtgaccaccctgacctacggcgtgcagtgcttcagccgctaccccgaccacatgaagcagcacgacttcttcaagtccgccatgcccgaaggctacgtccaggaggtagatttatgcatcctcttgtcatgagaagtcgaattgttcccattctgtgtgttgcagctacagatggagatacatagagatactcgtggattttgcttagtgttgagttttgttctggttgtgaactaaaagtttatacatttgcaggaaataaatagccttttgtttaaatcaaaaggtcttacctatgttagtgtgaagcattggatcccaaagaactccaaaatgcgatgaggcatatttaatcttgtctggactagtaacaggttgggatgaccacctgtgaagctccaacaggattgcctcctcacgcaatgtttgaggtctgatgttcaatagcttgttttgtttcactttgctttggactttcttttcgccaatgagctatgtttctgatggttttcactcttttggtgtgtagagaaccatcttcttcaaggacgacggcaactacaagacccgcgccgaggtgaagttcgagggcgacaccctggtgaaccgcatcgagctgaagggcatcgacttcaaggaggacggcaacacctggggcacaagctggagtacaactacaacagccacaacgtctatatcatggccgacaagcagaagaaggcatcaaggtgaacttcaagatccgccacaacatcgaggacggcagcgtgcagctcgccgaccactacagcagaacacccccatcggcgacggccccgtgctgctgcccgacaaccactacctgagcacccagtccgccctgagcaaagaccccaacgagaagcgcgatcacatggtcctgctggagttcgtgaccgccgccgggatcactctcggcatggacgagctgtacaagtaa

SEQ ID NO: 22 - DNA, 2074 bp, Arabidopsis thaliana
caattatgtgttaaagatacaaacttttgtctgatttgcttccaccggtttcacctaagatactcaattttcttactttttgtgtgttttgtaattctaattcttttatagcttcaatttttagattcattgaagcagttgtgagttaagttggagaaaatggttgtgtttgggaatgtttctgcggcgaatttgccttatcaaaacgggtttttggaggcactttcatctggaggttgtgaactaatgggacatagctttagggttcccacttctcaagcgcttaagacaagaacaaggaggaggagtactgctggtcctttgcaggtagtttgtgtggatattccaaggccagagctagagaacactgtcaatttcttggaagctgctagtttatctgcatccttccgtagtgctcctcgtcctgctaagcctttgaaagttgtaattgctggtgctggattggctggattgtcaactgcaaagtacctggctgatgcaggccacaaacctctgttgcttgaagcaagagatgttcttggtggaaagatagctgcatggaaggatgaagatggggactggtatgagactggtttacatattttcttcggtgcttatccgaatgtgcagaatttatttggagaacttgggatcaatgatcggttgcagtggaaggaacactccatgatttttgctatgccaagtaaacctggagaatttagtagatttgacttcccagatgtcctaccagcacccttaaatggtatttgggctattttgcggaacaacgagatgctgacatggccagagaaaataaagtttgctattggacttttgccagccatggtcggcggtcaggcttatgttgaggcccaagatggtttatcagtcaaagaatggatggaaaagcagggagtacctgagcgcgtgaccgacgaggtgtttattgccatgtcaaaggcgctaaactttataaaccctgatgaactgtcaatgcaatgcattttgatagctttgaaccggtttcttcaggaaaaacatggttccaagatggcattcttggatggtaatcctccggaaaggctttgtatgccagtagtggatcatattcgatcactaggtggggaagtgcaacttaattctaggataaagaaaattgagctcaatgacgatggcacggttaagagtttcttactcactaatggaagcactgtcgaaggagacgcttatgtgtttgccgctccagtcgatatcctgaagctccttttaccagatccctggaaagaaataccgtacttcaagaaattggataaattagttggagtaccagttattaatgttcatatatggtttgatcgaaaactgaagaacacatatgatcacctactctttagcagaagtaaccttctgagcgtgtatgccgacatgtccttaacttgtaaggaatattacgatcctaaccggtcaatgctggagctagtatttgcaccagcagaggaatggatatcacggactgattctgacatcatagatgcaacaatgaaagaacttgagaaactcttccctgatgaaatctcagctgaccaaagcaaagctaaaattctgaagtaccatgtcgttaagactccaagatctgtgtacaagaccatcccaaactgtgaaccatgtcgtcctctacaaagatcacctattgaaggattctacttagctggagattacacaaaacagaagtacttagcttccatggaaggcgctgtcctctctggcaaattctgctctcagtctattgttcaggattacgagctactggctgcgtctggaccaagaaagttgtcggaggcaacagtatcatcatcatgagaagaggacaaaacttaaagatgatttgcttgtaagcattattatttgtgtataaatctcattgcaatccaaacttaaccttactctcttcagtaaatgaatctcacagatttgacatctcacgtttctgtcaattttataatttttaaaaagtaattactgtcgaccttttgtaatcatagtgatttatcattatgtctctctttttaaaacc

SEQ ID NO: 23 - DNA, 1419 bp, Arabidopsis thaliana
ggagcatcttcattcttaagatatgaagataatcttcaaaaggcccctgggaatctgaaagaagagaagcaggcccatttatatgggaaagaacaatagtatttcttatataggcccatttaagttgaaaacaatcttcaaaagtcccacatcgcttagataagaaaacgaagctgagtttatatacagctagagtcgaagtagtgattgtgagacggatatcaatacgcaaaccgcctctccccgcgcgttggccgattcattaatgcagctggcacgacaggtttcccgactggaaagcgggcagtgagcgcaacgcaattaatgtgagttagctcactcattaggcaccccaggctttacactttatgcttccggctcgtatgttgtgtggaattgtgagcggataacaatttcacacatactagagaaagaggagaaatactagatggcttcctccgaggacgttatcaaagagttcatgcgtttcaaagttcgtatggaaggttccgttaacggtcacgagttcgaaatcgaaggtgaaggtgaaggtcgtccgtacgaaggtacccagaccgctaaactgaaagttaccaaaggtggtccgctgccgttcgcttgggacatcctgtccccgcagttccagtacggttccaaagcttacgttaaacacccggctgacatcccggactacctgaaactgtccttcccggaaggtttcaaatgggaacgtgttatgaacttcgaggacggtggtgttgttaccgttacccaggactcctccctgcaagacggtgagttcatctacaaagttaaactgcgtggtaccaacttcccgtccgacggtccggttatgcagaaaaaaaccatgggttgggaagcttccaccgaacgtatgtacccggaggacggtgctctgaaaggtgaaatcaaaatgcgtctgaaactgaaagacggtggtcactacgacgctgaagttaaaaccacctacatggctaaaaaaccggttcagctgccgggtgcttacaaaaccgacatcaaactggacatcacctcccacaacgaggactacaccatcgttgaacagtacgaacgtgctgaaggtcgtcactccaccggtgcttaataacgctgatagtgctagtgtagatcgctactagagccaggcatcaaataaaacgaaaggctcagtcgaaagactgggcctttcgttttatctgttgtttgtcggtgaacgctctctactagagtcacactggctcaccttcgggtgggcctttctgcgtttatacgtctcagttttagagctagaaatagcaagttaaaataaggctagtccgttatcaacttgaaaaagtggcaccgagtcggtgctttttttctagacccagctttcttgtacaaagttggcattacgct

SEQ ID NO: 24 - DNA, 1286 bp, Artificial sequence
  U6III-synthetic pol 3 promoter for sgRNA expression
ggagtatgatcaaaagtcccacatcgatcaggtgatatatagcagcttagtttatataatgatagagtcgacatagcgattgggagacgcaatacgcaaaccgcctctccccgcgcgttggccgattcattaatgcagctggcacgacaggtttcccgactggaaagcgggcagtgagcgcaacgcaattaatgtgagttagctcactcattaggcaccccaggctttacactttatgcttccggctcgtatgttgtgtggaattgtgagcggataacaatttcacacatactagagaaagaggagaaatactagatggcttcctccgaggacgttatcaaagagttcatgcgtttcaaagttcgtatggaaggttccgttaacggtcacgagttcgaaatcgaaggtgaaggtgaaggtcgtccgtacgaaggtacccagaccgctaaactgaaagttaccaaaggtggtccgctgccgttcgcttgggacatcctgtccccgcagttccagtacggttccaaagcttacgttaaacacccggctgacatcccggactacctgaaactgtccttcccggaaggtttcaaatgggaacgtgttatgaacttcgaggacggtggtgttgttaccgttacccaggactcctccctgcaagacggtgagttcatctacaaagttaaactgcgtggtaccaacttcccgtccgacggtccggttatgcagaaaaaaaccatgggttgggaagcttccaccgaacgtatgtacccggaggacggtgctctgaaaggtgaaatcaaaatgcgtctgaaactgaaagacggtggtcactacgacgctgaagttaaaaccacctacatggctaaaaaaccggttcagctgccgggtgcttacaaaaccgacatcaaactggacatcacctcccacaacgaggactacaccatcgttgaacagtacgaacgtgctgaaggtcgtcactccaccggtgcttaataacgctgatagtgctagtgtagatcgctactagagccaggcatcaaataaaacgaaaggctcagtcgaaagactgggcctttcgttttatctgttgtttgtcggtgaacgctctctactagagtcacactggctcaccttcgggtgggcctttctgcgtttatacgtctccgttttagagctagaaatagcaagttaaaataaggctagtccgttatcaacttgaaaaagtggcaccgagtcggtgctttttttctagacccagctttcttgtacaaagttggcattacgct

SEQ ID NO: 25 - DNA, 2074 bp, Arabidopsis thaliana; identical to SEQ ID NO: 22

SEQ ID NO: 26 - DNA, 2290 bp, Arabidopsis thaliana
ctttggtgggcaaaaacatattagctgagaggtcaatttctttttcccctaaaccaaattacgttgagatgcatggtctctctctactcaattaaccaaataaggaaaagaatcatatggtcatcaattcgtaaatcaaaattttaatttgtgtggtatttaatccatctacatgtttcgtaagcaacaaaagagcttggtctgaaaaccaaacaagaccatatgggcactcgaatactccattttgttatcggctacttccactagcctcctccttcgctgcgtctcctgtttctctacttcacgattactcgctagattcattgaagcagttgtgagttaagttggagaaaatggttgtgtttgggaatgtttctgcggcgaatttgccttatcaaaacgggtttttggaggcactttcatctggaggttgtgaactaatgggacatagctttagggttcccacttctcaagcgcttaagacaagaacaaggaggaggagtactgctggtcctttgcaggtagtttgtgtggatattccaaggccagagctagagaacactgtcaatttcttggaagctgctagtttatctgcatccttccgtagtgctcctcgtcctgctaagcctttgaaagttgtaattgctggtgctggattggctggattgtcaactgcaaagtacctggctgatgcaggccacaaacctctgttgcttgaagcaagagatgttcttggtggaaagatagctgcatggaaggatgaagatggggactggtatgagactggtttacatattttcttcggtgcttatccgaatgtgcagaatttatttggagaacttgggatcaatgatcggttgcagtggaaggaacactccatgatttttgctatgccaagtaaacctggagaatttagtagatttgacttcccagatgtcctaccagcacccttaaatggtatttgggctattttgcggaacaacgagatgctgacatggccagagaaaataaagtttgctattggacttttgccagccatggtcggcggtcaggcttatgttgaggcccaagatggtttatcagtcaaagaatggatggaaaagcagggagtacctgagcgcgtgaccgacgaggtgtttattgccatgtcaaaggcgctaaactttataaaccctgatgaactgtcaatgcaatgcattttgatagctttgaaccggtttcttcaggaaaaacatggttccaagatggcattcttggatggtaatcctccggaaaggctttgtatgccagtagtggatcatattcgatcactaggtggggaagtgcaacttaattctaggataaagaaaattgagctcaatgacgatggcacggttaagagtttcttactcactaatggaagcactgtcgaaggagacgcttatgtgtttgccgctccagtcgatatcctgaagctccttttaccagatccctggaaagaaataccgtacttcaagaaattggataaattagttggagtaccagttattaatgttcatatatggtttgatcgaaaactgaagaacacatatgatcacctactctttagcagaagtaaccttctgagcgtgtatgccgacatgtccttaacttgtaaggaatattacgatcctaaccggtcaatgctggagctagtatttgcaccagcagaggaatggatatcacggactgattctgacatcatagatgcaacaatgaaagaacttgagaaactcttccctgatgaaatctcagctgaccaaagcaaagctaaaattctgaagtaccatgtcgttaagactccaagatctgtgtacaagaccatcccaaactgtgaaccatgtcgtcctctacaaagatcacctattgaaggattctacttagctggagattacacaaaacagaagtacttagcttccatggaaggcgctgtcctctctggcaaattctgctctcagtctattgttcaggattacgagctactggctgcgtctggaccaagaaagttgtcggaggcaacagtatcatcatcatgagaagaggacaaaacttaaagatgatttgcttgtaagcattattatttgtgtataaatctcattgcaatccaaacttaaccttactctcttcagtaaatgaatctcacagatttgacatctcacgtttctgtcaattttataatttttaaaaagtaattactgtcgaccttttgtaatcatagtgatttatcattatgtctctctttttaaaaccttttctggtacaaattataaaa

SEQ ID NO: 27 - protein, 241 aa, Artificial sequence
  eGFP [synthetic construct] amino acid sequence
MSRVSKGEELFTGVVPILVELDGDVNGHKFSVSGEGEGDATYGKLTLKFICTTGKLPVPWPTLVTTLTYGVQCFSRYPDHMKQHDFFKSAMPEGYVQERTIFFKDDGNYKTRAEVKFEGDTLVNRIELKGIDFKEDGNILGHKLEYNYNSHNVYIMADKQKNGIKVNFKIRHNIEDGSVQLADHYQQNTPIGDGPVLLPDNHYLSTQSALSKDPNEKRDHMVLLEFVTAAGITLGMDELYK

SEQ ID NO: 28 - DNA, 107 bp, Arabidopsis thaliana
guagagaagaaucuguaaagcucaggagggauagcgccaugaugaucacauucguuaucuauuuuuuggcgcuauccauccugaguuucauuggcucuucuuacuac

SEQ ID NO: 29 - DNA, 102 bp, Arabidopsis thaliana
uaaguacuuucgcuugcagagagaaaucacaguggucaaaaaaguuguaguuuucuuaaagucucuuuccucugugauucucuguguaagcgaaagagcuug

SEQ ID NO: 30 - DNA, 711 bp, Artificial Sequence
  nucleic acid sequence encoding mCherry
atggtgagcaagggcgaggaggataacatggccatcatcaaggagttcatgcgcttcaaggtgcacatggagggctccgtgaacggccacgagttcgagatcgagggcgagggcgagggccgcccctacgagggcacccagaccgccaagctgaaggtgaccaagggtggccccctgcccttcgcctgggacatcctgtcccctcagttcatgtacggctccaaggcctacgtgaagcaccccgccgacatccccgactacttgaagctgtccttccccgagggcttcaagtgggagcgcgtgatgaacttcgaggacggcggcgtggtgaccgtgacccaggactcctccctgcaggacggcgagttcatctacaaggtgaagctgcgcggcaccaacttcccctccgacggcccagtaatgcagaagaaaaccatgggctgggaggcctcctccgagcggatgtaccccgaggacggcgccctgaagggcgagatcaagcagaggctgaagctgaaggacggcggccactacgacgctgaggtcaagaccacctacaaggccaagaagcccgtgcagctgcccggcgcctacaacgtcaacatcaagttggacatcacctcccacaacgaggactacaccatcgtggaacagtacgaacgcgccgagggccgccactccaccggcggcatggacgagctgtacaagtga

SEQ ID NO: 31 - DNA, 4100 bp, Artificial Sequence
  Plasmid-1: GEiGS_ mir173_si-GFP_1
cacttatcatttagacagtagattttaaatttgtatttacaatttcaaaactgaaattcatttgtaatcaaagaaaaacaaaacaagaaaagggaggaggagtgggatttgggttgcttaacagtattatatatacacgtcgttagttaatcaataaattatgagcaggtgtagtagctatgaacatggttttaccaaattggtaaattcatgtcattgttgtagcactttagcgaggccagcaaaatggcgttcttggaaagggcatggcggcccgtggccgccagggatatgtgtgcagctagaaggattagaaggagtaacttcacctttttgtagaaactgtaaattgccaagacgctcgtttggtaaataccttaacgcttcgtttgctggaatgtgtaccaccattagtagaagaaagtataataagactattaatgcaagagattttttcatattccttttctaagagtagaatggaatgaataaatgaatgaatgaaatagggtttttcttgtttagatcctgtcgcacccgagaataatagaagctgaattaattggtgaagagttttatggtggcgatgttgtatttatagagggaaatgatttcaagtttacaatgggatttttaatttgttttgttgactattatcttgcggagagatcttgactgttgacatgtatgtagtgtttgttattaaaataaatgcatttttgtagacccgattcttaaatatgttaggcatggtcaaattgttagactgtaaaagcttgagtagagacatcggtcaactttgtttacaagaattctctataaaatattatacaaattgatcggtagaaattagatggaacattttgaattaatgtttgacaatgtataaattggtttggtcaatatctaggaatgaaaacaagagctgcttcaaagttgttccattcttaagtatacatagaggtggcttgatgggaagtttcatggaagtgtagttttatatctacttccaaattcgttgatctgtttcttatctcaagctaaacatgtttagaaaagatgtgttaaaaacatgtgacaaaaaaagagtcaaatgtttggcaaacaaggtacttagatttttggcatctattcaaatataatagaatcccaaaattatgatatttgtcaatcaaatttgaaaaaaaaaaaaaaaaaaaaaaagattctacaaaagatcaaacgtattgccgtagatttatcataattttaattctttcacactaccactagtccactaccatatagtgatgagataatccataatcataaataagatataactttcgaattcttgtttttgttgcctcaaagttgttggatcattattttttacgtaaatgtggcttaatgagaatttatgtttgtgggaattgtagtttgcttccaactttttttttttttttttgaacacgtagtttgcttccaacttagtttatctttttcttatttcaagttaaacatgtaaaaaaacatgtgacgacgaaattcaatcagttcctccaatgtttggcagaagccaaatctttggtaaacaaagtaatttttttgccatttgattggttagtataggagaatttaaaaacgacgataaggtttaggtaaattatttcatttgaaaataattgagcaccgttaataattttcatccataaaataatatttcaaagatgatatttgatccccattaaattcattcgtaaccaaaaaaaagttatgaaaaaagagtggtcgtgtgagttgcccaagcaccattataataaaaaataaaataattagcaagtaataaggaataaaatcctgtaattatagctgaaaaaggaaaaatatttggagaccgtcagattcgaatctgaacaaagcataaaaaagtcaacaaaacttaaagcggcggtctcatcgtaatctcagcccaataccctattttcctctcccctatataaatactttcttcttctactgatcttcttctcacaaataaacccaaatatatcaatctactgtgttggtgattaagtacttaagtcgtgctgcttcatgtggagtggtcaaaaaagttgtagttttcttaaagtctctttcctctccacataagcaggacgagttaagagcttgctccctaaacttatctctctgatgatttaatgttagagatcttcgtaaatctatgtgtttgatagatctgatgcgttttttgagttgatgatttgattatttttcactggaaagtatctcattagggtaacgataatgttttatggatttggttgtataacagatccatgaaatcttgactggttataaaatctgaataatgtatttcaatttggagattcggtgataaaaattactgatttacgaatgacatttatatcgatagatgagtttgctgatttggttgttaaattgataaatcaaggacatgagaaactgtttttgtatgctaatttgtccatggaataaaattgggaggtgaggaccgtgagggtagtcaggaaaccttaatattgaagttgatgttgaaccaacaaatctgcccaaaaatgataaaagttgatgccgagcccacaaattttgatgacaatcgataagcccaagcccaaaaggcatctgtacctgagcccattattctttcattactagcaaaaaggatgcattagagaccccggtgtagtaaattgacctcacaattcactattgtattgtatacgtacatttcaagcgtaattaaaccctcatatttttatacgctttaaatataattggcctttaattagctcaaataaactagatgtcgtacgtgatcacggtggatgaaatcaatggtattatgaaaagactgtacatgatttcaaatattttaatgtggtcgtaaaaattgttgtttatagtggaaattgaagacaacaacgttactgaaacacatacagattgaaatttcgatcatttacttgcaaagtgttaccgtggaggcgtggcgtggacgtaaggtaccataatggtttgtgttacagtcacgccactacactcgaattcaagctaccatattataatacgttgttgattagaaaaaatagtcgccaattttctttaaaacaaatttcagtttttatttgtcagcaaaaaaaacttactaacacaacggaagaacacaaaaattagggagttgctcacagagcaaaagtaatagaaatgggaaaagctaatatacgtccgagtaggaaactaatcttgcaaaaactgatgaaagcaatcagaagccttgacgtttgtctggagagaggaattgtgttttggatcactttgttcagtttgttgtggatcgtcttccgttacgttctcaccaaaaatatttcataatgaaacaaaaaaattaattaataatggtagcttagaatgccaagttgagaacagatttgcagtttgtcccggaatgatcaagtagagcattcatagtgtcttgccaatatggtgtgatcaacgaagtttgacaaaaccgtgaagatataggaacatgtaatcatgcggctctccatacaatacatcttgttgacaaagttcccaagacctcattctacaaaccaatgtttcttttttctttttctttttggtgatagtttttgcaatcaaatgttgtaaaactatgattggaaatactactgtattttaccgaaaactttattatatatagtcattaacactcattaccaatcacataatcaatagtctattttgattatacaacttttaaacaataaagacatgtttatacagatttggtttaaattagtactccctatattttagaaaattttattttgtttcatattatagaatgtcttggaaagttctatgtaaatttaaatgtatttagtaacttgtgacgattttatattatgtagtcttttttaggatttgttgattttttaaaataaattttttaaagaaaaaaaacaaattattttaataaacatgcctttaccttatacagtttatattttgaaagagagatagtatgttttaggatatatttaaagaaaaaaaaataactctttaattta

SEQ ID NO: 32 - DNA, 4100 bp, Artificial Sequence
  Plasmid-2: GEiGS_ mir173_si-GFP_2
cacttatcatttagacagtagattttaaatttgtatttacaatttcaaaactgaaattcatttgtaatcaaagaaaaacaaaacaagaaaagggaggaggagtgggatttgggttgcttaacagtattatatatacacgtcgttagttaatcaataaattatgagcaggtgtagtagctatgaacatggttttaccaaattggtaaattcatgtcattgttgtagcactttagcgaggccagcaaaatggcgttcttggaaagggcatggcggcccgtggccgccagggatatgtgtgcagctagaaggattagaaggagtaacttcacctttttgtagaaactgtaaattgccaagacgctcgtttggtaaataccttaacgcttcgtttgctggaatgtgtaccaccattagtagaagaaagtataataagactattaatgcaagagattttttcatattccttttctaagagtagaatggaatgaataaatgaatgaatgaaatagggtttttcttgtttagatcctgtcgcacccgagaataatagaagctgaattaattggtgaagagttttatggtggcgatgttgtatttatagagggaaatgatttcaagtttacaatgggatttttaatttgttttgttgactattatcttgcggagagatcttgactgttgacatgtatgtagtgtttgttattaaaataaatgcatttttgtagacccgattcttaaatatgttaggcatggtcaaattgttagactgtaaaagcttgagtagagacatcggtcaactttgtttacaagaattctctataaaatattatacaaattgatcggtagaaattagatggaacattttgaattaatgtttgacaatgtataaattggtttggtcaatatctaggaatgaaaacaagagctgcttcaaagttgttccattcttaagtatacatagaggtggcttgatgggaagtttcatggaagtgtagttttatatctacttccaaattcgttgatctgtttcttatctcaagctaaacatgtttagaaaagatgtgttaaaaacatgtgacaaaaaaagagtcaaatgtttggcaaacaaggtacttagatttttggcatctattcaaatataatagaatcccaaaattatgatatttgtcaatcaaatttgaaaaaaaaaaaaaaaaaaaaaaagattctacaaaagatcaaacgtattgccgtagatttatcataattttaattctttcacactaccactagtccactaccatatagtgatgagataatccataatcataaataagatataactttcgaattcttgtttttgttgcctcaaagttgttggatcattattttttacgtaaatgtggcttaatgagaatttatgtttgtgggaattgtagtttgcttccaactttttttttttttttttgaacacgtagtttgcttccaacttagtttatctttttcttatttcaagttaaacatgtaaaaaaacatgtgacgacgaaattcaatcagttcctccaatgtttggcagaagccaaatctttggtaaacaaagtaatttttttgccatttgattggttagtataggagaatttaaaaacgacgataaggtttaggtaaattatttcatttgaaaataattgagcaccgttaataattttcatccataaaataatatttcaaagatgatatttgatccccattaaattcattcgtaaccaaaaaaaagttatgaaaaaagagtggtcgtgtgagttgcccaagcaccattataataaaaaataaaataattagcaagtaataaggaataaaatcctgtaattatagctgaaaaaggaaaaatatttggagaccgtcagattcgaatctgaacaaagcataaaaaagtcaacaaaacttaaagcggcggtctcatcgtaatctcagcccaataccctattttcctctcccctatataaatactttcttcttctactgatcttcttctcacaaataaacccaaatatatcaatctactgtgttggtgattaagtacttagttgtactccagcttgtgccagtggtcaaaaaagttgtagttttcttaaagtctctttcctctggcaaagctgcagtacaactaagagcttgctccctaaacttatctctctgatgatttaatgttagagatcttcgtaaatctatgtgtttgatagatctgatgcgttttttgagttgatgatttgattatttttcactggaaagtatctcattagggtaacgataatgttttatggatttggttgtataacagatccatgaaatcttgactggttataaaatctgaataatgtatttcaatttggagattcggtgataaaaattactgatttacgaatgacatttatatcgatagatgagtttgctgatttggttgttaaattgataaatcaaggacatgagaaactgtttttgtatgctaatttgtccatggaataaaattgggaggtgaggaccgtgagggtagtcaggaaaccttaatattgaagttgatgttgaaccaacaaatctgcccaaaaatgataaaagttgatgccgagcccacaaattttgatgacaatcgataagcccaagcccaaaaggcatctgtacctgagcccattattctttcattactagcaaaaaggatgcattagagaccccggtgtagtaaattgacctcacaattcactattgtattgtatacgtacatttcaagcgtaattaaaccctcatatttttatacgctttaaatataattggcctttaattagctcaaataaactagatgtcgtacgtgatcacggtggatgaaatcaatggtattatgaaaagactgtacatgatttcaaatattttaatgtggtcgtaaaaattgttgtttatagtggaaattgaagacaacaacgttactgaaacacatacagattgaaatttcgatcatttacttgcaaagtgttaccgtggaggcgtggcgtggacgtaaggtaccataatggtttgtgttacagtcacgccactacactcgaattcaagctaccatattataatacgttgttgattagaaaaaatagtcgccaattttctttaaaacaaatttcagtttttatttgtcagcaaaaaaaacttactaacacaacggaagaacacaaaaattagggagttgctcacagagcaaaagtaatagaaatgggaaaagctaatatacgtccgagtaggaaactaatcttgcaaaaactgatgaaagcaatcagaagccttgacgtttgtctggagagaggaattgtgttttggatcactttgttcagtttgttgtggatcgtcttccgttacgttctcaccaaaaatatttcataatgaaacaaaaaaattaattaataatggtagcttagaatgccaagttgagaacagatttgcagtttgtcccggaatgatcaagtagagcattcatagtgtcttgccaatatggtgtgatcaacgaagtttgacaaaaccgtgaagatataggaacatgtaatcatgcggctctccatacaatacatcttgttgacaaagttcccaagacctcattctacaaaccaatgtttcttttttctttttctttttggtgatagtttttgcaatcaaatgttgtaaaactatgattggaaatactactgtattttaccgaaaactttattatatatagtcattaacactcattaccaatcacataatcaatagtctattttgattatacaacttttaaacaataaagacatgtttatacagatttggtttaaattagtactccctatattttagaaaattttattttgtttcatattatagaatgtcttggaaagttctatgtaaatttaaatgtatttagtaacttgtgacgattttatattatgtagtcttttttaggatttgttgattttttaaaataaattttttaaagaaaaaaaacaaattattttaataaacatgcctttaccttatacagtttatattttgaaagagagatagtatgttttaggatatatttaaagaaaaaaaaataactctttaattta

SEQ ID NO: 33 - DNA, 4100 bp, Artificial Sequence
  Plasmid-3: GEiGS_ mir173_si-PDS_1
cacttatcatttagacagtagattttaaatttgtatttacaatttcaaaactgaaattcatttgtaatcaaagaaaaacaaaacaagaaaagggaggaggagtgggatttgggttgcttaacagtattatatatacacgtcgttagttaatcaataaattatgagcaggtgtagtagctatgaacatggttttaccaaattggtaaattcatgtcattgttgtagcactttagcgaggccagcaaaatggcgttcttggaaagggcatggcggcccgtggccgccagggatatgtgtgcagctagaaggattagaaggagtaacttcacctttttgtagaaactgtaaattgccaagacgctcgtttggtaaataccttaacgcttcgtttgctggaatgtgtaccaccattagtagaagaaagtataataagactattaatgcaagagattttttcatattccttttctaagagtagaatggaatgaataaatgaatgaatgaaatagggtttttcttgtttagatcctgtcgcacccgagaataatagaagctgaattaattggtgaagagttttatggtggcgatgttgtatttatagagggaaatgatttcaagtttacaatgggatttttaatttgttttgttgactattatcttgcggagagatcttgactgttgacatgtatgtagtgtttgttattaaaataaatgcatttttgtagacccgattcttaaatatgttaggcatggtcaaattgttagactgtaaaagcttgagtagagacatcggtcaactttgtttacaagaattctctataaaatattatacaaattgatcggtagaaattagatggaacattttgaattaatgtttgacaatgtataaattggtttggtcaatatctaggaatgaaaacaagagctgcttcaaagttgttccattcttaagtatacatagaggtggcttgatgggaagtttcatggaagtgtagttttatatctacttccaaattcgttgatctgtttcttatctcaagctaaacatgtttagaaaagatgtgttaaaaacatgtgacaaaaaaagagtcaaatgtttggcaaacaaggtacttagatttttggcatctattcaaatataatagaatcccaaaattatgatatttgtcaatcaaatttgaaaaaaaaaaaaaaaaaaaaaaagattctacaaaagatcaaacgtattgccgtagatttatcataattttaattctttcacactaccactagtccactaccatatagtgatgagataatccataatcataaataagatataactttcgaattcttgtttttgttgcctcaaagttgttggatcattattttttacgtaaatgtggcttaatgagaatttatgtttgtgggaattgtagtttgcttccaactttttttttttttttttgaacacgtagtttgcttccaacttagtttatctttttcttatttcaagttaaacatgtaaaaaaacatgtgacgacgaaattcaatcagttcctccaatgtttggcagaagccaaatctttggtaaacaaagtaatttttttgccatttgattggttagtataggagaatttaaaaacgacgataaggtttaggtaaattatttcatttgaaaataattgagcaccgttaataattttcatccataaaataatatttcaaagatgatatttgatccccattaaattcattcgtaaccaaaaaaaagttatgaaaaaagagtggtcgtgtgagttgcccaagcaccattataataaaaaataaaataattagcaagtaataaggaataaaatcctgtaattatagctgaaaaaggaaaaatatttggagaccgtcagattcgaatctgaacaaagcataaaaaagtcaacaaaacttaaagcggcggtctcatcgtaatctcagcccaataccctattttcctctcccctatataaatactttcttcttctactgatcttcttctcacaaataaacccaaatatatcaatctactgtgttggtgattaagtactttatccacacaaactacctgcaagtggtcaaaaaagttgtagttttcttaaagtctctttcctcttgcagtagttagtgtggataaagagcttgctccctaaacttatctctctgatgatttaatgttagagatcttcgtaaatctatgtgtttgatagatctgatgcgttttttgagttgatgatttgattatttttcactggaaagtatctcattagggtaacgataatgttttatggatttggttgtataacagatccatgaaatcttgactggttataaaatctgaataatgtatttcaatttggagattcggtgataaaaattactgatttacgaatgacatttatatcgatagatgagtttgctgatttggttgttaaattgataaatcaaggacatgagaaactgtttttgtatgctaatttgtccatggaataaaattgggaggtgaggaccgtgagggtagtcaggaaaccttaatattgaagttgatgttgaaccaacaaatctgcccaaaaatgataaaagttgatgccgagcccacaaattttgatgacaatcgataagcccaagcccaaaaggcatctgtacctgagcccattattctttcattactagcaaaaaggatgcattagagaccccggtgtagtaaattgacctcacaattcactattgtattgtatacgtacatttcaagcgtaattaaaccctcatatttttatacgctttaaatataattggcctttaattagctcaaataaactagatgtcgtacgtgatcacggtggatgaaatcaatggtattatgaaaagactgtacatgatttcaaatattttaatgtggtcgtaaaaattgttgtttatagtggaaattgaagacaacaacgttactgaaacacatacagattgaaatttcgatcatttacttgcaaagtgttaccgtggaggcgtggcgtggacgtaaggtaccataatggtttgtgttacagtcacgccactacactcgaattcaagctaccatattataatacgttgttgattagaaaaaatagtcgccaattttctttaaaacaaatttcagtttttatttgtcagcaaaaaaaacttactaacacaacggaagaacacaaaaattagggagttgctcacagagcaaaagtaatagaaatgggaaaagctaatatacgtccgagtaggaaactaatcttgcaaaaactgatgaaagcaatcagaagccttgacgtttgtctggagagaggaattgtgttttggatcactttgttcagtttgttgtggatcgtcttccgttacgttctcaccaaaaatatttcataatgaaacaaaaaaattaattaataatggtagcttagaatgccaagttgagaacagatttgcagtttgtcccggaatgatcaagtagagcattcatagtgtcttgccaatatggtgtgatcaacgaagtttgacaaaaccgtgaagatataggaacatgtaatcatgcggctctccatacaatacatcttgttgacaaagttcccaagacctcattctacaaaccaatgtttcttttttctttttctttttggtgatagtttttgcaatcaaatgttgtaaaactatgattggaaatactactgtattttaccgaaaactttattatatatagtcattaacactcattaccaatcacataatcaatagtctattttgattatacaacttttaaacaataaagacatgtttatacagatttggtttaaattagtactccctatattttagaaaattttattttgtttcatattatagaatgtcttggaaagttctatgtaaatttaaatgtatttagtaacttgtgacgattttatattatgtagtcttttttaggatttgttgattttttaaaataaattttttaaagaaaaaaaacaaattattttaataaacatgcctttaccttatacagtttatattttgaaagagagatagtatgttttaggatatatttaaagaaaaaaaaataactctttaattta

SEQ ID NO: 34 - DNA, 4100 bp, Artificial Sequence
  Plasmid-4: GEiGS_ mir173_si-PDS_2
cacttatcatttagacagtagattttaaatttgtatttacaatttcaaaactgaaattcatttgtaatcaaagaaaaacaaaacaagaaaagggaggaggagtgggatttgggttgcttaacagtattatatatacacgtcgttagttaatcaataaattatgagcaggtgtagtagctatgaacatggttttaccaaattggtaaattcatgtcattgttgtagcactttagcgaggccagcaaaatggcgttcttggaaagggcatggcggcccgtggccgccagggatatgtgtgcagctagaaggattagaaggagtaacttcacctttttgtagaaactgtaaattgccaagacgctcgtttggtaaataccttaacgcttcgtttgctggaatgtgtaccaccattagtagaagaaagtataataagactattaatgcaagagattttttcatattccttttctaagagtagaatggaatgaataaatgaatgaatgaaatagggtttttcttgtttagatcctgtcgcacccgagaataatagaagctgaattaattggtgaagagttttatggtggcgatgttgtatttatagagggaaatgatttcaagtttacaatgggatttttaatttgttttgttgactattatcttgcggagagatcttgactgttgacatgtatgtagtgtttgttattaaaataaatgcatttttgtagacccgattcttaaatatgttaggcatggtcaaattgttagactgtaaaagcttgagtagagacatcggtcaactttgtttacaagaattctctataaaatattatacaaattgatcggtagaaattagatggaacattttgaattaatgtttgacaatgtataaattggtttggtcaatatctaggaatgaaaacaagagctgcttcaaagttgttccattcttaagtatacatagaggtggcttgatgggaagtttcatggaagtgtagttttatatctacttccaaattcgttgatctgtttcttatctcaagctaaacatgtttagaaaagatgtgttaaaaacatgtgacaaaaaaagagtcaaatgtttggcaaacaaggtacttagatttttggcatctattcaaatataatagaatcccaaaattatgatatttgtcaatcaaatttgaaaaaaaaaaaaaaaaaaaaaaagattctacaaaagatcaaacgtattgccgtagatttatcataattttaattctttcacactaccactagtccactaccatatagtgatgagataatccataatcataaataagatataactttcgaattcttgtttttgttgcctcaaagttgttggatcattattttttacgtaaatgtggcttaatgagaatttatgtttgtgggaattgtagtttgcttccaactttttttttttttttttgaacacgtagtttgcttccaacttagtttatctttttcttatttcaagttaaacatgtaaaaaaacatgtgacgacgaaattcaatcagttcctccaatgtttggcagaagccaaatctttggtaaacaaagtaatttttttgccatttgattggttagtataggagaatttaaaaacgacgataaggtttaggtaaattatttcatttgaaaataattgagcaccgttaataattttcatccataaaataatatttcaaagatgatatttgatccccattaaattcattcgtaaccaaaaaaaagttatgaaaaaagagtggtcgtgtgagttgcccaagcaccattataataaaaaataaaataattagcaagtaataaggaataaaatcctgtaattatagctgaaaaaggaaaaatatttggagaccgtcagattcgaatctgaacaaagcataaaaaagtcaacaaaacttaaagcggcggtctcatcgtaatctcagcccaataccctattttcctctcccctatataaatactttcttcttctactgatcttcttctcacaaataaacccaaatatatcaatctactgtgttggtgattaagtactttgacaatccagccaatccagcagtggtcaaaaaagttgtagttttcttaaagtctctttcctctgctgattggcaggattgtcaaagagcttgctccctaaacttatctctctgatgatttaatgttagagatcttcgtaaatctatgtgtttgatagatctgatgcgttttttgagttgatgatttgattatttttcactggaaagtatctcattagggtaacgataatgttttatggatttggttgtataacagatccatgaaatcttgactggttataaaatctgaataatgtatttcaatttggagattcggtgataaaaattactgatttacgaatgacatttatatcgatagatgagtttgctgatttggttgttaaattgataaatcaaggacatgagaaactgtttttgtatgctaatttgtccatggaataaaattgggaggtgaggaccgtgagggtagtcaggaaaccttaatattgaagttgatgttgaaccaacaaatctgcccaaaaatgataaaagttgatgccgagcccacaaattttgatgacaatcgataagcccaagcccaaaaggcatctgtacctgagcccattattctttcattactagcaaaaaggatgcattagagaccccggtgtagtaaattgacctcacaattcactattgtattgtatacgtacatttcaagcgtaattaaaccctcatatttttatacgctttaaatataattggcctttaattagctcaaataaactagatgtcgtacgtgatcacggtggatgaaatcaatggtattatgaaaagactgtacatgatttcaaatattttaatgtggtcgtaaaaattgttgtttatagtggaaattgaagacaacaacgttactgaaacacatacagattgaaatttcgatcatttacttgcaaagtgttaccgtggaggcgtggcgtggacgtaaggtaccataatggtttgtgttacagtcacgccactacactcgaattcaagctaccatattataatacgttgttgattagaaaaaatagtcgccaattttctttaaaacaaatttcagtttttatttgtcagcaaaaaaaacttactaacacaacggaagaacacaaaaattagggagttgctcacagagcaaaagtaatagaaatgggaaaagctaatatacgtccgagtaggaaactaatcttgcaaaaactgatgaaagcaatcagaagccttgacgtttgtctggagagaggaattgtgttttggatcactttgttcagtttgttgtggatcgtcttccgttacgttctcaccaaaaatatttcataatgaaacaaaaaaattaattaataatggtagcttagaatgccaagttgagaacagatttgcagtttgtcccggaatgatcaagtagagcattcatagtgtcttgccaatatggtgtgatcaacgaagtttgacaaaaccgtgaagatataggaacatgtaatcatgcggctctccatacaatacatcttgttgacaaagttcccaagacctcattctacaaaccaatgtttcttttttctttttctttttggtgatagtttttgcaatcaaatgttgtaaaactatgattggaaatactactgtattttaccgaaaactttattatatatagtcattaacactcattaccaatcacataatcaatagtctattttgattatacaacttttaaacaataaagacatgtttatacagatttggtttaaattagtactccctatattttagaaaattttattttgtttcatattatagaatgtcttggaaagttctatgtaaatttaaatgtatttagtaacttgtgacgattttatattatgtagtcttttttaggatttgttgattttttaaaataaattttttaaagaaaaaaaacaaattattttaataaacatgcctttaccttatacagtttatattttgaaagagagatagtatgttttaggatatatttaaagaaaaaaaaataactctttaattta

SEQ ID NO: 35 - DNA, 4000 bp, Artificial Sequence
  Plasmid-5: GEiGS_ mir390a _si-GFP_1
accctcattgattttggtggccaaactcttgatcgtattcttttaggaacagtaattaattttaaatttgagaaaaatgtagtgatgaaagtgagatatatgggacgcactattgaaagcattgtccacaccgcatgatgtgagattgatgtgaatatggtaactaataacacccagactcacttttatgagaaaatgtatcttaaaaaatgttattcatcaaagcttagatgcgctataggggaacataatcattatttgaaaagaaccaattcaaatatttttttttttaagagttaaaatcctatataacataaccatccaaactttgggcatgaacacaacaatattttttttcgtttttgataaattctttcaattgcaatcaaaacttaccagctatacaaatgtttgctgcatccaatctaatacaccgttaaacaataaaatttgttatctctcaaatctgatcatctattccaacctgactgttttattctagtattttaaggccaggtataacgaaaacaaagaaaaaagttcagcgaccaagacattttgacatcaggctcaaacggtcaaacccacgaaaacttttacctcatttcttaaccacgcagtgttatttgaatagccttaataggctaatacaaaacaacaagccatcgattacagttttaactataatattacaaaatcttaaaccaaaacaagaaaagatatatattccgtaaaattaaaataatatttttaatatagtcattatgtaagttagctctttcgacaaaatcattataaattaggccattttgtaagttagttcttttatcgacaagccattataacttaggtaattttgtaagttagctggactataaccaatttttttgtttcacatctagagtataaaacacatatatattgaccgtacaactttagtcaaattagaaactctgttttatctgcagaaaagaaaaaaaaagaggatgaattatgtaaatacttcaggattagaaataatgtcatcgtatatctcttgatatgaatacatattttacttgactagtaccgtagtcggcaggaaaatgacacaaacaaccatctaaaaagataaagtaagaactaaaaagtcttgacattcattagtttaatcattttctgttaacatatatggaaaaaacaaacttcaccgttatttacctgaatttacctatttgggtaagaattgtacctctggacctctagtattttatatacacctaaaaatataattttggtcgggaaaatataactctgtttaattaattaaattttcagtattgtgtaagtgtaattatagaaatcaattttatccgcgtaacaaaataatataaaattatactttcaaatccacgaatatatattgtgaagtctcatagtttgcaaataagcattggtcttcggccgacaaaaaaaaaagcattggtcttcgaatattttgaatatcggaccaatggtatataattaataatatgtggtatataaatacatatttatttaaatcacaataggatatgcaatgtgtgtatatatacatatacgtaattaaagtccgggttaaactgatagcatatattataatagatgcatctataattgttcgtcaacaaaagcattatcatgtattttgaattaagcttccttcatttctgtgaatcaaaaggcctcagaagaagaaactaaagtcaaacaatcaacgggatccaataaatcacatctggactatatagtatcaatactttccacactaaaaaagctaagaaatttaataaatacattattataggggggaaaaaaaggtagtcatcagatatatattttggtaagaaaatatagaaatgaataatttcacgtttaacgaagaggagatgacgtgtgttccttcgaacccgagttttgttcgtctataaatagcaccttctcttctccttcttcctcacttccatctttttagcttcactatctctctataatcggttttatctttctctaagtcacaacccaaaaaaacaaagtagagaagaatctgtaaagtcgtgctgcttcatgtggatgatgatcacattcgttatctattttttccacatgaagaagcacgacttgattggctcttcttactacaatgaaaaaggccgaggcaaaacgcctaaaatcacttgagaatcaattctttttactgtccatttaagctatcttttataaacgtgtcttattttctatctcttttgtttaaactaagaaactatagtattttgtctaaaacaaaacatgaaagaacagattagatctcatctttagtctctttctccggtgcagtcagccaccgtcgggtaagtttcatctgtattttattaattaattacaattattagtgttcttattaccgttttggtaaaattagttaattaatgtcggtccaaacattctaaaccaattattctgaaaagggtgaacgccaatcagttatatacaatattcttacattaaagtagaatcggagatgttacatactaaccaaaagttacatatactagtatcattttctttaagatttgtttaggatttactcactttatagtgctcgcggttggggtcagggtaagtggggaacagatatgctctgcatgaaccacgtggaccaacatgcatatacacagttacatttattttttctagtaggttcatttgcaaattttccagtatcttgtatgttatcttcatggtgagttttttggtcgcatattcttggtgattcttcttctacgttttcactttcttcttcagagaccttattaatatgttaattgcatgaatttatgtaacattcaagaaaaagagatcgaatacaagaaaccggaaatttaatttctaatttgaattctatgcatgtttgtttctttgccaatttagtacgaatatatttatggtccggagttctaaccaaagatagttgctctgtatatagaagttatacatctcgcttgtttaaactaaataactatttagtttgtcttggtagtccagtgactttctgcaaacattgggatttataatatagtcaaaacgttgggatatgtagtattcattttcgttgtaaaaatcattatattttgcaaaggttgcaacgtaaaacgttgtattgaatttaggagaaagtagccatttacaatgaattttagtgacaaactgttgtatacagcctgtgccactaagtatgtctatatctaaatttggaatggatgataaccagtattggtcaataatggataatttggtatttagaattactaatttggtattttagtgacaaactgttgtatggaatttaggagaacgcgttcccaagctatatattatatgtatttcattctttcatatgttatattatgaattgttataaaaaagaccaatgagcaacggtttaaggtttaatcagtaatcgatccgaccaatcatatacaagttcctaacacatcttctaactactgagtaaaatagtaatgctattacaaaggttttttcttttcaaaatacagcctaatgctactacaaaattctaatgttataaaataatcataggagaagtaaaccccggtatttaattaataccttacaaacttacattattgataaagttgaatgaagagttatatggtccatttagtattatttacttaatatgatactagtgttagacgtgttactgtatttcaacgtgcataatcaggttgttcaaaaagagagaggataggtcttcttcttctgtaatttgctgggaccgcaagtcatgtgaggctgctctgctgatgctgcacggcgtcgcaactctctcaataaattcttttaactaacgctccaattttcgatgtaaattggctgacttcaattctatgccttactcttgtactctatgtttctttatctattaaaatccaactctgcttttgaacccaaaaaacaa

SEQ ID NO: 36 - DNA, 4000 bp, Artificial Sequence
  Plasmid-6: GEiGS_ mir390a _si-GFP_2
accctcattgattttggtggccaaactcttgatcgtattcttttaggaacagtaattaattttaaatttgagaaaaatgtagtgatgaaagtgagatatatgggacgcactattgaaagcattgtccacaccgcatgatgtgagattgatgtgaatatggtaactaataacacccagactcacttttatgagaaaatgtatcttaaaaaatgttattcatcaaagcttagatgcgctataggggaacataatcattatttgaaaagaaccaattcaaatatttttttttttaagagttaaaatcctatataacataaccatccaaactttgggcatgaacacaacaatattttttttcgtttttgataaattctttcaattgcaatcaaaacttaccagctatacaaatgtttgctgcatccaatctaatacaccgttaaacaataaaatttgttatctctcaaatctgatcatctattccaacctgactgttttattctagtattttaaggccaggtataacgaaaacaaagaaaaaagttcagcgaccaagacattttgacatcaggctcaaacggtcaaacccacgaaaacttttacctcatttcttaaccacgcagtgttatttgaatagccttaataggctaatacaaaacaacaagccatcgattacagttttaactataatattacaaaatcttaaaccaaaacaagaaaagatatatattccgtaaaattaaaataatatttttaatatagtcattatgtaagttagctctttcgacaaaatcattataaattaggccattttgtaagttagttcttttatcgacaagccattataacttaggtaattttgtaagttagctggactataaccaatttttttgtttcacatctagagtataaaacacatatatattgaccgtacaactttagtcaaattagaaactctgttttatctgcagaaaagaaaaaaaaagaggatgaattatgtaaatacttcaggattagaaataatgtcatcgtatatctcttgatatgaatacatattttacttgactagtaccgtagtcggcaggaaaatgacacaaacaaccatctaaaaagataaagtaagaactaaaaagtcttgacattcattagtttaatcattttctgttaacatatatggaaaaaacaaacttcaccgttatttacctgaatttacctatttgggtaagaattgtacctctggacctctagtattttatatacacctaaaaatataattttggtcgggaaaatataactctgtttaattaattaaattttcagtattgtgtaagtgtaattatagaaatcaattttatccgcgtaacaaaataatataaaattatactttcaaatccacgaatatatattgtgaagtctcatagtttgcaaataagcattggtcttcggccgacaaaaaaaaaagcattggtcttcgaatattttgaatatcggaccaatggtatataattaataatatgtggtatataaatacatatttatttaaatcacaataggatatgcaatgtgtgtatatatacatatacgtaattaaagtccgggttaaactgatagcatatattataatagatgcatctataattgttcgtcaacaaaagcattatcatgtattttgaattaagcttccttcatttctgtgaatcaaaaggcctcagaagaagaaactaaagtcaaacaatcaacgggatccaataaatcacatctggactatatagtatcaatactttccacactaaaaaagctaagaaatttaataaatacattattataggggggaaaaaaaggtagtcatcagatatatattttggtaagaaaatatagaaatgaataatttcacgtttaacgaagaggagatgacgtgtgttccttcgaacccgagttttgttcgtctataaatagcaccttctcttctccttcttcctcacttccatctttttagcttcactatctctctataatcggttttatctttctctaagtcacaacccaaaaaaacaaagtagagaagaatctgtaagttgtactccagcttgtgccatgatgatcacattcgttatctattttttggcacaagcttgagtacaactgattggctcttcttactacaatgaaaaaggccgaggcaaaacgcctaaaatcacttgagaatcaattctttttactgtccatttaagctatcttttataaacgtgtcttattttctatctcttttgtttaaactaagaaactatagtattttgtctaaaacaaaacatgaaagaacagattagatctcatctttagtctctttctccggtgcagtcagccaccgtcgggtaagtttcatctgtattttattaattaattacaattattagtgttcttattaccgttttggtaaaattagttaattaatgtcggtccaaacattctaaaccaattattctgaaaagggtgaacgccaatcagttatatacaatattcttacattaaagtagaatcggagatgttacatactaaccaaaagttacatatactagtatcattttctttaagatttgtttaggatttactcactttatagtgctcgcggttggggtcagggtaagtggggaacagatatgctctgcatgaaccacgtggaccaacatgcatatacacagttacatttattttttctagtaggttcatttgcaaattttccagtatcttgtatgttatcttcatggtgagttttttggtcgcatattcttggtgattcttcttctacgttttcactttcttcttcagagaccttattaatatgttaattgcatgaatttatgtaacattcaagaaaaagagatcgaatacaagaaaccggaaatttaatttctaatttgaattctatgcatgtttgtttctttgccaatttagtacgaatatatttatggtccggagttctaaccaaagatagttgctctgtatatagaagttatacatctcgcttgtttaaactaaataactatttagtttgtcttggtagtccagtgactttctgcaaacattgggatttataatatagtcaaaacgttgggatatgtagtattcattttcgttgtaaaaatcattatattttgcaaaggttgcaacgtaaaacgttgtattgaatttaggagaaagtagccatttacaatgaattttagtgacaaactgttgtatacagcctgtgccactaagtatgtctatatctaaatttggaatggatgataaccagtattggtcaataatggataatttggtatttagaattactaatttggtattttagtgacaaactgttgtatggaatttaggagaacgcgttcccaagctatatattatatgtatttcattctttcatatgttatattatgaattgttataaaaaagaccaatgagcaacggtttaaggtttaatcagtaatcgatccgaccaatcatatacaagttcctaacacatcttctaactactgagtaaaatagtaatgctattacaaaggttttttcttttcaaaatacagcctaatgctactacaaaattctaatgttataaaataatcataggagaagtaaaccccggtatttaattaataccttacaaacttacattattgataaagttgaatgaagagttatatggtccatttagtattatttacttaatatgatactagtgttagacgtgttactgtatttcaacgtgcataatcaggttgttcaaaaagagagaggataggtcttcttcttctgtaatttgctgggaccgcaagtcatgtgaggctgctctgctgatgctgcacggcgtcgcaactctctcaataaattcttttaactaacgctccaattttcgatgtaaattggctgacttcaattctatgccttactcttgtactctatgtttctttatctattaaaatccaactctgcttttgaacccaaaaaacaa

SEQ ID NO: 37 - DNA, 4000 bp, Artificial Sequence
  Plasmid-7: GEiGS_ mir390a _si-PDS_1
accctcattgattttggtggccaaactcttgatcgtattcttttaggaacagtaattaattttaaatttgagaaaaatgtagtgatgaaagtgagatatatgggacgcactattgaaagcattgtccacaccgcatgatgtgagattgatgtgaatatggtaactaataacacccagactcacttttatgagaaaatgtatcttaaaaaatgttattcatcaaagcttagatgcgctataggggaacataatcattatttgaaaagaaccaattcaaatatttttttttttaagagttaaaatcctatataacataaccatccaaactttgggcatgaacacaacaatattttttttcgtttttgataaattctttcaattgcaatcaaaacttaccagctatacaaatgtttgctgcatccaatctaatacaccgttaaacaataaaatttgttatctctcaaatctgatcatctattccaacctgactgttttattctagtattttaaggccaggtataacgaaaacaaagaaaaaagttcagcgaccaagacattttgacatcaggctcaaacggtcaaacccacgaaaacttttacctcatttcttaaccacgcagtgttatttgaatagccttaataggctaatacaaaacaacaagccatcgattacagttttaactataatattacaaaatcttaaaccaaaacaagaaaagatatatattccgtaaaattaaaataatatttttaatatagtcattatgtaagttagctctttcgacaaaatcattataaattaggccattttgtaagttagttcttttatcgacaagccattataacttaggtaattttgtaagttagctggactataaccaatttttttgtttcacatctagagtataaaacacatatatattgaccgtacaactttagtcaaattagaaactctgttttatctgcagaaaagaaaaaaaaagaggatgaattatgtaaatacttcaggattagaaataatgtcatcgtatatctcttgatatgaatacatattttacttgactagtaccgtagtcggcaggaaaatgacacaaacaaccatctaaaaagataaagtaagaactaaaaagtcttgacattcattagtttaatcattttctgttaacatatatggaaaaaacaaacttcaccgttatttacctgaatttacctatttgggtaagaattgtacctctggacctctagtattttatatacacctaaaaatataattttggtcgggaaaatataactctgtttaattaattaaattttcagtattgtgtaagtgtaattatagaaatcaattttatccgcgtaacaaaataatataaaattatactttcaaatccacgaatatatattgtgaagtctcatagtttgcaaataagcattggtcttcggccgacaaaaaaaaaagcattggtcttcgaatattttgaatatcggaccaatggtatataattaataatatgtggtatataaatacatatttatttaaatcacaataggatatgcaatgtgtgtatatatacatatacgtaattaaagtccgggttaaactgatagcatatattataatagatgcatctataattgttcgtcaacaaaagcattatcatgtattttgaattaagcttccttcatttctgtgaatcaaaaggcctcagaagaagaaactaaagtcaaacaatcaacgggatccaataaatcacatctggactatatagtatcaatactttccacactaaaaaagctaagaaatttaataaatacattattataggggggaaaaaaaggtagtcatcagatatatattttggtaagaaaatatagaaatgaataatttcacgtttaacgaagaggagatgacgtgtgttccttcgaacccgagttttgttcgtctataaatagcaccttctcttctccttcttcctcacttccatctttttagcttcactatctctctataatcggttttatctttctctaagtcacaacccaaaaaaacaaagtagagaagaatctgtatatccacacaaactacctgcaatgatgatcacattcgttatctatttttttgcaggtagtgtgtgtggatagattggctcttcttactacaatgaaaaaggccgaggcaaaacgcctaaaatcacttgagaatcaattctttttactgtccatttaagctatcttttataaacgtgtcttattttctatctcttttgtttaaactaagaaactatagtattttgtctaaaacaaaacatgaaagaacagattagatctcatctttagtctctttctccggtgcagtcagccaccgtcgggtaagtttcatctgtattttattaattaattacaattattagtgttcttattaccgttttggtaaaattagttaattaatgtcggtccaaacattctaaaccaattattctgaaaagggtgaacgccaatcagttatatacaatattcttacattaaagtagaatcggagatgttacatactaaccaaaagttacatatactagtatcattttctttaagatttgtttaggatttactcactttatagtgctcgcggttggggtcagggtaagtggggaacagatatgctctgcatgaaccacgtggaccaacatgcatatacacagttacatttattttttctagtaggttcatttgcaaattttccagtatcttgtatgttatcttcatggtgagttttttggtcgcatattcttggtgattcttcttctacgttttcactttcttcttcagagaccttattaatatgttaattgcatgaatttatgtaacattcaagaaaaagagatcgaatacaagaaaccggaaatttaatttctaatttgaattctatgcatgtttgtttctttgccaatttagtacgaatatatttatggtccggagttctaaccaaagatagttgctctgtatatagaagttatacatctcgcttgtttaaactaaataactatttagtttgtcttggtagtccagtgactttctgcaaacattgggatttataatatagtcaaaacgttgggatatgtagtattcattttcgttgtaaaaatcattatattttgcaaaggttgcaacgtaaaacgttgtattgaatttaggagaaagtagccatttacaatgaattttagtgacaaactgttgtatacagcctgtgccactaagtatgtctatatctaaatttggaatggatgataaccagtattggtcaataatggataatttggtatttagaattactaatttggtattttagtgacaaactgttgtatggaatttaggagaacgcgttcccaagctatatattatatgtatttcattctttcatatgttatattatgaattgttataaaaaagaccaatgagcaacggtttaaggtttaatcagtaatcgatccgaccaatcatatacaagttcctaacacatcttctaactactgagtaaaatagtaatgctattacaaaggttttttcttttcaaaatacagcctaatgctactacaaaattctaatgttataaaataatcataggagaagtaaaccccggtatttaattaataccttacaaacttacattattgataaagttgaatgaagagttatatggtccatttagtattatttacttaatatgatactagtgttagacgtgttactgtatttcaacgtgcataatcaggttgttcaaaaagagagaggataggtcttcttcttctgtaatttgctgggaccgcaagtcatgtgaggctgctctgctgatgctgcacggcgtcgcaactctctcaataaattcttttaactaacgctccaattttcgatgtaaattggctgacttcaattctatgccttactcttgtactctatgtttctttatctattaaaatccaactctgcttttgaacccaaaaaacaa

SEQ ID NO: 38 - DNA, 4000 bp, Artificial Sequence
  Plasmid-8: GEiGS_ mir390a _si-PDS_2
accctcattgattttggtggccaaactcttgatcgtattcttttaggaacagtaattaattttaaatttgagaaaaatgtagtgatgaaagtgagatatatgggacgcactattgaaagcattgtccacaccgcatgatgtgagattgatgtgaatatggtaactaataacacccagactcacttttatgagaaaatgtatcttaaaaaatgttattcatcaaagcttagatgcgctataggggaacataatcattatttgaaaagaaccaattcaaatatttttttttttaagagttaaaatcctatataacataaccatccaaactttgggcatgaacacaacaatattttttttcgtttttgataaattctttcaattgcaatcaaaacttaccagctatacaaatgtttgctgcatccaatctaatacaccgttaaacaataaaatttgttatctctcaaatctgatcatctattccaacctgactgttttattctagtattttaaggccaggtataacgaaaacaaagaaaaaagttcagcgaccaagacattttgacatcaggctcaaacggtcaaacccacgaaaacttttacctcatttcttaaccacgcagtgttatttgaatagccttaataggctaatacaaaacaacaagccatcgattacagttttaactataatattacaaaatcttaaaccaaaacaagaaaagatatatattccgtaaaattaaaataatatttttaatatagtcattatgtaagttagctctttcgacaaaatcattataaattaggccattttgtaagttagttcttttatcgacaagccattataacttaggtaattttgtaagttagctggactataaccaatttttttgtttcacatctagagtataaaacacatatatattgaccgtacaactttagtcaaattagaaactctgttttatctgcagaaaagaaaaaaaaagaggatgaattatgtaaatacttcaggattagaaataatgtcatcgtatatctcttgatatgaatacatattttacttgactagtaccgtagtcggcaggaaaatgacacaaacaaccatctaaaaagataaagtaagaactaaaaagtcttgacattcattagtttaatcattttctgttaacatatatggaaaaaacaaacttcaccgttatttacctgaatttacctatttgggtaagaattgtacctctggacctctagtattttatatacacctaaaaatataattttggtcgggaaaatataactctgtttaattaattaaattttcagtattgtgtaagtgtaattatagaaatcaattttatccgcgtaacaaaataatataaaattatactttcaaatccacgaatatatattgtgaagtctcatagtttgcaaataagcattggtcttcggccgacaaaaaaaaaagcattggtcttcgaatattttgaatatcggaccaatggtatataattaataatatgtggtatataaatacatatttatttaaatcacaataggatatgcaatgtgtgtatatatacatatacgtaattaaagtccgggttaaactgatagcatatattataatagatgcatctataattgttcgtcaacaaaagcattatcatgtattttgaattaagcttccttcatttctgtgaatcaaaaggcctcagaagaagaaactaaagtcaaacaatcaacgggatccaataaatcacatctggactatatagtatcaatactttccacactaaaaaagctaagaaatttaataaatacattattataggggggaaaaaaaggtagtcatcagatatatattttggtaagaaaatatagaaatgaataatttcacgtttaacgaagaggagatgacgtgtgttccttcgaacccgagttttgttcgtctataaatagcaccttctcttctccttcttcctcacttccatctttttagcttcactatctctctataatcggttttatctttctctaagtcacaacccaaaaaaacaaagtagagaagaatctgtatgacaatccagccaatccagcatgatgatcacattcgttatctattttttgctggattggatggattgtcagattggctcttcttactacaatgaaaaaggccgaggcaaaacgcctaaaatcacttgagaatcaattctttttactgtccatttaagctatcttttataaacgtgtcttattttctatctcttttgtttaaactaagaaactatagtattttgtctaaaacaaaacatgaaagaacagattagatctcatctttagtctctttctccggtgcagtcagccaccgtcgggtaagtttcatctgtattttattaattaattacaattattagtgttcttattaccgttttggtaaaattagttaattaatgtcggtccaaacattctaaaccaattattctgaaaagggtgaacgccaatcagttatatacaatattcttacattaaagtagaatcggagatgttacatactaaccaaaagttacatatactagtatcattttctttaagatttgtttaggatttactcactttatagtgctcgcggttggggtcagggtaagtggggaacagatatgctctgcatgaaccacgtggaccaacatgcatatacacagttacatttattttttctagtaggttcatttgcaaattttccagtatcttgtatgttatcttcatggtgagttttttggtcgcatattcttggtgattcttcttctacgttttcactttcttcttcagagaccttattaatatgttaattgcatgaatttatgtaacattcaagaaaaagagatcgaatacaagaaaccggaaatttaatttctaatttgaattctatgcatgtttgtttctttgccaatttagtacgaatatatttatggtccggagttctaaccaaagatagttgctctgtatatagaagttatacatctcgcttgtttaaactaaataactatttagtttgtcttggtagtccagtgactttctgcaaacattgggatttataatatagtcaaaacgttgggatatgtagtattcattttcgttgtaaaaatcattatattttgcaaaggttgcaacgtaaaacgttgtattgaatttaggagaaagtagccatttacaatgaattttagtgacaaactgttgtatacagcctgtgccactaagtatgtctatatctaaatttggaatggatgataaccagtattggtcaataatggataatttggtatttagaattactaatttggtattttagtgacaaactgttgtatggaatttaggagaacgcgttcccaagctatatattatatgtatttcattctttcatatgttatattatgaattgttataaaaaagaccaatgagcaacggtttaaggtttaatcagtaatcgatccgaccaatcatatacaagttcctaacacatcttctaactactgagtaaaatagtaatgctattacaaaggttttttcttttcaaaatacagcctaatgctactacaaaattctaatgttataaaataatcataggagaagtaaaccccggtatttaattaataccttacaaacttacattattgataaagttgaatgaagagttatatggtccatttagtattatttacttaatatgatactagtgttagacgtgttactgtatttcaacgtgcataatcaggttgttcaaaaagagagaggataggtcttcttcttctgtaatttgctgggaccgcaagtcatgtgaggctgctctgctgatgctgcacggcgtcgcaactctctcaataaattcttttaactaacgctccaattttcgatgtaaattggctgacttcaattctatgccttactcttgtactctatgtttctttatctattaaaatccaactctgcttttgaacccaaaaaacaa

SEQ ID NO: 39 - DNA, 22 bp, Artificial sequence
  Single strand oligonucleotide
ttcgcttgcagagagaaatcac

SEQ ID NO: 40 - DNA, 21 bp, Artificial sequence
  Single strand oligonucleotide
aagctcaggagggatagcgcc

SEQ ID NO: 41 - DNA, 23 bp, Artificial sequence
  Single strand oligonucleotide
cttgcagagagaaatcacagtgg

SEQ ID NO: 42 - DNA, 23 bp, Artificial sequence
  Single strand oligonucleotide
gcttacacagagaatcacagagg

SEQ ID NO: 43 - DNA, 23 bp, Artificial sequence
  Single strand oligonucleotide
aagaatctgtaaagctcaggagg

SEQ ID NO: 44 - DNA, 23 bp, Artificial sequence
  Single strand oligonucleotide
ctatccatcctgagtttcattgg

SEQ ID NO: 45 - DNA, 21 bp, Artificial sequence
  Single strand oligonucleotide
aagtcgtgctgcttcatgtgg

SEQ ID NO: 46 - DNA, 22 bp, Artificial sequence
  Single strand oligonucleotide
ccacataagcaggacgagttaa

SEQ ID NO: 47 - DNA, 21 bp, Artificial sequence
  Single strand oligonucleotide
agttgtactccagcttgtgcc

SEQ ID NO: 48 - DNA, 21 bp, Artificial sequence
  Single strand oligonucleotide
gcaaagctgcagtacaactaa

SEQ ID NO: 49 - DNA, 21 bp, Artificial sequence
  Single strand oligonucleotide
tatccacacaaactacctgca

SEQ ID NO: 50 - DNA, 21 bp, Artificial sequence
  Single strand oligonucleotide
gcagtagttagtgtggataaa

SEQ ID NO: 51 - DNA, 21 bp, Artificial sequence
  Single strand oligonucleotide
tgacaatccagccaatccagc

SEQ ID NO: 52 - DNA, 21 bp, Artificial sequence
  Single strand oligonucleotide
ctgattggcaggattgtcaaa

SEQ ID NO: 53 - DNA, 21 bp, Artificial sequence
  Single strand oligonucleotide
taaagatcggcaacacatgat

SEQ ID NO: 54 - DNA, 19 bp, Artificial sequence
  Single strand oligonucleotide
tcagtgttggcgatcttta

SEQ ID NO: 55 - DNA, 21 bp, Artificial sequence
  Single strand oligonucleotide
tgacctttcttgggtttagcc

SEQ ID NO: 56 - DNA, 19 bp, Artificial sequence
  Single strand oligonucleotide
gctaacccatgaaaggtca

SEQ ID NO: 57 - DNA, 102 bp, Artificial sequence
  Single strand oligonucleotide
taagtactttcgcttgcagagagaaatcacagtggtcaaaaaagttgtagttttcttaaagtctctttcctctgtgattctctgtgtaagcgaaagagcttg

SEQ ID NO: 58 - DNA, 102 bp, Artificial sequence
  Single strand oligonucleotide
taagtacttaagtcgtgctgcttcatgtggagtggtcaaaaaagttgtagttttcttaaagtctctttcctctccacataagcaggacgagttaagagcttg

SEQ ID NO: 59 - DNA, 102 bp, Artificial sequence
  Single strand oligonucleotide
taagtacttagttgtactccagcttgtgccagtggtcaaaaaagttgtagttttcttaaagtctctttcctctggcaaagctgcagtacaactaagagcttg

SEQ ID NO: 60 - DNA, 102 bp, Artificial sequence
  Single strand oligonucleotide
taagtactttatccacacaaactacctgcaagtggtcaaaaaagttgtagttttcttaaagtctctttcctcttgcagtagttagtgtggataaagagcttg

SEQ ID NO: 61 - DNA, 102 bp, Artificial sequence
  Single strand oligonucleotide
taagtactttgacaatccagccaatccagcagtggtcaaaaaagttgtagttttcttaaagtctctttcctctgctgattggcaggattgtcaaagagcttg

SEQ ID NO: 62 - DNA, 102 bp, Artificial sequence
  Single strand oligonucleotide
taagtactttaaagatcggcaacacatgatagtggtcaaaaaagttgtagttttcttaaagtctctttcctctgatcagtgttggcgatctttaagagcttg

SEQ ID NO: 63 - DNA, 102 bp, Artificial sequence
  Single strand oligonucleotide
taagtactttgacctttcttgggtttagccagtggtcaaaaaagttgtagttttcttaaagtctctttcctctgggctaacccatgaaaggtcaagagcttg

SEQ ID NO: 64 - DNA, 107 bp, Artificial sequence
  Single strand oligonucleotide
gtagagaagaatctgtaaagctcaggagggatagcgccatgatgatcacattcgttatctattttttggcgctatccatcctgagtttcattggctcttcttactac

SEQ ID NO: 65 - DNA, 107 bp, Artificial sequence
  Single strand oligonucleotide
gtagagaagaatctgtaaagtcgtgctgcttcatgtggatgatgatcacattcgttatctattttttccacatgaagaagcacgacttgattggctcttcttactac

SEQ ID NO: 66 - DNA, 107 bp, Artificial sequence
  Single strand oligonucleotide
gtagagaagaatctgtaagttgtactccagcttgtgccatgatgatcacattcgttatctattttttggcacaagcttgagtacaactgattggctcttcttactac

SEQ ID NO: 67 - DNA, 107 bp, Artificial sequence
  Single strand oligonucleotide
gtagagaagaatctgtatatccacacaaactacctgcaatgatgatcacattcgttatctatttttttgcaggtagtgtgtgtggatagattggctcttcttactac

SEQ ID NO: 68 - DNA, 107 bp, Artificial sequence
  Single strand oligonucleotide
gtagagaagaatctgtatgacaatccagccaatccagcatgatgatcacattcgttatctattttttgctggattggatggattgtcagattggctcttcttactac

SEQ ID NO: 69 - DNA, 107 bp, Artificial sequence
  Single strand oligonucleotide
gtagagaagaatctgtataaagatcggcaacacatgatatgatgatcacattcgttatctattttttatcatgtgttaccgatctttacattggctcttcttactac

SEQ ID NO: 70 - DNA, 107 bp, Artificial sequence
  Single strand oligonucleotide
gtagagaagaatctgtatgacctttcttgggtttagccatgatgatcacattcgttatctattttttggctaaaccccagaaaggtcacattggctcttcttactac

SEQ ID NO: 71 - DNA, 4100 bp, Artificial sequence
  Single strand oligonucleotide
cacttatcatttagacagtagattttaaatttgtatttacaatttcaaaactgaaattcatttgtaatcaaagaaaaacaaaacaagaaaagggaggaggagtgggatttgggttgcttaacagtattatatatacacgtcgttagttaatcaataaattatgagcaggtgtagtagctatgaacatggttttaccaaattggtaaattcatgtcattgttgtagcactttagcgaggccagcaaaatggcgttcttggaaagggcatggcggcccgtggccgccagggatatgtgtgcagctagaaggattagaaggagtaacttcacctttttgtagaaactgtaaattgccaagacgctcgtttggtaaataccttaacgcttcgtttgctggaatgtgtaccaccattagtagaagaaagtataataagactattaatgcaagagattttttcatattccttttctaagagtagaatggaatgaataaatgaatgaatgaaatagggtttttcttgtttagatcctgtcgcacccgagaataatagaagctgaattaattggtgaagagttttatggtggcgatgttgtatttatagagggaaatgatttcaagtttacaatgggatttttaatttgttttgttgactattatcttgcggagagatcttgactgttgacatgtatgtagtgtttgttattaaaataaatgcatttttgtagacccgattcttaaatatgttaggcatggtcaaattgttagactgtaaaagcttgagtagagacatcggtcaactttgtttacaagaattctctataaaatattatacaaattgatcggtagaaattagatggaacattttgaattaatgtttgacaatgtataaattggtttggtcaatatctaggaatgaaaacaagagctgcttcaaagttgttccattcttaagtatacatagaggtggcttgatgggaagtttcatggaagtgtagttttatatctacttccaaattcgttgatctgtttcttatctcaagctaaacatgtttagaaaagatgtgttaaaaacatgtgacaaaaaaagagtcaaatgtttggcaaacaaggtacttagatttttggcatctattcaaatataatagaatcccaaaattatgatatttgtcaatcaaatttgaaaaaaaaaaaaaaaaaaaaaaagattctacaaaagatcaaacgtattgccgtagatttatcataattttaattctttcacactaccactagtccactaccatatagtgatgagataatccataatcataaataagatataactttcgaattcttgtttttgttgcctcaaagttgttggatcattattttttacgtaaatgtggcttaatgagaatttatgtttgtgggaattgtagtttgcttccaactttttttttttttttttgaacacgtagtttgcttccaacttagtttatctttttcttatttcaagttaaacatgtaaaaaaacatgtgacgacgaaattcaatcagttcctccaatgtttggcagaagccaaatctttggtaaacaaagtaatttttttgccatttgattggttagtataggagaatttaaaaacgacgataaggtttaggtaaattatttcatttgaaaataattgagcaccgttaataattttcatccataaaataatatttcaaagatgatatttgatccccattaaattcattcgtaaccaaaaaaaagttatgaaaaaagagtggtcgtgtgagttgcccaagcaccattataataaaaaataaaataattagcaagtaataaggaataaaatcctgtaattatagctgaaaaaggaaaaatatttggagaccgtcagattcgaatctgaacaaagcataaaaaagtcaacaaaacttaaagcggcggtctcatcgtaatctcagcccaataccctattttcctctcccctatataaatactttcttcttctactgatcttcttctcacaaataaacccaaatatatcaatctactgtgttggtgattaagtactttcgcttgcagagagaaatcacagtggtcaaaaaagttgtagttttcttaaagtctctttcctctgtgattctctgtgtaagcgaaagagcttgctccctaaacttatctctctgatgatttaatgttagagatcttcgtaaatctatgtgtttgatagatctgatgcgttttttgagttgatgatttgattatttttcactggaaagtatctcattagggtaacgataatgttttatggatttggttgtataacagatccatgaaatcttgactggttataaaatctgaataatgtatttcaatttggagattcggtgataaaaattactgatttacgaatgacatttatatcgatagatgagtttgctgatttggttgttaaattgataaatcaaggacatgagaaactgtttttgtatgctaatttgtccatggaataaaattgggaggtgaggaccgtgagggtagtcaggaaaccttaatattgaagttgatgttgaaccaacaaatctgcccaaaaatgataaaagttgatgccgagcccacaaattttgatgacaatcgataagcccaagcccaaaaggcatctgtacctgagcccattattctttcattactagcaaaaaggatgcattagagaccccggtgtagtaaattgacctcacaattcactattgtattgtatacgtacatttcaagcgtaattaaaccctcatatttttatacgctttaaatataattggcctttaattagctcaaataaactagatgtcgtacgtgatcacggtggatgaaatcaatggtattatgaaaagactgtacatgatttcaaatattttaatgtggtcgtaaaaattgttgtttatagtggaaattgaagacaacaacgttactgaaacacatacagattgaaatttcgatcatttacttgcaaagtgttaccgtggaggcgtggcgtggacgtaaggtaccataatggtttgtgttacagtcacgccactacactcgaattcaagctaccatattataatacgttgttgattagaaaaaatagtcgccaattttctttaaaacaaatttcagtttttatttgtcagcaaaaaaaacttactaacacaacggaagaacacaaaaattagggagttgctcacagagcaaaagtaatagaaatgggaaaagctaatatacgtccgagtaggaaactaatcttgcaaaaactgatgaaagcaatcagaagccttgacgtttgtctggagagaggaattgtgttttggatcactttgttcagtttgttgtggatcgtcttccgttacgttctcaccaaaaatatttcataatgaaacaaaaaaattaattaataatggtagcttagaatgccaagttgagaacagatttgcagtttgtcccggaatgatcaagtagagcattcatagtgtcttgccaatatggtgtgatcaacgaagtttgacaaaaccgtgaagatataggaacatgtaatcatgcggctctccatacaatacatcttgttgacaaagttcccaagacctcattctacaaaccaatgtttcttttttctttttctttttggtgatagtttttgcaatcaaatgttgtaaaactatgattggaaatactactgtattttaccgaaaactttattatatatagtcattaacactcattaccaatcacataatcaatagtctattttgattatacaacttttaaacaataaagacatgtttatacagatttggtttaaattagtactccctatattttagaaaattttattttgtttcatattatagaatgtcttggaaagttctatgtaaatttaaatgtatttagtaacttgtgacgattttatattatgtagtcttttttaggatttgttgattttttaaaataaattttttaaagaaaaaaaacaaattattttaataaacatgcctttaccttatacagtttatattttgaaagagagatagtatgttttaggatatatttaaagaaaaaaaaataactctttaattta

SEQ ID NO: 72 - DNA, 4100 bp, Artificial sequence; identical to SEQ ID NO: 31
  Single strand oligonucleotide

SEQ ID NO: 73 - DNA, 4100 bp, Artificial sequence; identical to SEQ ID NO: 32
  Single strand oligonucleotide

SEQ ID NO: 74 - DNA, 4100 bp, Artificial sequence; identical to SEQ ID NO: 33
  Single strand oligonucleotide

SEQ ID NO: 75 - DNA, 4100 bp, Artificial sequence; identical to SEQ ID NO: 34
  Single strand oligonucleotide

SEQ ID NO: 76 - DNA, 4100 bp, Artificial sequence
  Single strand oligonucleotide
cacttatcatttagacagtagattttaaatttgtatttacaatttcaaaactgaaattcatttgtaatcaaagaaaaacaaaacaagaaaagggaggaggagtgggatttgggttgcttaacagtattatatatacacgtcgttagttaatcaataaattatgagcaggtgtagtagctatgaacatggttttaccaaattggtaaattcatgtcattgttgtagcactttagcgaggccagcaaaatggcgttcttggaaagggcatggcggcccgtggccgccagggatatgtgtgcagctagaaggattagaaggagtaacttcacctttttgtagaaactgtaaattgccaagacgctcgtttggtaaataccttaacgcttcgtttgctggaatgtgtaccaccattagtagaagaaagtataataagactattaatgcaagagattttttcatattccttttctaagagtagaatggaatgaataaatgaatgaatgaaatagggtttttcttgtttagatcctgtcgcacccgagaataatagaagctgaattaattggtgaagagttttatggtggcgatgttgtatttatagagggaaatgatttcaagtttacaatgggatttttaatttgttttgttgactattatcttgcggagagatcttgactgttgacatgtatgtagtgtttgttattaaaataaatgcatttttgtagacccgattcttaaatatgttaggcatggtcaaattgttagactgtaaaagcttgagtagagacatcggtcaactttgtttacaagaattctctataaaatattatacaaattgatcggtagaaattagatggaacattttgaattaatgtttgacaatgtataaattggtttggtcaatatctaggaatgaaaacaagagctgcttcaaagttgttccattcttaagtatacatagaggtggcttgatgggaagtttcatggaagtgtagttttatatctacttccaaattcgttgatctgtttcttatctcaagctaaacatgtttagaaaagatgtgttaaaaacatgtgacaaaaaaagagtcaaatgtttggcaaacaaggtacttagatttttggcatctattcaaatataatagaatcccaaaattatgatatttgtcaatcaaatttgaaaaaaaaaaaaaaaaaaaaaaagattctacaaaagatcaaacgtattgccgtagatttatcataattttaattctttcacactaccactagtccactaccatatagtgatgagataatccataatcataaataagatataactttcgaattcttgtttttgttgcctcaaagttgttggatcattattttttacgtaaatgtggcttaatgagaatttatgtttgtgggaattgtagtttgcttccaactttttttttttttttttgaacacgtagtttgcttccaacttagtttatctttttcttatttcaagttaaacatgtaaaaaaacatgtgacgacgaaattcaatcagttcctccaatgtttggcagaagccaaatctttggtaaacaaagtaatttttttgccatttgattggttagtataggagaatttaaaaacgacgataaggtttaggtaaattatttcatttgaaaataattgagcaccgttaataattttcatccataaaataatatttcaaagatgatatttgatccccattaaattcattcgtaaccaaaaaaaagttatgaaaaaagagtggtcgtgtgagttgcccaagcaccattataataaaaaataaaataattagcaagtaataaggaataaaatcctgtaattatagctgaaaaaggaaaaatatttggagaccgtcagattcgaatctgaacaaagcataaaaaagtcaacaaaacttaaagcggcggtctcatcgtaatctcagcccaataccctattttcctctcccctatataaatactttcttcttctactgatcttcttctcacaaataaacccaaatatatcaatctactgtgttggtgattaagtactttaaagatcggcaacacatgatagtggtcaaaaaagttgtagttttcttaaagtctctttcctctgatcagtgttggcgatctttaagagcttgctccctaaacttatctctctgatgatttaatgttagagatcttcgtaaatctatgtgtttgatagatctgatgcgttttttgagttgatgatttgattatttttcactggaaagtatctcattagggtaacgataatgttttatggatttggttgtataacagatccatgaaatcttgactggttataaaatctgaataatgtatttcaatttggagattcggtgataaaaattactgatttacgaatgacatttatatcgatagatgagtttgctgatttggttgttaaattgataaatcaaggacatgagaaactgtttttgtatgctaatttgtccatggaataaaattgggaggtgaggaccgtgagggtagtcaggaaaccttaatattgaagttgatgttgaaccaacaaatctgcccaaaaatgataaaagttgatgccgagcccacaaattttgatgacaatcgataagcccaagcccaaaaggcatctgtacctgagcccattattctttcattactagcaaaaaggatgcattagagaccccggtgtagtaaattgacctcacaattcactattgtattgtatacgtacatttcaagcgtaattaaaccctcatatttttatacgctttaaatataattggcctttaattagctcaaataaactagatgtcgtacgtgatcacggtggatgaaatcaatggtattatgaaaagactgtacatgatttcaaatattttaatgtggtcgtaaaaattgttgtttatagtggaaattgaagacaacaacgttactgaaacacatacagattgaaatttcgatcatttacttgcaaagtgttaccgtggaggcgtggcgtggacgtaaggtaccataatggtttgtgttacagtcacgccactacactcgaattcaagctaccatattataatacgttgttgattagaaaaaatagtcgccaattttctttaaaacaaatttcagtttttatttgtcagcaaaaaaaacttactaacacaacggaagaacacaaaaattagggagttgctcacagagcaaaagtaatagaaatgggaaaagctaatatacgtccgagtaggaaactaatcttgcaaaaactgatgaaagcaatcagaagccttgacgtttgtctggagagaggaattgtgttttggatcactttgttcagtttgttgtggatcgtcttccgttacgttctcaccaaaaatatttcataatgaaacaaaaaaattaattaataatggtagcttagaatgccaagttgagaacagatttgcagtttgtcccggaatgatcaagtagagcattcatagtgtcttgccaatatggtgtgatcaacgaagtttgacaaaaccgtgaagatataggaacatgtaatcatgcggctctccatacaatacatcttgttgacaaagttcccaagacctcattctacaaaccaatgtttcttttttctttttctttttggtgatagtttttgcaatcaaatgttgtaaaactatgattggaaatactactgtattttaccgaaaactttattatatatagtcattaacactcattaccaatcacataatcaatagtctattttgattatacaacttttaaacaataaagacatgtttatacagatttggtttaaattagtactccctatattttagaaaattttattttgtttcatattatagaatgtcttggaaagttctatgtaaatttaaatgtatttagtaacttgtgacgattttatattatgtagtcttttttaggatttgttgattttttaaaataaattttttaaagaaaaaaaacaaattattttaataaacatgcctttaccttatacagtttatattttgaaagagagatagtatgttttaggatatatttaaagaaaaaaaaataactctttaattta

SEQ ID NO: 77 - DNA, 4100 bp, Artificial sequence
  Single strand oligonucleotide
cacttatcatttagacagtagattttaaatttgtatttacaatttcaaaactgaaattcatttgtaatcaaagaaaaacaaaacaagaaaagggaggaggagtgggatttgggttgcttaacagtattatatatacacgtcgttagttaatcaataaattatgagcaggtgtagtagctatgaacatggttttaccaaattggtaaattcatgtcattgttgtagcactttagcgaggccagcaaaatggcgttcttggaaagggcatggcggcccgtggccgccagggatatgtgtgcagctagaaggattagaaggagtaacttcacctttttgtagaaactgtaaattgccaagacgctcgtttggtaaataccttaacgcttcgtttgctggaatgtgtaccaccattagtagaagaaagtataataagactattaatgcaagagattttttcatattccttttctaagagtagaatggaatgaataaatgaatgaatgaaatagggtttttcttgtttagatcctgtcgcacccgagaataatagaagctgaattaattggtgaagagttttatggtggcgatgttgtatttatagagggaaatgatttcaagtttacaatgggatttttaatttgttttgttgactattatcttgcggagagatcttgactgttgacatgtatgtagtgtttgttattaaaataaatgcatttttgtagacccgattcttaaatatgttaggcatggtcaaattgttagactgtaaaagcttgagtagagacatcggtcaactttgtttacaagaattctctataaaatattatacaaattgatcggtagaaattagatggaacattttgaattaatgtttgacaatgtataaattggtttggtcaatatctaggaatgaaaacaagagctgcttcaaagttgttccattcttaagtatacatagaggtggcttgatgggaagtttcatggaagtgtagttttatatctacttccaaattcgttgatctgtttcttatctcaagctaaacatgtttagaaaagatgtgttaaaaacatgtgacaaaaaaagagtcaaatgtttggcaaacaaggtacttagatttttggcatctattcaaatataatagaatcccaaaattatgatatttgtcaatcaaatttgaaaaaaaaaaaaaaaaaaaaaaagattctacaaaagatcaaacgtattgccgtagatttatcataattttaattctttcacactaccactagtccactaccatatagtgatgagataatccataatcataaataagatataactttcgaattcttgtttttgttgcctcaaagttgttggatcattattttttacgtaaatgtggcttaatgagaatttatgtttgtgggaattgtagtttgcttccaactttttttttttttttttgaacacgtagtttgcttccaacttagtttatctttttcttatttcaagttaaacatgtaaaaaaacatgtgacgacgaaattcaatcagttcctccaatgtttggcagaagccaaatctttggtaaacaaagtaatttttttgccatttgattggttagtataggagaatttaaaaacgacgataaggtttaggtaaattatttcatttgaaaataattgagcaccgttaataattttcatccataaaataatatttcaaagatgatatttgatccccattaaattcattcgtaaccaaaaaaaagttatgaaaaaagagtggtcgtgtgagttgcccaagcaccattataataaaaaataaaataattagcaagtaataaggaataaaatcctgtaattatagctgaaaaaggaaaaatatttggagaccgtcagattcgaatctgaacaaagcataaaaaagtcaacaaaacttaaagcggcggtctcatcgtaatctcagcccaataccctattttcctctcccctatataaatactttcttcttctactgatcttcttctcacaaataaacccaaatatatcaatctactgtgttggtgattaagtactttgacctttcttgggtttagccagtggtcaaaaaagttgtagttttcttaaagtctctttcctctgggctaacccatgaaaggtcaagagcttgctccctaaacttatctctctgatgatttaatgttagagatcttcgtaaatctatgtgtttgatagatctgatgcgttttttgagttgatgatttgattatttttcactggaaagtatctcattagggtaacgataatgttttatggatttggttgtataacagatccatgaaatcttgactggttataaaatctgaataatgtatttcaatttggagattcggtgataaaaattactgatttacgaatgacatttatatcgatagatgagtttgctgatttggttgttaaattgataaatcaaggacatgagaaactgtttttgtatgctaatttgtccatggaataaaattgggaggtgaggaccgtgagggtagtcaggaaaccttaatattgaagttgatgttgaaccaacaaatctgcccaaaaatgataaaagttgatgccgagcccacaaattttgatgacaatcgataagcccaagcccaaaaggcatctgtacctgagcccattattctttcattactagcaaaaaggatgcattagagaccccggtgtagtaaattgacctcacaattcactattgtattgtatacgtacatttcaagcgtaattaaaccctcatatttttatacgctttaaatataattggcctttaattagctcaaataaactagatgtcgtacgtgatcacggtggatgaaatcaatggtattatgaaaagactgtacatgatttcaaatattttaatgtggtcgtaaaaattgttgtttatagtggaaattgaagacaacaacgttactgaaacacatacagattgaaatttcgatcatttacttgcaaagtgttaccgtggaggcgtggcgtggacgtaaggtaccataatggtttgtgttacagtcacgccactacactcgaattcaagctaccatattataatacgttgttgattagaaaaaatagtcgccaattttctttaaaacaaatttcagtttttatttgtcagcaaaaaaaacttactaacacaacggaagaacacaaaaattagggagttgctcacagagcaaaagtaatagaaatgggaaaagctaatatacgtccgagtaggaaactaatcttgcaaaaactgatgaaagcaatcagaagccttgacgtttgtctggagagaggaattgtgttttggatcactttgttcagtttgttgtggatcgtcttccgttacgttctcaccaaaaatatttcataatgaaacaaaaaaattaattaataatggtagcttagaatgccaagttgagaacagatttgcagtttgtcccggaatgatcaagtagagcattcatagtgtcttgccaatatggtgtgatcaacgaagtttgacaaaaccgtgaagatataggaacatgtaatcatgcggctctccatacaatacatcttgttgacaaagttcccaagacctcattctacaaaccaatgtttcttttttctttttctttttggtgatagtttttgcaatcaaatgttgtaaaactatgattggaaatactactgtattttaccgaaaactttattatatatagtcattaacactcattaccaatcacataatcaatagtctattttgattatacaacttttaaacaataaagacatgtttatacagatttggtttaaattagtactccctatattttagaaaattttattttgtttcatattatagaatgtcttggaaagttctatgtaaatttaaatgtatttagtaacttgtgacgattttatattatgtagtcttttttaggatttgttgattttttaaaataaattttttaaagaaaaaaaacaaattattttaataaacatgcctttaccttatacagtttatattttgaaagagagatagtatgttttaggatatatttaaagaaaaaaaaataactctttaattta

SEQ ID NO: 78 - DNA, 4000 bp, Artificial sequence
  Single strand oligonucleotide
accctcattgattttggtggccaaactcttgatcgtattcttttaggaacagtaattaattttaaatttgagaaaaatgtagtgatgaaagtgagatatatgggacgcactattgaaagcattgtccacaccgcatgatgtgagattgatgtgaatatggtaactaataacacccagactcacttttatgagaaaatgtatcttaaaaaatgttattcatcaaagcttagatgcgctataggggaacataatcattatttgaaaagaaccaattcaaatatttttttttttaagagttaaaatcctatataacataaccatccaaactttgggcatgaacacaacaatattttttttcgtttttgataaattctttcaattgcaatcaaaacttaccagctatacaaatgtttgctgcatccaatctaatacaccgttaaacaataaaatttgttatctctcaaatctgatcatctattccaacctgactgttttattctagtattttaaggccaggtataacgaaaacaaagaaaaaagttcagcgaccaagacattttgacatcaggctcaaacggtcaaacccacgaaaacttttacctcatttcttaaccacgcagtgttatttgaatagccttaataggctaatacaaaacaacaagccatcgattacagttttaactataatattacaaaatcttaaaccaaaacaagaaaagatatatattccgtaaaattaaaataatatttttaatatagtcattatgtaagttagctctttcgacaaaatcattataaattaggccattttgtaagttagttcttttatcgacaagccattataacttaggtaattttgtaagttagctggactataaccaatttttttgtttcacatctagagtataaaacacatatatattgaccgtacaactttagtcaaattagaaactctgttttatctgcagaaaagaaaaaaaaagaggatgaattatgtaaatacttcaggattagaaataatgtcatcgtatatctcttgatatgaatacatattttacttgactagtaccgtagtcggcaggaaaatgacacaaacaaccatctaaaaagataaagtaagaactaaaaagtcttgacattcattagtttaatcattttctgttaacatatatggaaaaaacaaacttcaccgttatttacctgaatttacctatttgggtaagaattgtacctctggacctctagtattttatatacacctaaaaatataattttggtcgggaaaatataactctgtttaattaattaaattttcagtattgtgtaagtgtaattatagaaatcaattttatccgcgtaacaaaataatataaaattatactttcaaatccacgaatatatattgtgaagtctcatagtttgcaaataagcattggtcttcggccgacaaaaaaaaaagcattggtcttcgaatattttgaatatcggaccaatggtatataattaataatatgtggtatataaatacatatttatttaaatcacaataggatatgcaatgtgtgtatatatacatatacgtaattaaagtccgggttaaactgatagcatatattataatagatgcatctataattgttcgtcaacaaaagcattatcatgtattttgaattaagcttccttcatttctgtgaatcaaaaggcctcagaagaagaaactaaagtcaaacaatcaacgggatccaataaatcacatctggactatatagtatcaatactttccacactaaaaaagctaagaaatttaataaatacattattataggggggaaaaaaaggtagtcatcagatatatattttggtaagaaaatatagaaatgaataatttcacgtttaacgaagaggagatgacgtgtgttccttcgaacccgagttttgttcgtctataaatagcaccttctcttctccttcttcctcacttccatctttttagcttcactatctctctataatcggttttatctttctctaagtcacaacccaaaaaaacaaagtagagaagaatctgtaaagctcaggagggatagcgccatgatgatcacattcgttatctattttttggcgctatccatcctgagtttcattggctcttcttactacaatgaaaaaggccgaggcaaaacgcctaaaatcacttgagaatcaattctttttactgtccatttaagctatcttttataaacgtgtcttattttctatctcttttgtttaaactaagaaactatagtattttgtctaaaacaaaacatgaaagaacagattagatctcatctttagtctctttctccggtgcagtcagccaccgtcgggtaagtttcatctgtattttattaattaattacaattattagtgttcttattaccgttttggtaaaattagttaattaatgtcggtccaaacattctaaaccaattattctgaaaagggtgaacgccaatcagttatatacaatattcttacattaaagtagaatcggagatgttacatactaaccaaaagttacatatactagtatcattttctttaagatttgtttaggatttactcactttatagtgctcgcggttggggtcagggtaagtggggaacagatatgctctgcatgaaccacgtggaccaacatgcatatacacagttacatttattttttctagtaggttcatttgcaaattttccagtatcttgtatgttatcttcatggtgagttttttggtcgcatattcttggtgattcttcttctacgttttcactttcttcttcagagaccttattaatatgttaattgcatgaatttatgtaacattcaagaaaaagagatcgaatacaagaaaccggaaatttaatttctaatttgaattctatgcatgtttgtttctttgccaatttagtacgaatatatttatggtccggagttctaaccaaagatagttgctctgtatatagaagttatacatctcgcttgtttaaactaaataactatttagtttgtcttggtagtccagtgactttctgcaaacattgggatttataatatagtcaaaacgttgggatatgtagtattcattttcgttgtaaaaatcattatattttgcaaaggttgcaacgtaaaacgttgtattgaatttaggagaaagtagccatttacaatgaattttagtgacaaactgttgtatacagcctgtgccactaagtatgtctatatctaaatttggaatggatgataaccagtattggtcaataatggataatttggtatttagaattactaatttggtattttagtgacaaactgttgtatggaatttaggagaacgcgttcccaagctatatattatatgtatttcattctttcatatgttatattatgaattgttataaaaaagaccaatgagcaacggtttaaggtttaatcagtaatcgatccgaccaatcatatacaagttcctaacacatcttctaactactgagtaaaatagtaatgctattacaaaggttttttcttttcaaaatacagcctaatgctactacaaaattctaatgttataaaataatcataggagaagtaaaccccggtatttaattaataccttacaaacttacattattgataaagttgaatgaagagttatatggtccatttagtattatttacttaatatgatactagtgttagacgtgttactgtatttcaacgtgcataatcaggttgttcaaaaagagagaggataggtcttcttcttctgtaatttgctgggaccgcaagtcatgtgaggctgctctgctgatgctgcacggcgtcgcaactctctcaataaattcttttaactaacgctccaattttcgatgtaaattggctgacttcaattctatgccttactcttgtactctatgtttctttatctattaaaatccaactctgcttttgaacccaaaaaacaa

SEQ ID NO: 79 - DNA, 4000 bp, Artificial sequence; identical to SEQ ID NO: 35
  Single strand oligonucleotide

SEQ ID NO: 80 - DNA, 4000 bp, Artificial sequence; identical to SEQ ID NO: 36
  Single strand oligonucleotide

SEQ ID NO: 81 - DNA, 4000 bp, Artificial sequence; identical to SEQ ID NO: 37
  Single strand oligonucleotide

SEQ ID NO: 82 - DNA, 4000 bp, Artificial sequence; identical to SEQ ID NO: 38
  Single strand oligonucleotide

SEQ ID NO: 83 - DNA, 4000 bp, Artificial sequence
  Single strand oligonucleotide
accctcattgattttggtggccaaactcttgatcgtattcttttaggaacagtaattaattttaaatttgagaaaaatgtagtgatgaaagtgagatatatgggacgcactattgaaagcattgtccacaccgcatgatgtgagattgatgtgaatatggtaactaataacacccagactcacttttatgagaaaatgtatcttaaaaaatgttattcatcaaagcttagatgcgctataggggaacataatcattatttgaaaagaaccaattcaaatatttttttttttaagagttaaaatcctatataacataaccatccaaactttgggcatgaacacaacaatattttttttcgtttttgataaattctttcaattgcaatcaaaacttaccagctatacaaatgtttgctgcatccaatctaatacaccgttaaacaataaaatttgttatctctcaaatctgatcatctattccaacctgactgttttattctagtattttaaggccaggtataacgaaaacaaagaaaaaagttcagcgaccaagacattttgacatcaggctcaaacggtcaaacccacgaaaacttttacctcatttcttaaccacgcagtgttatttgaatagccttaataggctaatacaaaacaacaagccatcgattacagttttaactataatattacaaaatcttaaaccaaaacaagaaaagatatatattccgtaaaattaaaataatatttttaatatagtcattatgtaagttagctctttcgacaaaatcattataaattaggccattttgtaagttagttcttttatcgacaagccattataacttaggtaattttgtaagttagctggactataaccaatttttttgtttcacatctagagtataaaacacatatatattgaccgtacaactttagtcaaattagaaactctgttttatctgcagaaaagaaaaaaaaagaggatgaattatgtaaatacttcaggattagaaataatgtcatcgtatatctcttgatatgaatacatattttacttgactagtaccgtagtcggcaggaaaatgacacaaacaaccatctaaaaagataaagtaagaactaaaaagtcttgacattcattagtttaatcattttctgttaacatatatggaaaaaacaaacttcaccgttatttacctgaatttacctatttgggtaagaattgtacctctggacctctagtattttatatacacctaaaaatataattttggtcgggaaaatataactctgtttaattaattaaattttcagtattgtgtaagtgtaattatagaaatcaattttatccgcgtaacaaaataatataaaattatactttcaaatccacgaatatatattgtgaagtctcatagtttgcaaataagcattggtcttcggccgacaaaaaaaaaagcattggtcttcgaatattttgaatatcggaccaatggtatataattaataatatgtggtatataaatacatatttatttaaatcacaataggatatgcaatgtgtgtatatatacatatacgtaattaaagtccgggttaaactgatagcatatattataatagatgcatctataattgttcgtcaacaaaagcattatcatgtattttgaattaagcttccttcatttctgtgaatcaaaaggcctcagaagaagaaactaaagtcaaacaatcaacgggatccaataaatcacatctggactatatagtatcaatactttccacactaaaaaagctaagaaatttaataaatacattattataggggggaaaaaaaggtagtcatcagatatatattttggtaagaaaatatagaaatgaataatttcacgtttaacgaagaggagatgacgtgtgttccttcgaacccgagttttgttcgtctataaatagcaccttctcttctccttcttcctcacttccatctttttagcttcactatctctctataatcggttttatctttctctaagtcacaacccaaaaaaacaaagtagagaagaatctgtataaagatcggcaacacatgatatgatgatcacattcgttatctattttttatcatgtgttaccgatctttacattggctcttcttactacaatgaaaaaggccgaggcaaaacgcctaaaatcacttgagaatcaattctttttactgtccatttaagctatcttttataaacgtgtcttattttctatctcttttgtttaaactaagaaactatagtattttgtctaaaacaaaacatgaaagaacagattagatctcatctttagtctctttctccggtgcagtcagccaccgtcgggtaagtttcatctgtattttattaattaattacaattattagtgttcttattaccgttttggtaaaattagttaattaatgtcggtccaaacattctaaaccaattattctgaaaagggtgaacgccaatcagttatatacaatattcttacattaaagtagaatcggagatgttacatactaaccaaaagttacatatactagtatcattttctttaagatttgtttaggatttactcactttatagtgctcgcggttggggtcagggtaagtggggaacagatatgctctgcatgaaccacgtggaccaacatgcatatacacagttacatttattttttctagtaggttcatttgcaaattttccagtatcttgtatgttatcttcatggtgagttttttggtcgcatattcttggtgattcttcttctacgttttcactttcttcttcagagaccttattaatatgttaattgcatgaatttatgtaacattcaagaaaaagagatcgaatacaagaaaccggaaatttaatttctaatttgaattctatgcatgtttgtttctttgccaatttagtacgaatatatttatggtccggagttctaaccaaagatagttgctctgtatatagaagttatacatctcgcttgtttaaactaaataactatttagtttgtcttggtagtccagtgactttctgcaaacattgggatttataatatagtcaaaacgttgggatatgtagtattcattttcgttgtaaaaatcattatattttgcaaaggttgcaacgtaaaacgttgtattgaatttaggagaaagtagccatttacaatgaattttagtgacaaactgttgtatacagcctgtgccactaagtatgtctatatctaaatttggaatggatgataaccagtattggtcaataatggataatttggtatttagaattactaatttggtattttagtgacaaactgttgtatggaatttaggagaacgcgttcccaagctatatattatatgtatttcattctttcatatgttatattatgaattgttataaaaaagaccaatgagcaacggtttaaggtttaatcagtaatcgatccgaccaatcatatacaagttcctaacacatcttctaactactgagtaaaatagtaatgctattacaaaggttttttcttttcaaaatacagcctaatgctactacaaaattctaatgttataaaataatcataggagaagtaaaccccggtatttaattaataccttacaaacttacattattgataaagttgaatgaagagttatatggtccatttagtattatttacttaatatgatactagtgttagacgtgttactgtatttcaacgtgcataatcaggttgttcaaaaagagagaggataggtcttcttcttctgtaatttgctgggaccgcaagtcatgtgaggctgctctgctgatgctgcacggcgtcgcaactctctcaataaattcttttaactaacgctccaattttcgatgtaaattggctgacttcaattctatgccttactcttgtactctatgtttctttatctattaaaatccaactctgcttttgaacccaaaaaacaa

SEQ ID NO: 84 - DNA, 4000 bp, Artificial sequence
  Single strand oligonucleotide
accctcattgattttggtggccaaactcttgatcgtattcttttaggaacagtaattaattttaaatttgagaaaaatgtagtgatgaaagtgagatatatgggacgcactattgaaagcattgtccacaccgcatgatgtgagattgatgtgaatatggtaactaataacacccagactcacttttatgagaaaatgtatcttaaaaaatgttattcatcaaagcttagatgcgctataggggaacataatcattatttgaaaagaaccaattcaaatatttttttttttaagagttaaaatcctatataacataaccatccaaactttgggcatgaacacaacaatattttttttcgtttttgataaattctttcaattgcaatcaaaacttaccagctatacaaatgtttgctgcatccaatctaatacaccgttaaacaataaaatttgttatctctcaaatctgatcatctattccaacctgactgttttattctagtattttaaggccaggtataacgaaaacaaagaaaaaagttcagcgaccaagacattttgacatcaggctcaaacggtcaaacccacgaaaacttttacctcatttcttaaccacgcagtgttatttgaatagccttaataggctaatacaaaacaacaagccatcgattacagttttaactataatattacaaaatcttaaaccaaaacaagaaaagatatatattccgtaaaattaaaataatatttttaatatagtcattatgtaagttagctctttcgacaaaatcattataaattaggccattttgtaagttagttcttttatcgacaagccattataacttaggtaattttgtaagttagctggactataaccaatttttttgtttcacatctagagtataaaacacatatatattgaccgtacaactttagtcaaattagaaactctgttttatctgcagaaaagaaaaaaaaagaggatgaattatgtaaatacttcaggattagaaataatgtcatcgtatatctcttgatatgaatacatattttacttgactagtaccgtagtcggcaggaaaatgacacaaacaaccatctaaaaagataaagtaagaactaaaaagtcttgacattcattagtttaatcattttctgttaacatatatggaaaaaacaaacttcaccgttatttacctgaatttacctatttgggtaagaattgtacctctggacctctagtattttatatacacctaaaaatataattttggtcgggaaaatataactctgtttaattaattaaattttcagtattgtgtaagtgtaattatagaaatcaattttatccgcgtaacaaaataatataaaattatactttcaaatccacgaatatatattgtgaagtctcatagtttgcaaataagcattggtcttcggccgacaaaaaaaaaagcattggtcttcgaatattttgaatatcggaccaatggtatataattaataatatgtggtatataaatacatatttatttaaatcacaataggatatgcaatgtgtgtatatatacatatacgtaattaaagtccgggttaaactgatagcatatattataatagatgcatctataattgttcgtcaacaaaagcattatcatgtattttgaattaagcttccttcatttctgtgaatcaaaaggcctcagaagaagaaactaaagtcaaacaatcaacgggatccaataaatcacatctggactatatagtatcaatactttccacactaaaaaagctaagaaatttaataaatacattattataggggggaaaaaaaggtagtcatcagatatatattttggtaagaaaatatagaaatgaataatttcacgtttaacgaagaggagatgacgtgtgttccttcgaacccgagttttgttcgtctataaatagcaccttctcttctccttcttcctcacttccatctttttagcttcactatctctctataatcggttttatctttctctaagtcacaacccaaaaaaacaaagtagagaagaatctgtatgacctttcttgggtttagccatgatgatcacattcgttatctattttttggctaaaccccagaaaggtcacattggctcttcttactacaatgaaaaaggccgaggcaaaacgcctaaaatcacttgagaatcaattctttttactgtccatttaagctatcttttataaacgtgtcttattttctatctcttttgtttaaactaagaaactatagtattttgtctaaaacaaaacatgaaagaacagattagatctcatctttagtctctttctccggtgcagtcagccaccgtcgggtaagtttcatctgtattttattaattaattacaattattagtgttcttattaccgttttggtaaaattagttaattaatgtcggtccaaacattctaaaccaattattctgaaaagggtgaacgccaatcagttatatacaatattcttacattaaagtagaatcggagatgttacatactaaccaaaagttacatatactagtatcattttctttaagatttgtttaggatttactcactttatagtgctcgcggttggggtcagggtaagtggggaacagatatgctctgcatgaaccacgtggaccaacatgcatatacacagttacatttattttttctagtaggttcatttgcaaattttccagtatcttgtatgttatcttcatggtgagttttttggtcgcatattcttggtgattcttcttctacgttttcactttcttcttcagagaccttattaatatgttaattgcatgaatttatgtaacattcaagaaaaagagatcgaatacaagaaaccggaaatttaatttctaatttgaattctatgcatgtttgtttctttgccaatttagtacgaatatatttatggtccggagttctaaccaaagatagttgctctgtatatagaagttatacatctcgcttgtttaaactaaataactatttagtttgtcttggtagtccagtgactttctgcaaacattgggatttataatatagtcaaaacgttgggatatgtagtattcattttcgttgtaaaaatcattatattttgcaaaggttgcaacgtaaaacgttgtattgaatttaggagaaagtagccatttacaatgaattttagtgacaaactgttgtatacagcctgtgccactaagtatgtctatatctaaatttggaatggatgataaccagtattggtcaataatggataatttggtatttagaattactaatttggtattttagtgacaaactgttgtatggaatttaggagaacgcgttcccaagctatatattatatgtatttcattctttcatatgttatattatgaattgttataaaaaagaccaatgagcaacggtttaaggtttaatcagtaatcgatccgaccaatcatatacaagttcctaacacatcttctaactactgagtaaaatagtaatgctattacaaaggttttttcttttcaaaatacagcctaatgctactacaaaattctaatgttataaaataatcataggagaagtaaaccccggtatttaattaataccttacaaacttacattattgataaagttgaatgaagagttatatggtccatttagtattatttacttaatatgatactagtgttagacgtgttactgtatttcaacgtgcataatcaggttgttcaaaaagagagaggataggtcttcttcttctgtaatttgctgggaccgcaagtcatgtgaggctgctctgctgatgctgcacggcgtcgcaactctctcaataaattcttttaactaacgctccaattttcgatgtaaattggctgacttcaattctatgccttactcttgtactctatgtttctttatctattaaaatccaactctgcttttgaacccaaaaaacaa

SEQ ID NO: 85 - DNA, 19 bp, Artificial sequence
  Single strand oligonucleotide
acaccctgggaattggttt

SEQ ID NO: 86 - DNA, 20 bp, Artificial sequence
  Single strand oligonucleotide
gtatgcgccaataagaccac

SEQ ID NO: 87 - DNA, 20 bp, Artificial sequence
  Single strand oligonucleotide
gtactgctggtcctttgcag

SEQ ID NO: 88 - DNA, 20 bp, Artificial sequence
  Single strand oligonucleotide
aggagcactacggaaggatg

SEQ ID NO: 89 - DNA, 22 bp, Artificial sequence
  Single strand oligonucleotide
gttgagagtgttggagaaggag

SEQ ID NO: 90 - DNA, 21 bp, Artificial sequence
  Single strand oligonucleotide
ctcggtgttgatcctgagaag

SEQ ID NO: 91 - DNA, 23 bp, Artificial sequence
  Single strand oligonucleotide
agcttccttcatttctgtgaatc

SEQ ID NO: 92 - DNA, 21 bp, Artificial sequence
  Single strand oligonucleotide
ctgttccccacttaccctgac

SEQ ID NO: 93 - DNA, 21 bp, Artificial sequence
  Single strand oligonucleotide
ctcctcatctgattccttctc

SEQ ID NO: 94 - DNA, 21 bp, Artificial sequence
  Single strand oligonucleotide
ctgttccccacttaccctgac

SEQ ID NO: 95 - DNA, 23 bp, Artificial sequence
  Single strand oligonucleotide
gtgtgtggaaagtttatcaacac

SEQ ID NO: 96 - DNA, 27 bp, Artificial sequence
  Single strand oligonucleotide
gttagtatgtaacatctccgattctac

SEQ ID NO: 97 - DNA, 20 bp, Artificial sequence
  Single strand oligonucleotide
agagtggtcgtgtgagttgc

SEQ ID NO: 98 - DNA, 25 bp, Artificial sequence
  Single strand oligonucleotide
ccagtcaagatttcatggatctgtt

SEQ ID NO: 99 - DNA, 28 bp, Artificial sequence
  Single strand oligonucleotide
ctaacataatcgagaacagatggaagac

SEQ ID NO: 100 - DNA, 32 bp, Artificial sequence
  Single strand oligonucleotide
ttctcatgtccttgatttatcaatttaacaac

SEQ ID NO: 101 - DNA, 20 bp, Artificial sequence
  Single strand oligonucleotide
agagtggtcgtgtgagttgc

SEQ ID NO: 102 - DNA, 26 bp, Artificial sequence
  Single strand oligonucleotide
cgcatcagatctatcaaacacataga

SEQ ID NO: 103 - DNA, 277 bp, Artificial sequence
  Single strand oligonucleotide
gcuacucuggugaaccaucguuggccaugcuugccuuauucucccauggcaaucuuacuacggccguaggaaacuucuccggacaagcgaauaggcuucacagacucuacgaaaaccccuaaaacaaacacuaacaaagggacugaagagccuaccaccacccaaugcgucgauuacugacgcacguacguggucagcgaaggcgcugagcucgugguauuggcagcggugaacagaauaaucaaacaagccaacggugguaucauccagaacaucu

SEQ ID NO: 104 - DNA, 110 bp, Artificial sequence
  Single strand oligonucleotide
cgcaaagaaagaggaggaggaugaugaguaaacaaaugcacucugcauguucgaugcacaugcaucucuugcuugcucauugauccaucuuucuugcuccggcaccgagu

SEQ ID NO: 105 - DNA, 277 bp, Artificial sequence
  Single strand oligonucleotide
gaaucuguucucaucuuuuccuuagggguguuuaccuguucugccacguuaucucuucuuuccuugauuccgacggaaccaaauaauaguggccaggacagacagacaacgaaaacccaaaaaacaaacacgaacaauguuagucaauucuggcguccaacauaacgcaugcaacacguaugcgcggacguugggaguggaagcauucgccggaaggaaacagcaaaggugaagagaauagagagugcguugaggaggaggaugaugaguaaugacg

SEQ ID NO: 106 - DNA, 277 bp, Artificial sequence
  Single strand oligonucleotide
gaccagguuaugaccccguggguucaagacaugccacuagcagccgagcuaagccugccgucacuaaacaaccuuugucuagagaauacgcuaugcuacaaauaagcgacgaaaacccuacaaacaaucuccaacaacgcucguuaauaguauacugccgcgaauugcgcuaaacacuagcgcaugcaagcggcgagcuuacgagcuccgaugacgguaacgccaaggucgaagugcugguucauauugggauucgugggguucacuaauccgcccu

SEQ ID NO: 107 - DNA, 277 bp, Artificial sequence
  Single strand oligonucleotide
ggcccagguacgauggaguccauucaggacuugcuagcaacgcacgcgaggggcgauuggugugucauugaggcuuagcgacagauaauauauaacauaagacguccuacgaaaaaccuacaaacaaacacuaacaaaggaagucaaguguuaucaaccucaucuagcuucuagaacagaagcucccacgaggugaguguaggcauucgcaauauugauagguaacuggcgaaucguugcuccaaaucaggauggauucuauucgauauuuagagaa

SEQ ID NO: 108 - DNA, 110 bp, Artificial sequence
  Single strand oligonucleotide
cgcaaagaaacucaaagaaaauuuucgauaaacaaaugcacuucgcaugaacgaugcguuugcaucccuugcuuguugaaguauuuaucuuugaggcuccggcaccgauu

SEQ ID NO: 109 - DNA, 208 bp, Artificial sequence
  Single strand oligonucleotide
uuggugggagggcuaggcuggcgguacguuauucugaaaaaauauuacggacgugaugcaagcacauauggauguugcaugacacggccggugcaugugaacaaaaacaaaaccaaggcaaaagagcgagagagagagcaugcauugcaaaucugucguguuuuuuuauggguggcagccacccuggaugcggcauccuucagaccga

SEQ ID NO: 110 - DNA, 277 bp, Artificial sequence
  Single strand oligonucleotide
gcuacgguuauggcccuacggguacgagacgagcugaugucacccgaguuacuccuacauacgcuguauccaacggauccagagacaauaggggucaagauuacgagauagaaaacccagcacacaauauugaacauuuuuuuagaguugauccacaccacaucgugcaguuaacacaauugcaagcacguggugagcgcagacguucgacuguauguaaagacaaagucgaaaugauguuucucaucgguauucgugggguucacuaauccuaucc

SEQ ID NO: 111 - DNA, 277 bp, Artificial sequence
  Single strand oligonucleotide
gcaucuuugcguccgucuuccgugcucgacuugccgguacccgccaugacaaaccuccgagcuauguguagugccuacccauauaacacccaucucuaaacguauucuaagaaaaaccacaaaacaaucgcgaacaagggaggcgacuagagauccaccucaucgagcuuugacuacuaaagcugcuacggggucggguaagggcccgaggaguuuggaaaguaaguggugaaggggugcuacagauuuguauggaagaugagacugcaaaaguacc

SEQ ID NO: 112 - DNA, 105 bp, Artificial sequence
  Single strand oligonucleotide
gaagagaagaaucuguaaaguuuagaaaggauaaacaaaccacgaucacacacaucgauauacuuuuguuuguccauucugagcuucacuggcucuucuuacuuc

SEQ ID NO: 113 - DNA, 208 bp, Artificial sequence
  Single strand oligonucleotide
ucggucggguaguuacgcuggcaucgauugauggauaguaauaauaaagucagucuugcgagcacagauggauguaucaucacaccaccuguggaugacuacaaaaagaaaaccaaggcaaaagagcgagagagagagcccgcagggcaacgguuucguuguuacuauaccguugcagccaccguaaaaccucccucugccgaaccga

SEQ ID NO: 114 - DNA, 277 bp, Artificial sequence
  Single strand oligonucleotide
gagucgguuauggcccugugaauucaggucaugcgucccucugccuagugaagccaccccucgcuggggaugucguccacagagaacagaacggucugcagacgcacuacgaaaaccauugaaacuagcccaaacaaagugggucaccagauugccagcucgcggugcucacagaacgugagcaggaaaggguugaggccauggucucguccgagggguaagccacaguggaaaagagggaacauaaugggauucgugggguucacuaauccuugca

SEQ ID NO: 115 - DNA, 341 bp, Artificial sequence
  Single strand oligonucleotide
aacgagaugccaacuucucaagauugcaaaagcaaccagcuaguacguugguacacaccaaugggauaaccggucagcaauuagauccuguuaccaucaacaggauccgagggcucauccccgaugaggaaucggaucggccaucagaucucgagcaagaaccaagaggucugccgguauaucuccuuagaauccaaacacgaccaggguuggacccguuccuuccucgcccccaaaaaguaagggcggaggaaugaguuccugguuguuucagggagagaaucagcaucaucggcguugauugguaccggcuuugcagcuggagggguuggcaacucgcc

SEQ ID NO: 116 - DNA, 103 bp, Artificial sequence
  Single strand oligonucleotide
agagagagcuacaggccggcgcuggagagcauacgcagguaauuuuauuagaaaauaacuuugcaggugcgugcucucuaagcgucggccugcgccaucuugg

SEQ ID NO: 117 - DNA, 341 bp, Artificial sequence
  Single strand oligonucleotide
ugggggaggguccaggcaucagggaugaaaagcaagcagcuacccuguugagacaguucgacaauacuacccuaaagcagugugauugaauuacugagaauuugauccuuggacucguugcaagcgagcaaaaguuggggauguaacuucgcgaggaagcaggaagcggagucauggguuaucgccagauaaaccaagcacuucgucagccccagggugaccuauguggcccccgaaaauuaagggccuaggucacguugugacggaguuuacugguggguuugaugagcucaguaugucaagggacccaugguucgugauagugucuggaccuaccccgu

SEQ ID NO: 118 - DNA, 341 bp, Artificial sequence
  Single strand oligonucleotide
agagugauuuauucgugggguucacuaauccguaagcaacgcugaugccaucauaggaugguaaugaagccggauagauacaaguugcuauuuccaauaauagcaaccauggaggcugcgcagcagcucaaaugguucggggucagaucaucgggcaaugacgaagaugaucauagggguagcgcgugagaagccaaccacgcucugcgaucgagccuuaacucgagcgcccacaaaaaggaaggguggaguuaagccuuguagagcguuuccgcgcgugguaguacagccgcgcaguauuacgacuccugugguuaguaaguccgcgaguaagacacugg

SEQ ID NO: 119 - DNA, 239 bp, Artificial sequence
  Single strand oligonucleotide
gcggaggucaaguucuccucauuauaaacaugaaggugucucucguccuaacacacagcgaucaacaaaaaguaacuaacccacacauaugguagaaaccaaaaccauaacguggauacccuuauucugcguauaaguuugacaaaauucgggggaaggaaccauguuuguauugggcggagcaagcgcguggcuccuagagcacgucggccacaaagcacguuggggaccaagaacgg

SEQ ID NO: 120 - DNA, 94 bp, Artificial sequence
  Single strand oligonucleotide
gggaagucuuggauuguggagaauuuaaaaagaaauaacuuucgucacgaacgaaagcaauuauuuuuuaacaccaccacagccuaagauuuuc

SEQ ID NO: 121 - DNA, 225 bp, Artificial sequence
  Single strand oligonucleotide
caacagaagagacacccccgaggagagaaccugcucaucuuuaauguuuuuuuugaaaaccugaccagcgccgcuccugccugcaacaaccauccaucagaacaaaaaguucguauggcgaaaggccauugauggugggcaggucuccccuuggggaagucuagcgucaacgagcuggggucugaugguuucacaauugcuaaaacuugugcuucaggugacaaa

SEQ ID NO: 122 - DNA, 239 bp, Artificial sequence
  Single strand oligonucleotide
ggggagagcauggauucgugguuccuguggauagccccgcacauaaucgcacuucgucccauaaacaaaaacaaaagaaaccacacaaccuguagaaaccaaaacagguggcaccgaucacgacccggugccgccgcucagacaugaguuauguguacacagauucgugggguucacuaauccuaaccacccagcucguagcgggucgggcguaucacuugggaucggcucaagaucgg

SEQ ID NO: 123 - DNA, 341 bp, Artificial sequence
  Single strand oligonucleotide
accgugagauuuuugaggugagcgaggguagucaaacagacgauggucaguaauauuauuggcgcuacgcccuuuauguaccauggugcgggccgggauucguaucaccuggaaucauuucgaaugaugaaaggggagggauuagaacguacgaccaacuagcaaguguguugagggaucaucuccuuuagcuccaaucacuagcacaggauguccuugcucuauucugcccccaaaaauaaagggcauaggguaaagacuguguuagugcuagggagacauucuuaagcgcugcauaggaaucgguccuucuacccucuugaucucaaagaucacacgua

SEQ ID NO: 124 - DNA, 96 bp, Artificial sequence
  Single strand oligonucleotide
gacaacugguuauuggugcggggcguuaagaaaacggugcucaauacuuuuugagcuccgcuuucugaacguucuguauugauaacgagugccacg

SEQ ID NO: 125 - DNA, 341 bp, Artificial sequence
  Single strand oligonucleotide
cgugggagauaaaauuauuuuugauacacuagagagcaucuacaguuaaaauaaagauuuugaguagcaccccacagguuucaguacuuuuggcuaaauaaaaguaccagguuuucuuuccuaaagaauaauuggugggggacuaagaucucgcgcaauuaugaagaggucugugggaucagcucccucgaagccaaucacgcuuaagggcccaacuagaucgucucggcccccuaaaacgaaggguuacgguuuacuugcuugagcguuucagggggugaugcguuaccaacggagacguaugggucccgcagugugggauggugguuuuauuacccaag

SEQ ID NO: 126 - DNA, 341 bp, Artificial sequence
  Single strand oligonucleotide
gcugggagggguuaguggaguuacacggaugggaaccacccuaccuugauauaaacauauuaaccauagacagagagggagaaggucucuggucaugcucagagacccaaggggucuauucuauagacgaauugcuuuguagguguuggcucgcgaaacuaaaaagaguugagucgggaaaucgccagauugaccaaucucacacauugggguaacgggaccauccucgcccacaaaaaggaagggcggugguccuauuagguguguggcgacuggcgaggguucgcagcuacgcaguggaucguucccgacauucgugggguucacuaauccuacccaca

SEQ ID NO: 127 - DNA, 193 bp, Artificial sequence
  Single strand oligonucleotide
ggguucuuccagaagggcggacaaccaacggcgaccgcccccuagggaccccaggcggacguuaaguuaggauuucccauuuacauucggaugggaugugggcgagccgccgucacgaaaacggcggcagcgccaagagcgcuggacguucgcagaagacagaaccugguugcucgcucuucuggaagaaccu

SEQ ID NO: 128 - DNA, 193 bp, Artificial sequence
  Single strand oligonucleotide
ggguuuuuucagaaggguggacauccaucgcccaucuccgcuugugccccccaggagaaggguacgccaggauuucggauagagugaccuauucgaggaguuuccgccgcugccucgaaagcagcggcugcuccaacugagcagaagaagcucuuaaaacagaaccuggaugcucgcucuucuggaagaaccu

SEQ ID NO: 129 - DNA, 193 bp, Artificial sequence
  Single strand oligonucleotide
ggguucuuucaggagggugaacaucccacgccgaccucucauuauugcccccaggaggaugguacaacuggucgucuauuugaagugcuaaguggaggugccccggcugcugacccgaaaucagcagcagcuccaaaagagcugggggggcgcugaauccagaaccgggaugcucgcucuucuggaagaaccu

SEQ ID NO: 130 - DNA, 193 bp, Artificial sequence
  Single strand oligonucleotide
gcggugguauugcuuuuucaucagccugcgcccaucacaccagggggcagacaugugaagggcaauacaggacuacuagcuuaaagacgggcugguuggguagcagcugcaggcgcgaaaucugcagccgccccaaaagggcgggggcugcccacaaggcagaacaaggcuguuggagggguaaugccauugc

SEQ ID NO: 131 - DNA, 216 bp, Artificial sequence
  Single strand oligonucleotide
gggaaucagacauggcgagauuucaucgggaucuggggcgagggcgagggcgugacaguggggagcgcagucgauacaugcaccaggcacacccaguaucgccuuggaaagcaaggcgcacuggguccgccggaugcaugugacgagugcaacgcgcccgcugcaagcaucgcgacucguuccagauuccgaugauucuccgucgcacugaugccc

SEQ ID NO: 132 - DNA, 89 bp, Artificial sequence
  Single strand oligonucleotide
caugcuaucggugcuucguacgguauuugcagagagcacaucgaacaccgauggccuccguggaugucguauguggugccguuaguaug

SEQ ID NO: 133 - DNA, 142 bp, Artificial sequence
  Single strand oligonucleotide
gcggccugaaacaccguuugauuggugugcuggggucaacguguccaaugccagaagacgucagcaagggaagaacagguguuccugggcgaugaacgcguuggugcuucuacaucaaccgaagguaaacuuucacgcaacg

SEQ ID NO: 134 - DNA, 186 bp, Artificial sequence
  Single strand oligonucleotide
guggcgugaccugagcaaguauucgugggguucacuaauccugaccgacccuugcgcaggccaggcguccaugauugguaagucaccccacaaagugcaagaccagaauggacagccagguugccuuaaccagcagagggucggcgagcguuggugaggaccgccgaugcaugaccaccacgccac

SEQ ID NO: 135 - DNA, 216 bp, Artificial sequence
  Single strand oligonucleotide
uggauacacgcgugggaagaucuggucuucuugaccggucuugguuaggucaugacggggguccgcgcaguccacucaggcgcucggcacccccgcuaccuucacggaaagugugaagcggcggggcagccagucgccugagaggagugcaacgcagcccccgcaagaauaacagaggacuggucaagaagacuauucuguuucggaguguagcca

SEQ ID NO: 136 - DNA, 83 bp, Artificial sequence
  Single strand oligonucleotide
uacguauauuguguaguuaauuuacucaggugugugugggguuacggugcaccuccaauagugaagacuaucagcaucacgua

SEQ ID NO: 137 - DNA, 140 bp, Artificial sequence
  Single strand oligonucleotide
cccggaguuugugggcaaguccgcucguacgacuucaaggaacagccuccgaaaacaggaguacaugugagauagaauaauuccugggccggcucccuguugucuuguugugcgaacaagacaugccgggagcucccggg

SEQ ID NO: 138 - DNA, 186 bp, Artificial sequence
  Single strand oligonucleotide
aaggugggaguggagagagaauucgugggguucacuaauccucacuagcucuggcccuagaggugacacccggauauggaaagcuccacacggugagacagccguaacgggugcucaacuugggcagagccagccgggagcuagccagaguugguggaagccgccaguucacuagcugcccaccuu

SEQ ID NO: 139 - DNA, 375 bp, Artificial sequence
  Single strand oligonucleotide
uuugcgaggcuagcaacuggauucuacuauauaaaaacacagacuuggaaucaugucacccaccaggacucuccgagaauccccguccgaaagacaugaacggguggaaaaagacucucaaucaucgacgacaagcuaacacaagguauccaguaagguacucuaaaggagguugaugugauggagcacuguagaacacgugcuaaacucacaucgacuaaagaugaguguucaaggucgucaaguauccgagccaggauacaaacgacucacacauauugguccuauacccuaaaggauacccuccgaaagggcaauucggacagcaaaagcuguguuuuccuauaugguagaugugguuguuagccacgcaaa

SEQ ID NO: 140 - DNA, 99 bp, Artificial sequence
  Single strand oligonucleotide
ucagcguauguaguaggcucugcuucaucaaguggucuuguguucaaauucagcuccaagcacauggucaacuggauucuacuauauaugugaauauaa

SEQ ID NO: 141 - DNA, 375 bp, Artificial sequence
  Single strand oligonucleotide
cuugcgaggucagcguguccauccaacuuauguaaugcucccaugcaauguuuguccaccccagaggccuuauuuuaaagcugaugcuaccagggcaaaaaauggugaaaaacccaucuagacaauuccgauauccaacuucaaggcuuccagguaguaucacgaaacgugaaacacgugaaggaucuuugcagagcaugggauaaaaucacguguuuuggucuggaguuuccaaugacaucaagucgcagagccaugcgacaaauguuacagauaaauugcagugaauacgacaaggaagcccuccugacgguuaaucagggcggcccguaggggguauuccauucgggcucuuaugcgcguugaccacgcaau

SEQ ID NO: 142 - DNA, 375 bp, Artificial sequence
  Single strand oligonucleotide
aaagagagggauucgugggguucacuaauccguuagccucacaccccuuauucccucaccucucaugccuuagaaugaagcaccagucacuagagggaaaaaaggcgaaaaacccuuccaaacaauagugagcaccaaacccaagguaagcagcugguagcuugaagcaaguuauacggggcggaaaacagaagaucucguuuuaaacccccguauaagaaccaagagcgcucacuggccccaaguuucugagccaagaaacaagggucacagcuguguuguugcuacuacaagaaguuuacccaccagaaggccaaucugguuagcacgggguggggcuaccacggguuaguaagucugcggaucccacucuuc

SEQ ID NO: 143 - DNA, 375 bp, Artificial sequence
  Single strand oligonucleotide
auugugaggccaaacagaagauuaagggguugucuaccgcucaccuauuacugucacaccuagcaugcccagaaccugugcacccuccacaagugauagcaauggcgaaaaaaccauccaaccaacagugcuccagaaaaccaaggcuuccaggacggaucucuaagggagacaauagggugggauauaugaagaucauuguauaaagguccuguugugccaguagguuccacacccucuccaauaggcugagccaagcuuaaagagaggccgacggaacguauacaauucauuaaggaagcccacuaguagcgcaagcuagucaccagagggagcgguagccacaauuccuuauguuuuguuuggucacacaaa

SEQ ID NO: 144 - DNA, 125 bp, Artificial sequence
  Single strand oligonucleotide
cacugugcggucucuaauacgacuguucagagugaugaaccgguuuccgcgcggaacggaggagcgggcgccggcgccgaauuggaucguuccucugagcagcuguaucggaggccgcggugaac

SEQ ID NO: 145 - DNA, 375 bp, Artificial sequence
  Single strand oligonucleotide
uuugagaggccaggaaggauauuacgaugaugaaucccacauacuugauuguuacucaccuugcaagcccaccgugugagcucccaccauuagaguaacuguaggggaaaaaaccuagacuucaacugaccuucacaaacacaagguuuccagucgguaucacuaacggugauaaaaguuucgguaccuucuagaagauggguaaaaaaaacuuuuauugauuuagagcaaacacuuuaugcaauggucagagccaugaccaaauauggacagacuuguuguaacaaauacggaaaggaaacccaccacaagggcaaugugguaagcaaaagaugugggauccucauugucguggcuccuucuuggucacucaac

SEQ ID NO: 146 - DNA, 375 bp, Artificial sequence
  Single strand oligonucleotide
gaugagagguuuggagggguaaugccauugcguugcacacauacuuccacuuugcccaccccucauggcgccgacggcaccaccagcaaauagggcaaacagagaccaaaaauucuuauacacaaacacucgcggcaaauacaagguaaccagugagggcgaccaaagguuugucuagcgaggguacucggcagagcuaggguaaaaguugcuggacacguaacugacaucgaaagaucugcaagugucugagccaagacauaauagauccggaggauguggguccagcucccaaagguuacccaccaggaggacaacuuggucaucauaagaugugugcgccaugugguggcuucucuuuccaaaccacucaua

SEQ ID NO: 147 - DNA, 375 bp, Artificial sequence
  Single strand oligonucleotide
aacgagagguaugauaaaacaugcuuaugaaugaaaucacucacugcgcccauucccaacccggaugccuuaugaugaagcacgcgauucgagggaaugaauuagggauaaagcuaacuacgcaaacuaauaccacaaagucaagguugccagaggggaacacgaaccgugauaagagaggaggcucgccguagaacgcgugggaaaacuucucuuaugagacuugugagaacaauuaccacaagaucccgagccagggaucaauggugaccgagucuuaggagcaauuccacuaagguaacccacccgaagggcaauuggguaaucaacaggagugguuugccauuuguaagaucuuuugucguaucacucguc

SEQ ID NO: 148 - DNA, 111 bp, Artificial sequence
  Single strand oligonucleotide
cauguuuggauacuaguuaauauuaauguuuaaagcuacucuacaaaaaauauaugauauauuuccgguagaguagcuuuaaauauugauauuggcuaguauccaaacaga

SEQ ID NO: 149 - DNA, 375 bp, Artificial sequence
  Single strand oligonucleotide
uuugggaggucuaguuaauauuaauguuuaauuuaaucucagacuauuauuugucacaccacuaaugccugaggcucaagcaccagaaauaagugacaacauugguguaaaauccagccucccaagucaaaucgaacaauucaaggcugccagauagucucacuaagggugguuaaagcgaggguggcguguagaacaccgucaaaaaucgcuuuagcgcgucgagauuucgcaauaucuucaagucucugagccaagagauaaaagauacccaagaaaugucguuaagaccauaaggcagcccaccugaagggcaaucagguuaucauuagcugggguugccaguugugcuccacguugaguggaucacccaac

SEQ ID NO: 150 - DNA, 375 bp, Artificial sequence
  Single strand oligonucleotide
gacgugagguuuggagggguaaugccauugcguaaacccccgacucagaauucucccaccgcacagcgcaagcuccuuacguccugacaagagggagaacauuggggaaaaagccagccacacaaguaacuaaagcaaaaugaagguguccagaaacuucccccaaggggguaaaacgugugggguugccgaagaucgugcgacaaagacacguuuuaggguuucgagcgcgcaauuacuccaagugacugagccaaguuauaagagugaccgaagcguuggaaugaggagcuuaggggcacccgccuggagggcaaccgggcaagcaggagcggggguuuccacgcgguggcuucucccucugaaucacacgug

SEQ ID NO: 151 - DNA, 375 bp, Artificial sequence
  Single strand oligonucleotide
guagcgaggucgaaucuuguuuauaacuuaaguuugucgcuaaccuggcgcagucucaccucaccagccauagacuauagcuccugucauaagagauugaaaugguuaaaaacccauacauacaaaucugauacccaaacucaaggauuccaggaaguauggccaauggucaauucagucaugggucacagcagagcucguggcaaacugacuggauuacacuuagguuucccagucacgucaacuguccgagccaggacagaaacgugaggcacgaagcguaacggauacaucaaggaaucccuccugaaggacaauuagggcaacaaagguagcggcagccacuuggguugaaccgagguucgaucacgcuag

SEQ ID NO: 152 - DNA, 102 bp, Artificial sequence
  Single strand oligonucleotide
gugaagccacuggauggaucgguucaauccucucuuccggaaucguuguugaacauaagaaccuagaaucgaggauuaaacuuauuuauuuagcgcucacuc

SEQ ID NO: 153 - DNA, 375 bp, Artificial sequence
  Single strand oligonucleotide
guugugagggcgaaucuuguuuauaacuuaacuaaaucacccacucaagucugcgucaccacucauauuuuaggcuaagguaccaggccauagacguaguaauggagaaaaaaccaucgaaucaaaacuacccuacaaaaccaagguuuccgaugaguaucacuacgagugaaaauagcuggggaguuuagaagaucuggggcuaaaacggcuguuuugcccuuugaguauacauugucugcaagagucugagccaagacucaacagauaccgagauacuggaaugaauacccaaaggaaacccucccuaagggcaauaggggcaccacgaggggugguuuccaguuggguugggugaagauucgcucacgcaaa

SEQ ID NO: 154 - DNA, 375 bp, Artificial sequence
  Single strand oligonucleotide
gaugugaguaauucgugggguucacuaauccgguuaccacagacagccuaaugacacaccacacaugccaagccgcuuagcaccugccacaaguguuauaaacgccgaaaaaugcgucaacacaaccauuugaaccaaagacaagguacccagcaaguaucuccaaaggaggaauaagugaggguguccgagagacucggggcaaaaauuacuuguucagcguugguguucgcauucucaccaagcuccugagccaaggagcaagugagacucaggaacaguaaaaaauaccugaaggguacccuccacgaggacaacgugggcaugaccugcugugguagcuccggguugguaagucugcggauuacacgcaua

SEQ ID NO: 155 - DNA, 367 bp, Artificial sequence
  Single strand oligonucleotide
aguaccgagggaaacgagaugcugcucauauaauggcggauagccccaacuucacaacuaucgggccuuccggugcacgagcggagguucuuagagcuagcaagucccucgguaagauuccacagccugugggacagcuacucacagggcccuaccggacagcuggaaguagacuugguaugccugacguaacagaccaguuacucagacagccaaauccauaucguacaaaugauaggaaagagggaucuuaccgagggaaccaauuaacucuaagaacccucacuaagugaccgggagagcugguaguuauggauugagggcuaaaagcuauuguauggguagcauucuguuucccucgauacug

SEQ ID NO: 156 - DNA, 87 bp, Artificial sequence
  Single strand oligonucleotide
cacgucagcacgacaggaugccaaugcaaaaaaacguguccuugagggcgcguuuuuuugcauuggcauccugucacgcugacgugg

SEQ ID NO: 157 - DNA, 168 bp, Artificial sequence
  Single strand oligonucleotide
ggaggacaacaugccaaugcaaaaaaaguuuugguagaaggagacgguacgcagagcagaagaggaacgguggacuuaacugagaccaucuucuccuagauaagaucucacaaaccccucuccaugcagaucuacuaaggaucugcugcguugguguguuguccuccc

SEQ ID NO: 158 - DNA, 372 bp, Artificial sequence
  Single strand oligonucleotide
guggacggucauucgugggguucacuaauccaaaagaagaccgcagauccaaaggacaaguuaagggccauguugccccuagacacagaggauggcccggcggugucacuggguuaggggaggaccucugggcgaaggaaaucagagcacacggccuggcucuaucuugaacccgugcauaguaaacggcagauguggguaagaacaccacauuaugcacggguuggagacggacccaggccaaaauucggaacauggcuccccuaaccuggugacaccgccaggccauaggggcaaaacaugacccuuaauucaucuauuggguccgcgagcuccuuacggauuagugaacuuugcgguugaccgugcacc

SEQ ID NO: 159 - DNA, 367 bp, Artificial sequence
  Single strand oligonucleotide
cguaccacgguggcagggagaagagaacgauaauugcaaauugccccugcgucucgcauuacgggcuaaacuguuccggcuaguagggacaaugagcuagcaagucuaucugugguuagaaacacccuguacuacaggcaaguacgggaccagacauggcagcgugacucagacggggcacgccaguaguuucagcccagagacacugacggccccaacgacauaaaacaauuuaugcguaauauucuaacuacagauagaaccaacuaacucauuguucccacgagaacggauaguuugagccguggugcaagaccagagggcaaaaggcaauugucguucucuuuuuguugccgccgugauacga

SEQ ID NO: 160 - DNA, 101 bp, Artificial sequence
  Single strand oligonucleotide
guugcaaacagaagauuaagggguuagaugauggcgugcaaucaggagucuugaagcaaugcaucccacuccuuuggucucuugaugcuucuguuuucacc

SEQ ID NO: 161 - DNA, 214 bp, Artificial sequence
  Single strand oligonucleotide
ggcugucggccucgcuagguauguuuaacaauguuaugccaagcggugggccaaaaacucgaaaaacaaccccuuugaggaguaggcgcugcagucaaacccuguacuccccgacgggaucuccgaugagaucggagacaaaacacgggucuaaaaccgagcauagacaccagggcacaauauuguuaaguguccuugguggcaccagccgccc

SEQ ID NO: 162 - DNA, 367 bp, Artificial sequence
  Single strand oligonucleotide
ugggccaagguauucgugggguucacuaauccucggcacaacgccccuucuccgcugaaaaccggcguaacauuaccuguacgcaugcccauagagcgagccagccgcacugucucuacgaacagccaguuuuacagcuaaaaacugggccccauccggcagcggaaggaauaccaggcaugccgcuaggaacagucuaguuccagcgacagccugaacacguucauacaagugaauuguaauaucguagagacagugcggaccaacucccucuaugggcgcgccuaaaaggaguguuacagcgguuuucgauggaaagagggcguaaagcugaggguuggugaguccuuuggauaccuugacucau

SEQ ID NO: 163 - DNA, 367 bp, Artificial sequence
  Single strand oligonucleotide
gguaccauggugcacagcaguauuuguguauaugugccgaacgcccccucaucucguggcaggggcaaaucauucagaggucguauggucucugugccagccagccuuucagccguccuaaauaaccagguugacagucacaaucugggcaccacucgucagcgagaggaacacgggguaugccaauguugacaggaaagucagauugccggcccuaacaacuucuuacaaaagaaguguaagauuaggacggcugaaaggaccaauugacgcggggaccacacaauaaucuaaugauuuagcccugccacaagguaggagggcguaaugcacauguacacgaauacuggugugcaccaugauacca

SEQ ID NO: 164 - DNA, 101 bp, Artificial sequence
  Single strand oligonucleotide
gcuguuggguggaguuccagaguaaagaugagggagugcaauuaggagucuugaagcaaugcauccccguccuuuuugcucuggaaucuucauucaucacc

SEQ ID NO: 165 - DNA, 148 bp, Artificial sequence
  Single strand oligonucleotide
agaggagccccuggucgaucaugguacgcaaugaacgucgucauguaucgaccuaaggacaaucggcagugauuaacuuucuuaaacagacccgagcaugacacauggcgacccucauagugugcuuggguccguuacggacuccgac

SEQ ID NO: 166 - DNA, 372 bp, Artificial sequence
  Single strand oligonucleotide
ggggucggccauucgugggguucacuaauccaacgugugaccggcggggcggagcucacauauagugccugguagccucaagagucggagguuugcccuacugucggucaguguuugggggggaccuccuuacgaaggaaaaaggagcaagcggccaggcuguauaaagaacccuugggauuaacauggcacuagcggguaagaacaccgcuaauuucaaggguuguuuacauaccuuggccaaaagaccaaacacauccccccaaacguugacuggcggugaggcaguugaggcuaaaccagacgcuauaugcaagcacuguccccucgagcagacgacggguugguggguccugugauuggccgagcccc

SEQ ID NO: 167 - DNA, 206 bp, Artificial sequence
  Single strand oligonucleotide
gggugccgaagcaauccgaggcuuuuuacuugggugcuuggucggcagggaaucaaacucucgcgugaauuaugccguugucgucgcccuaucucguuccggggagcccuaaaaccugacuaaauaauuauagccuucaaugugaugaguugugaugauagccgaaccaagggccugaucaagaaguuccggacauuucggcaccc

SEQ ID NO: 168 - DNA, 104 bp, Artificial sequence
  Single strand oligonucleotide
ggcgcgagcuaccacaagauguacggcaaacggccgggcgugacggcaccggcggucgugccgucgcggccgcuugcuguaugaucuuugugguagccggugcc

SEQ ID NO: 169 - DNA, 139 bp, Artificial sequence
  Single strand oligonucleotide
aagguccggaaccgaacggcaagagagcucggcaagggccugaucaagaacucuuggaucucaagccaaggaguggguggcugauggggguucuugguucuguccuuaucgagcgggccaaguucacgcuaucagccuu

SEQ ID NO: 170 - DNA, 206 bp, Artificial sequence
  Single strand oligonucleotide
gggggcccauccaaucugaggauucgugggguucacuaauccccccuaaaagugacucacacguccgggcgagccuuuucgcgaugaccgaucucgagccgguguucacgcaaaaacaucccacgaaagcuugaauccaggguguagugagcucacgucuggggaggguugaugagccaugcggguccccagacagaugggccccc

SEQ ID NO: 171 - DNA, 206 bp, Artificial sequence
  Single strand oligonucleotide
gggagccccgccaagaugaggauccgaauuuauguaccuuaucgucacccgauuacgcucacgggagucgccagcuugacuauuucaccaagccagaucgagugaucgcgaaaaucgaaacgaagucacuggccagacauuccguagagcgcugaugccggaugaauagggagcaugaucucggauccccauccagcggggcuccc

SEQ ID NO: 172 - DNA, 99 bp, Artificial sequence
  Single strand oligonucleotide
ggaauggggcuggcugucacgucgacacucaucuagagcaacaaacuucugcgagagguugccuaugauggauguugauguuacagccaacuuuauucc

SEQ ID NO: 173 - DNA, 165 bp, Artificial sequence
  Single strand oligonucleotide
ugggggcggggcggguacgggaacacguaagcugugaucguugauguuacagccaacuuuaagggugcggcgggcaguacucagcggggguucuuccuccacccccggggauggucggaucgagggaacaucgcacgucgcccccgcccgcaacccccgccccua

SEQ ID NO: 174 - DNA, 206 bp, Artificial sequence
  Single strand oligonucleotide
gggagccagugcaaucugaggauucgugggguucacuaauccccucgacgaaaugcucacaccuacuuacgcuucggcgcuagaucgcccauccagguccccugaccacgcaaaaggaucagaagcgcaagugaaugacguggguggugagacguugacggaggaggguugaugagucaaacgaguccccagacacacuggcuccc

SEQ ID NO: 175 - DNA, 206 bp, Artificial sequence
  Single strand oligonucleotide
gggagccuauccaaaaggauugggauuaugcugggguuuggccuacuucgaguuaggcacacggguggcaucccguagacggguuagccgcgaacgauuguccaaucccuaaacuguagcaggcgucugggaucagccaacccgucgugcugugacgucuguagagcuaaaguuuaguuaaaucuuaacccuucagaugggcuccc

SEQ ID NO: 176 - DNA, 165 bp, Artificial sequence
  Single strand oligonucleotide
uuggggcggggcgggaucgagcauaugaaaggcgagauugaggucuggauagaguuugcacacggcgcggcggccagccaucggcgggaugccugcccccgccgcgugcaagcugcuauuccagauuuuaucucucaucacucccucccgcaccccccgccccga

SEQ ID NO: 177 - DNA, 139 bp, Artificial sequence
  Single strand oligonucleotide
aaggacucguacaggccggcuagagagcguaaacuuuucauauuguuuuacucuuggggcacauuccuuggcgugauaggaggccggggguggggcggucugaggagaugacgcgugccaaggccccucgccccuccuu

SEQ ID NO: 178 - DNA, 206 bp, Artificial sequence
  Single strand oligonucleotide
gggagccgagccaaucagagguuggagggguaaugccauugccgacgaguauccaccggcucgugugaucgcuccauagcuggucucccgaggcagugcgcgggcacgaacaaaacaggcagaagcuagagugcagucaacgugauguuggauggggaaggucgagcgaugacguugcaacuucaaccccugacaguucggcuccc

SEQ ID NO: 179 - DNA, 292 bp, Artificial sequence
  Single strand oligonucleotide
gaaccaaugcggaagauaccaaugcacggucgcauguaaaauugggcaguuggucaguuuuguuggggugaagucuugccccaguuagccgggaggaaagauauuacacccgacucauucugacgaacgccucagguaguaugcaaccugauacugaggugaacggcagaaugaugcggguguauauauccaccuccgcuaacugggcgaagacuucacuccaacauaacggacccgcugucaccggcccauacccgacguauugggcucuuugguaacaguggucggguuc

SEQ ID NO: 180 - DNA, 84 bp, Artificial sequence
  Single strand oligonucleotide
auaccgagauaagcagaggaagaauaauuaggugcuaauuggaagcugcaccuacauuccuuuuuaucuguuuaguuuugguag

SEQ ID NO: 181 - DNA, 199 bp, Artificial sequence
  Single strand oligonucleotide
agggcguaccaggagguaugaagccucgcaugggagaucugcgagguauugggguagacuucguaaaaggcgcaaacaagcucgcacaaaagcgugaggaugauguagcuaaagaugcauaauucaacagcgauucacgcacccagggugauucguggaccucuuguugagagcuguacuuuggauaguaagacgcccu

SEQ ID NO: 182 - DNA, 292 bp, Artificial sequence
  Single strand oligonucleotide
cgccccaugaguuagaaacgaguucggggccaaaguucuaacacguagguuggaaaggguuuggugaaccuugcggacacggaggucguggucggaggagaauuaucgcccgacgcuugcccgcuaacccgugaggugccaggaaacgcgauacucacgggaaggaggguagguugcgggcgauaaauucgguccggacgaccuccgcauucgugggguucacuaaucccguuccuaccuaccccggucacugaauggcgaacuugguucuaaauuacaaggagaacgggug

SEQ ID NO: 183 - DNA, 292 bp, Artificial sequence
  Single strand oligonucleotide
gccccacuaagcuugaagccauucccgcgucucgggagaaaagcgggcgugggauauuuaguugugcugacaugucuagcaacggaugacgaagguuaagaaauaucgcccgacucguccucacaaacgccagagcacgaacgcaaccguacacucuggcgaauggggggacgaagcgggcgauaauuucacgccuuucauccguugagggacauguuagcauaauaaaaaguccagcgcccuacggugcccacaagacggaauggagucgagauuaaaaugggacgggggc

SEQ ID NO: 184 - DNA, 91 bp, Artificial sequence
  Single strand oligonucleotide
aaggcuugcuacuguggagcaaucauucugaacgauagagaaaaugggauuuaauuuaucggucagaaugauacuccacaauacuaagccu

SEQ ID NO: 185 - DNA, 195 bp, Artificial sequence
  Single strand oligonucleotide
ggaggguaccuagccggcuguaacuuguggacuaucggcgggguaauggggggcaacuagcugccgacccauuccuccaucccguccguggcuacgagagggugggcgcgacuuggaaugagggaauggagcgggagauaguuggaguccccgcccgugccuauccuuuucagguuguagccucugaugagcucu

SEQ ID NO: 186 - DNA, 292 bp, Artificial sequence
  Single strand oligonucleotide
gccccacucugacagagaccaugucgcgcaauaugaacaaacggggcugagggagguggcuugguggaccuugcgaacccauagguagacgaggguaccgaaaagacgcccgacucuggcauacaaacccgguuggauccaagaaaugauaaacgaccgggaaugggugccagaagcggguguuauuuucucgcccuucuaucugugcauucgugggguucacuaauccagcuccaucagccgacagcaucgccaauuggacauggguucuguaggacuaagugcagggggc

SEQ ID NO: 187 - DNA, 292 bp, Artificial sequence
  Single strand oligonucleotide
ggccccgaggucuugugcccaaagacaugucugagacuccagggggaaguggguaauuuaguuuaagguguaugccacucucagguaggcgaagguuaggauugcccccccgacgcaggcuuacaaacgcggauggguugacggaagaacagacauccgugaaugagagucugucacgggggggacaaucgcaccuuccuaucugagcuuggcauauauuuuaaauaaaacuaccaacuuucgaagacuucugaaagacuuuuuggcggcagguucuaaaggugagcggguc

SEQ ID NO: 188 - DNA, 84 bp, Artificial sequence
  Single strand oligonucleotide
uugggauauguuaggaaauaagaaaaucgaggugcuaauuggaagcugcaccuuagguccucuugauuccuagccguaucucau

SEQ ID NO: 189 - DNA, 199 bp, Artificial sequence
  Single strand oligonucleotide
agggcuuucacgggcuucguaggccuugcuaagagauuuuuuaaaauuaacuggaugacuuagaaaauuacgcaaacaaguagaaauaaacgcauguguggugcguugccaaagaaguguuccacaaaagauacgcaugcuccaucuuaguuugggggacuuucuuacgagagcccgaagcuagagggagagaagcccu

SEQ ID NO: 190 - DNA, 292 bp, Artificial sequence
  Single strand oligonucleotide
guccccaaccaguuguagccaauucggaugcugauggacaacacguaagaaggauguggcuuggugagcuccgcggacccguagguuuuugugggaguugaucgugaucccgacucaugcacgcaaacgcaacgggcuguacgaaaucagagaccguugcgaaugaguguaugacgcgggauugucgaucuaucccaggaaccugcgcauucgugggguucacuaauccgaguccgucuuaccucgccgcguaaaaguagaauugggggcaacggguauagacgagaggggc

SEQ ID NO: 191 - DNA, 237 bp, Artificial sequence
  Single strand oligonucleotide
cugacccguacauaucgagaguugucuggcccgccacagccccuagcaaaucucgucgcggagccacgcguaguauggucgcgagccacgcccgaagcuaaaccagaagcaccgaaggcuacgcgucccuuauacacuguaacggcaccccgaacacgggaagagggcuccgaaggccgacgagauuuccuaggggcuguggcggguuggacaacuuuggauaugugccggucaggg

SEQ ID NO: 192 - DNA, 64 bp, Artificial sequence
  Single strand oligonucleotide
cgcugcggagcucaagaagaacccucuucgaauaauccaggguucuuuuagggcuuugcgguau

SEQ ID NO: 193 - DNA, 110 bp, Artificial sequence
  Single strand oligonucleotide
aaaguuaggggagcacuaggguugauuggucgucacaguuagaucuuucugacccuagagacgaaaaagcuguggcggguuggacaacuucauaccucccaaccauagcg

SEQ ID NO: 194 - DNA, 237 bp, Artificial sequence
  Single strand oligonucleotide
cgggacaguucauugcggggguugguggaccccacgaguucccaagcaggaguaggcgcagaguagcuugacgcaagguaccggcccacggacgaccucaaacaguagagaccuaacgcgucaggcuccuauggaacccauacgaaacccccagcaggggaagaguacucuguagaccgucuacuccuccuugggaauucgugggguucacuaaucccggcagugagccgucccggg

SEQ ID NO: 195 - DNA, 237 bp, Artificial sequence
  Single strand oligonucleotide
cugaaccgaucgcaacggagugguaucauucacugccugucacuuucauauuguggcgcaggucugccuguggcaugggcgugcuccacacagaauucauaaccucuugauccaaacgcugcgggugacgcauugaaaauguuucuggcccgaacucggggaaaaggaccuggaggcugucgcaauaucaaagugacaggcggugaaugauguuauucgguugcgauccguucaggg

SEQ ID NO: 196 - DNA, 64 bp, Artificial sequence
  Single strand oligonucleotide
accggaagagguaaaugaauuaccuuuccgaauaauccaggugguuuauaugccuuuuccggau

SEQ ID NO: 197 - DNA, 110 bp, Artificial sequence
  Single strand oligonucleotide
aaggcgggggaagcaucuggacgccggaagagguaaaugaagaucuuccacauuggugggacgaaaaucguuugcuauguaucaucgucccauaacuuccaauuaggaca

SEQ ID NO: 198 - DNA, 237 bp, Artificial sequence
  Single strand oligonucleotide
cugaucagagcauugcgaggguugguggaccccgcggauacacucucugucaagggcccugagucgcuuggcggaugguucgcagcccgcgcguaggacaaacuggagucaccaaacccgccagguccauaagcgacguuuacggaaccccaagcaugggcagaggacucaggaggcgguccuugauacagaguguauucgugggguucacuaauccuggcaaugcuccggucaggg

SEQ ID NO: 199 - DNA, 237 bp, Artificial sequence
  Single strand oligonucleotide
cagaacagauccggacgguuguguugugcuuuugcuggaacacuagcuuuuguaggcccagcguuccaaggcgcaaggugacacgcucuguacgaaccuaaacccaaaggaccuaacgcgucuuggagacucuagacuagggccuuauugcaagcaugcgcggacgacgcugaagacggccuauagaaccuaguguuccagcaaaaguacagcacaacgguccggauccguucuggg

SEQ ID NO: 200 - DNA, 52 bp, Artificial sequence
  Single strand oligonucleotide
uuuggucccauguuggagcuggucgcacccagcuccacauggaagacuuacc

SEQ ID NO: 201 - DNA, 118 bp, Artificial sequence
  Single strand oligonucleotide
aaacaggaaaugggaagcggcagaaaugccauucuccguuuacguucuucgacgcuucccgcuuuccugggacgugaguagggaauaguguuuuucccacuucucaagaccgacccgc

SEQ ID NO: 202 - DNA, 237 bp, Artificial sequence
  Single strand oligonucleotide
ccgagccgaucaugucgcggauuggugagccccacgggugcaccuacgucauuugucgcugaguaacaugcugcaagugacgcgcccugcggauauuacaaacuagaguauacuaacgcggcauguucggaagcaacgcuucagaaaccccgaucacgggcagaguacucgggagcccggcaaaugaucuaggugcauucgugggguucacuaauccgggauaugguccgcucgggg

SEQ ID NO: 203 - DNA, 193 bp, Artificial sequence
  Single strand oligonucleotide
gguggugugucaaagguucgcugccucugcaucuacccucuaauugccauaugagacccuaaacuacccaagccacuggaauaaaaaugaggccgccguuccaaccaaaacgauaacauaacaaauguuauuacaagggugaaaagggcgaaggggggugggugcacgggcgacgcaccggacgcaccgccac

SEQ ID NO: 204 - DNA, 111 bp, Artificial sequence
  Single strand oligonucleotide
gccgugcacccacuagcaguuacaguguucaugaaauccuuaacuuccuucccugucgggaggauagauagggguuuuugggugcuguaccuguuguugggaucacgaaga

SEQ ID NO: 205 - DNA, 138 bp, Artificial sequence
  Single strand oligonucleotide
gaacgccgcagcguuaaaagcugccucugccucugcaucuaucuucgguuagaaggugaaggggggcgccaagaccgcgguucuaacccuagcuagguguagcccgagggagccagcuccuggcggcuuggggcccca

SEQ ID NO: 206 - DNA, 193 bp, Artificial sequence
  Single strand oligonucleotide
gcaggcgucgccaggggcuguuggagggguaaugccauugcaauggcuauaagggacugaauacuaccgagagcgcggaugccaaacccaagagacagcaucuaagacaacgaagaaccaauaagguucuuuaaaucgguaaaaagagccaagcggugguauugccauuccauuaacccaguggcgccugcac

SEQ ID NO: 207 - DNA, 351 bp, Artificial sequence
  Single strand oligonucleotide
caggggagugaagcgagugcaucuucauucaucgaagcaugcaccuucacauucggaaaaauccccacggcuggaaccguccacccaacacuaggcagagucgagcccgcgcgguaccaaaucuggguuggagaauaagucccggggguagcccuccagagggggcccaaggccacaugagggaugcgugcaagggagggacacagcauggaccggccugacuacuauugaaagccgaacguggaucagagucggccgaaggggcagaaucuacggcccgaaucuugauccaaaccccauagagucagggcgccaugggugggugaaauccacucgcuucacacccccaca

SEQ ID NO: 208 - DNA, 93 bp, Artificial sequence
  Single strand oligonucleotide
aaaaccaagcuggugcuauaaugcacaauaaggaucaaucagcaccuggaucugagauucgaguugugcguuggcgcacccacguggauccua

SEQ ID NO: 209 - DNA, 351 bp, Artificial sequence
  Single strand oligonucleotide
gcugggaggucagcguacaacucaugaauauuugaaucucccaccaucccgaaccucucugaccccaugcccgguaucgaccaccgauccacgaagacagaccaggccgcccgauucccaauuugugaucgauaaaugggcucgggguuuucccuuagcagggggacccagucccuaggauggaugggggaaugggugguaaaagccagggcuaggucuguaaucuauacaaaccccaacggggcuaguagucagcugaggggggaaaacucauagccugaauaccuagccuaacaccauaguuacagggcucccugagguguucauaugugugcguugaucacccaccca

SEQ ID NO: 210 - DNA, 351 bp, Artificial sequence
  Single strand oligonucleotide
uuugagaggcuuggagggguaaugccauugcgugaaacaucaaccggucccagcaucgaauggcgcaagucagggcccgcccaccguuccuuugcgauacuccaggccgcccgauagccaggcaaagaacgagaaauuggcacgcgucacgucccaacugggaguugccacgacgaagaccggauugguguaaggggggcagagaacaggguggugaccuuccaucaucuaaagacuaacgggguaucgacucagcugaggugguagaaaccacagccugaaucagauaccuaacgacauggggagggugaccccugacgugguggcuucucuuuccgagccacucacgca

SEQ ID NO: 211 - DNA, 351 bp, Artificial sequence
  Single strand oligonucleotide
gaugagagguauggguuuugagacaaaauuugagaaccgaaccccaucccaccgauaaagggaccgaagucggcuacauagcaccgucucuacagaauaguccaggccgcccguagcccagcuguaagacgagaacaugaugccgguccgcccccauuuggggagaucgaaucucuaggauggagguucggacgggcgacagagauggcggugaggacgggccaccaguaaaaauccaacggggcguuaaguuagcguagugggcagaaugcaacgccuaaguucaaugccuaacaccuugggguuugugcuccgccucaaguuuugcugggagcccguaccacucacgca

SEQ ID NO: 212 - DNA, 91 bp, Artificial sequence
  Single strand oligonucleotide
caguagcaguuggcgccaugaucaagaagaaaacuucccuaaacaagccaaggaaagaucuuuucuugucguggccucaccuguugauggg

SEQ ID NO: 213 - DNA, 351 bp, Artificial sequence
  Single strand oligonucleotide
aucgagagugcagauucuucuuggcgaauuagugaagcuaacaccuucucagccaccacagaccccaggccgggacccguccaccgauccaccacaagagcccaggccgcccgucgccaacguggugaucgagaauucggcgcggggucaaauuccgacgaaugguucgaagcccaaggagggauguuagcaagggcgguaaauaacauggugagggucguuugcaauuuuaacucuaacgugguuaauauuucgcugaggagguagaauccacagccgaacuacuuaaccgaacuccauugagaugacguuccaugacuaguucgggcuggggaucuguacacucgcuca

SEQ ID NO: 214 - DNA, 351 bp, Artificial sequence
  Single strand oligonucleotide
aaagagaggaauucgugggguucacuaauccuuaaaacuuccaccuacccgaacaucucugucucggcgucuggauacguccacugagccugaucgaaagaccagaccgcucgcuucccaagaucagcucaccacggaggcugcgaggcuagucaaacgugacggacccaguccacaggugggauggggguauacguguuauagagauuggaguugccugucugcgaccaaaauccaaacgcggguuuucggcagcugagggggaacaacccauagccugcagacaaacccgaacgccgucgagauagggaaccaauagggguuaguagguccgcgaauuucacucucgca

SEQ ID NO: 215 - DNA, 351 bp, Artificial sequence
  Single strand oligonucleotide
aacccgaguucagaaucucacuugagauucugugaacgaugcaccucgcuccccuauuccgaccccaggaccggacccguccaccguccacggaauaaaggccacuccgcagaacccccacuuucgggacgacaaauggucacggggucucuggucauuaccguguauguugcaauuguggggaugcguugagaauaggcaaauacccuggcgguguguguuucagaucacaaagcgaacgggguucugagugugccgagggggcauaacucauggccacagucaagaaccuaaccccauuuagauacggacccaggauagggucucggcgggguuuugaacacgggcgca

SEQ ID NO: 216 - DNA, 100 bp, Artificial sequence
  Single strand oligonucleotide
aacaguugaguggggcucugucugcgucuagaccacucgcaccaaguacagacauaaucugaaugaucuaggcgcagauuccaccccauccaacucaaca

SEQ ID NO: 217 - DNA, 351 bp, Artificial sequence
  Single strand oligonucleotide
uauggcagggcagaaucucacuugagauucugugaaacaaacaccagcucauucuguucaaaccccacgucugguaacgaccaccggaccgugaucacaguucaggccgcccgauacccaagucgcguccgaaaaguaggcccgggguuggcgcuccaaagcgggaccgaguccuaagguuggauguuuguaagggucggauacaucagggugagggcugucugcuuuaaaaaacccaacgcggguuugucagugcugagucgggacaagacacagccauuagcaaaacccgaacgcgaaagagauagcguucccugauagggucuuggcgauguaugguucagucacgca

SEQ ID NO: 218 - DNA, 351 bp, Artificial sequence
  Single strand oligonucleotide
gaugagagcuauucgugggguucacuaaucccugaaucacacaccugcccucccagucccgcccccuagucagaugacgaucccggccgcuugaucauagcccaacccgcgugcagcccacgucgacggucaaaacuuggcacgggggcuccgcccgauggcgggguucaacccgcaggcaggaugugugaauagggaggaagcaccacggcgagggcuguauucuugauaaaaccaaaccuggagugcacuuggcggaguuggaagaaagcauugcccaauugccacuccgaacgcccaagauauagugcuccgugagggguuaguaagccugcgaguagcacucacaca

SEQ ID NO: 219 - DNA, 351 bp, Artificial sequence
  Single strand oligonucleotide
ccggggacgucaccuguggcuucuaccgcaagagaacugcaauccguaucacgccggaauaaccacagguuugggagcgcccaccguccagcuguuaaaguccaggccgcccgucgcccaugcagcggacgaaaauuaagcacgugguucgcccuuacuagggggcucgaagccauaauacggaauugcggacggggggcacauaucacggaacggcccuacggcguugagaacacuaaggcgguacuugauaagcccagugggaaaaaugcagggccuuaccacgguaccgaaagcaaaugcguaggggcgccguguuuugugguaaacucacgggugaugacccuccca

SEQ ID NO: 220 - DNA, 99 bp, Artificial sequence
  Single strand oligonucleotide
guuuuuagaggugaaugcuggauggcucgucgcauucacauaagaagaagaaauauaagugaaggcugcgaaucgcucuucguuuaucucuaauauaca

SEQ ID NO: 221 - DNA, 351 bp, Artificial sequence
  Single strand oligonucleotide
cacgugagguccaagccaccauccaagccaagcgaaacaaacacaagcccauuagccccuuaccccacggcuggguccgcccacaguuccacuacgaaaggacaggcagcccggaccccaaguagugaacuagaauaagucccgggguacccgcguauacgcgugaucuaaucagcagguuugauguuuguaagggagguauacaacuuggcgguugaguuccacuguucuaacacuaucgggguccuaauucagccgauggggaaaaauuaacggccugauuucaggacccaacgucacagggaguuugacccagggcuugguuuccuuguggcuuggaucacgcgcgca

SEQ ID NO: 222 - DNA, 351 bp, Artificial sequence
  Single strand oligonucleotide
agugugaggaauucgugggguucacuaauccgggaaacugucgccuucacuuacugcccguaccccaagucaggaacaguccacagggccagugcgaaagaccaugccgccagccucccaggcauugcccuacaacguggccagggguaaagacuaucgaguugggcccagccccuaugaaggauggcagucaaggcaggaaauacacgggaggcguccgcaccaugucccaauacgaacgggguucaucauacgcugagccgguagaaggcauagccguaggacugaaccuaacaccacgugugugggggucccguucggguugguaagucugcgaauuccacacaauca

SEQ ID NO: 223 - DNA, 213 bp, Artificial sequence
  Single strand oligonucleotide
ugauuguguggcuugagguccggggucagcgucccccgcuccgacccgaacuagaagugaguagaagcuagagugaacgguaccacacagacccgcaucucggaccaacccuccgccugcaaccccuuccaccccgaccccccucucgagguccgagacagggcggugggagacgagggggcaagaacuccguacuuuauuucacguaaccaa

SEQ ID NO: 224 - DNA, 100 bp, Artificial sequence
  Single strand oligonucleotide
aggauuugccugggcuacaguauggcacucaccuagagcaacgacagcuugggaggguugccuauaagguggaugccguacuuuauuucacguaaaucuc

SEQ ID NO: 225 - DNA, 167 bp, Artificial sequence
  Single strand oligonucleotide
cggcggccagaaugcgcgcaaaaaaaaaaaaaaaaaaaaagcggcggccggacugcaccuguggacggccgccccaaagcgacggagagacggguuccuaaccaagguguaggagcagccgccggcgcuuuuuuuuaguagcuuuucucuugucagucucuccucca

SEQ ID NO: 226 - DNA, 213 bp, Artificial sequence
  Single strand oligonucleotide
ugaggauucgugggguucacuaaucccagacgccgccgcuccccccugagcagggacaucgcccagaccugaggcaacgcggcgccaccaaccacccacucguucccgcacugaaacauccaccacaacguacguagccccccccacacggagcgaguucuggcgggcggagacgagcggcggagaggguugaugagccgaguggauccccaa

SEQ ID NO: 227 - DNA, 213 bp, Artificial sequence
  Single strand oligonucleotide
cgauuuuuuaugcuuuuugguucggucagccgccgccgcgccagcccaccucguacccccagaccacacgacgcccacgcagcggcaacaaggcccagcccgagcccccgcacccucgucuuccacaucaaccgcagccccccaccccaggcucgggcccgcccggucggugacgagcggcguagaaccgaggcaaagauaauaaaaaaccga

SEQ ID NO: 228 - DNA, 76 bp, Artificial sequence
  Single strand oligonucleotide
ugguuaugacgagcgugccguacgagccacggcugcugcugcgccgccgcgggcuacggcacucuuuucauaauua

SEQ ID NO: 229 - DNA, 155 bp, Artificial sequence
  Single strand oligonucleotide
auggccgccggcuuagagagugaaaaaauauauuucugcaaaaggcccaccggccgugggcggcagaaugccgauuucugcgccugggagagaggggcccgcgcagcgauaaagcuuuuguggguguguauuuuuacaacccucucuagccuaca

SEQ ID NO: 230 - DNA, 213 bp, Artificial sequence
  Single strand oligonucleotide
cgaggauucgugggguucacuaauccccgccgccuccgcgccgcccggccgcuuacucccuucauccaagcacaugacgcgaaaugacccacuccaagcccuaccccacgaaccugcgacgacugcuacacccuccgacccccccccccggguagggcccgagaggggggugacgagaggugaacaggauugaugagccggaugaguccccga

SEQ ID NO: 231 - DNA, 213 bp, Artificial sequence
  Single strand oligonucleotide
acauugguuuuacugaguccgcggggcagagcccgccgccaugaagauccaguauaacccaucuagcuacucgaguacccugccuccccgacaccaagcucgaccccucgcuccaacguaaacaacagaucccccagccccccccaccugggucgagcccgugcuuugguggacgagcgggcgagaucucgcagauuuacaaaaacuaacgua

SEQ ID NO: 232 - DNA, 74 bp, Artificial sequence
  Single strand oligonucleotide
gugcaggauugugagggagcauuuccccagcucgaucauugcaugauuagaagaguuucuucauguuccugcau

SEQ ID NO: 233 - DNA, 213 bp, Artificial sequence
  Single strand oligonucleotide
ugagggugcucgaucacggcccugggccaacgccgccgcucccgcccccuaucgccucuccacacaccgaucagcaacacgccgcuacccacuccuaacgcgagcccacccguccacuucuucuucaaccgccgcgaccccccccccccggcucguguccgagcggucggagacgagugguggagauccaggauugugagggagcauuuccaa

SEQ ID NO: 234 - DNA, 213 bp, Artificial sequence
  Single strand oligonucleotide
agaggauucgugggguucacuaauccccgccuccgccgcuccaaccaauagcuacaggucgagaauauagcaugcuaaccgccgcaaccaacgcccaucucgugccagccccacaccaugcccuccuacagccucagacaccccaacaggguacgagaccgcgcggucggagacgagcggagcaaaggauugaugagucagauggauccccua

SEQ ID NO: 235 - DNA, 23 bp, Artificial sequence
  Single strand oligonucleotide
agaaataggcaagtcatccttgg

SEQ ID NO: 236 - DNA, 23 bp, Artificial sequence
  Single strand oligonucleotide
agaagagagtgagcacacaaagg

SEQ ID NO: 237 - DNA, 23 bp, Artificial sequence
  Single strand oligonucleotide
agaaataggcaagtcatccttgg

SEQ ID NO: 238 - DNA, 23 bp, Artificial sequence
  Single strand oligonucleotide
agaaataggcaagtcatccttgg

SEQ ID NO: 239 - DNA, 23 bp, Artificial sequence
  Single strand oligonucleotide
agaaataggcaagtcatccttgg

SEQ ID NO: 240 - DNA, 23 bp, Artificial sequence
  Single strand oligonucleotide
agaagagagtgagcacacaaagg

SEQ ID NO: 241 - DNA, 23 bp, Artificial sequence
  Single strand oligonucleotide
acagaagatagagagcactaagg

SEQ ID NO: 242 - DNA, 23 bp, Artificial sequence
  Single strand oligonucleotide
agaaataggcaagtcatccttgg

SEQ ID NO: 243 - DNA, 23 bp, Artificial sequence
  Single strand oligonucleotide
agaaataggcaagtcatccttgg

SEQ ID NO: 244 - DNA, 23 bp, Artificial sequence
  Single strand oligonucleotide
aagaatctgtaaagctcaggagg

SEQ ID NO: 245 - DNA, 23 bp, Artificial sequence
  Single strand oligonucleotide
acagaagatagagagcactaagg

SEQ ID NO: 246 - DNA, 23 bp, Artificial sequence
  Single strand oligonucleotide
agaaataggcaagtcatccttgg

SEQ ID NO: 247 - DNA, 23 bp, Artificial sequence
  Single strand oligonucleotide
cgtagatgaatggttccatcagg

SEQ ID NO: 248 - DNA, 23 bp, Artificial sequence
  Single strand oligonucleotide
aaaaatgacgctgacagaagagg

SEQ ID NO: 249 - DNA, 23 bp, Artificial sequence
  Single strand oligonucleotide
cgtagatgaatggttccatcagg

SEQ ID NO: 250 - DNA, 23 bp, Artificial sequence
  Single strand oligonucleotide
cgtagatgaatggttccatcagg

SEQ ID NO: 251 - DNA, 23 bp, Artificial sequence
  Single strand oligonucleotide
aaggtgccgcggtcatgatgggg

SEQ ID NO: 252 - DNA, 23 bp, Artificial sequence
  Single strand oligonucleotide
aatcttagggatgggaggtgtgg

SEQ ID NO: 253 - DNA, 23 bp, Artificial sequence
  Single strand oligonucleotide
aggagtgaacctgagaacagagg

SEQ ID NO: 254 - DNA, 23 bp, Artificial sequence
  Single strand oligonucleotide
aaggtgccgcggtcatgatgggg

SEQ ID NO: 255 - DNA, 23 bp, Artificial sequence
  Single strand oligonucleotide
cgtagatgaatggttccatcagg

SEQ ID NO: 256 - DNA, 23 bp, Artificial sequence
  Single strand oligonucleotide
agtggcacgtgatattggcacgg

SEQ ID NO: 257 - DNA, 23 bp, Artificial sequence
  Single strand oligonucleotide
cgtagatgaatggttccatcagg

SEQ ID NO: 258 - DNA, 23 bp, Artificial sequence
  Single strand oligonucleotide
cgtagatgaatggttccatcagg

SEQ ID NO: 259 - DNA, 23 bp, Artificial sequence
  Single strand oligonucleotide
catcatcaagattctcatcctgg

SEQ ID NO: 260 - DNA, 23 bp, Artificial sequence
  Single strand oligonucleotide
catcatcaagattctcatcctgg

SEQ ID NO: 261 - DNA, 23 bp, Artificial sequence
  Single strand oligonucleotide
catcatcaagattctcatcctgg

SEQ ID NO: 262 - DNA, 23 bp, Artificial sequence
  Single strand oligonucleotide
catcatcaagattctcatcctgg

SEQ ID NO: 263 - DNA, 23 bp, Artificial sequence
  Single strand oligonucleotide
ccgctgcttgtatttcccattgg

SEQ ID NO: 264 - DNA, 23 bp, Artificial sequence
  Single strand oligonucleotide
caaatggcatacagggagccagg

SEQ ID NO: 265 - DNA, 23 bp, Artificial sequence
  Single strand oligonucleotide
ctgaatgatgatctcggaccagg

SEQ ID NO: 266 - DNA, 23 bp, Artificial sequence
  Single strand oligonucleotide
aaggtgtgagttgagcaagatgg

SEQ ID NO: 267 - DNA, 23 bp, Artificial sequence
  Single strand oligonucleotide
ccgctgcttgtatttcccattgg

SEQ ID NO: 268 - DNA, 23 bp, Artificial sequence
  Single strand oligonucleotide
ctggcagcttcaactattggagg

SEQ ID NO: 269 - DNA, 23 bp, Artificial sequence
  Single strand oligonucleotide
ggaggcaggcaagtcatccttgg

SEQ ID NO: 270 - DNA, 23 bp, Artificial sequence
  Single strand oligonucleotide
aaggtgtgagttgagcaagatgg

SEQ ID NO: 271 - DNA, 23 bp, Artificial sequence
  Single strand oligonucleotide
tgtgatttaccagatcatgctgg

SEQ ID NO: 272 - DNA, 23 bp, Artificial sequence
  Single strand oligonucleotide
cctcaagcacatggttaaccagg

SEQ ID NO: 273 - DNA, 23 bp, Artificial sequence
  Single strand oligonucleotide
tgtgatttaccagatcatgctgg

SEQ ID NO: 274 - DNA, 23 bp, Artificial sequence
  Single strand oligonucleotide
tgtgatttaccagatcatgctgg

SEQ ID NO: 275 - DNA, 23 bp, Artificial sequence
  Single strand oligonucleotide
tgtgatttaccagatcatgctgg

SEQ ID NO: 276 - DNA, 23 bp, Artificial sequence
  Single strand oligonucleotide
cctccattccgcgcgaaaaccgg

SEQ ID NO: 277 - DNA, 23 bp, Artificial sequence
  Single strand oligonucleotide
tgtgatttaccagatcatgctgg

SEQ ID NO: 278 - DNA, 23 bp, Artificial sequence
  Single strand oligonucleotide
tgtgatttaccagatcatgctgg

SEQ ID NO: 279 - DNA, 23 bp, Artificial sequence
  Single strand oligonucleotide
tgtgatttaccagatcatgctgg

SEQ ID NO: 280 - DNA, 23 bp, Artificial sequence
  Single strand oligonucleotide
gaagctctcaaaagagcttatgg

SEQ ID NO: 281 - DNA, 23 bp, Artificial sequence
  Single strand oligonucleotide
tgtgatttaccagatcatgctgg

SEQ ID NO: 282 - DNA, 23 bp, Artificial sequence
  Single strand oligonucleotide
tgtgatttaccagatcatgctgg

SEQ ID NO: 283 - DNA, 23 bp, Artificial sequence
  Single strand oligonucleotide
tgtgatttaccagatcatgctgg

SEQ ID NO: 284 - DNA, 23 bp, Artificial sequence
  Single strand oligonucleotide
gaggtttatcgatcgattcatgg

SEQ ID NO: 285 - DNA, 23 bp, Artificial sequence
  Single strand oligonucleotide
tgtgatttaccagatcatgctgg

SEQ ID NO: 286 - DNA, 23 bp, Artificial sequence
  Single strand oligonucleotide
tgtgatttaccagatcatgctgg

SEQ ID NO: 287 - DNA, 23 bp, Artificial sequence
  Single strand oligonucleotide
agcaatccgactctcaatacagg

SEQ ID NO: 288 - DNA, 23 bp, Artificial sequence
  Single strand oligonucleotide
gcacgacttgctgacgtggaagg

SEQ ID NO: 289 - DNA, 23 bp, Artificial sequence
  Single strand oligonucleotide
ggacaactaagtgaagaaagagg

SEQ ID NO: 290 - DNA, 23 bp, Artificial sequence
  Single strand oligonucleotide
ggtctcggatcttcaaacggtgg

SEQ ID NO: 291 - DNA, 23 bp, Artificial sequence
  Single strand oligonucleotide
agcaatccgactctcaatacagg

SEQ ID NO: 292 - DNA, 23 bp, Artificial sequence
  Single strand oligonucleotide
aagatagagagcacagatgatgg

SEQ ID NO: 293 - DNA, 23 bp, Artificial sequence
  Single strand oligonucleotide
accggaccctctaacagtggagg

SEQ ID NO: 294 - DNA, 23 bp, Artificial sequence
  Single strand oligonucleotide
agcaatccgactctcaatacagg

SEQ ID NO: 295 - DNA, 23 bp, Artificial sequence
  Single strand oligonucleotide
agcaatccgactctcaatacagg

SEQ ID NO: 296 - DNA, 23 bp, Artificial sequence
  Single strand oligonucleotide
aagatagagagcacagatgatgg

SEQ ID NO: 297 - DNA, 23 bp, Artificial sequence
  Single strand oligonucleotide
caacattctagccctacttctgg

SEQ ID NO: 298 - DNA, 23 bp, Artificial sequence
  Single strand oligonucleotide
ggtctcggatcttcaaacggtgg

SEQ ID NO: 299 - DNA, 23 bp, Artificial sequence
  Single strand oligonucleotide
aggggaatgttgtctggctcggg

SEQ ID NO: 300 - DNA, 23 bp, Artificial sequence
  Single strand oligonucleotide
gacagaagagagtgagcacacgg

SEQ ID NO: 301 - DNA, 23 bp, Artificial sequence
  Single strand oligonucleotide
catggattgggctacatgagtgg

SEQ ID NO: 302 - DNA, 23 bp, Artificial sequence
  Single strand oligonucleotide
aggggaatgttgtctggctcggg

SEQ ID NO: 303 - DNA, 23 bp, Artificial sequence
  Single strand oligonucleotide
aggggaatgttgtctggctcggg

SEQ ID NO: 304 - DNA, 23 bp, Artificial sequence
  Single strand oligonucleotide
agtttgttgctctagatgagtgg

SEQ ID NO: 305 - DNA, 23 bp, Artificial sequence
  Single strand oligonucleotide
aaagaggagcgagcacgcggcgg

SEQ ID NO: 306 - DNA, 23 bp, Artificial sequence
  Single strand oligonucleotide
aggggaatgttgtctggctcggg

SEQ ID NO: 307 - DNA, 23 bp, Artificial sequence
  Single strand oligonucleotide
aggggaatgttgtctggctcggg

SEQ ID NO: 308 - DNA, 23 bp, Artificial sequence
  Single strand oligonucleotide
tgagagatgctgacagaaagagg

SEQ ID NO: 309 - DNA, 23 bp, Artificial sequence
  Single strand oligonucleotide
catggattgggctacatgagtgg

SEQ ID NO: 310 - DNA, 23 bp, Artificial sequence
  Single strand oligonucleotide
aggggaatgttgtctggctcggg

SEQ ID NO: 311 - DNA, 23 bp, Artificial sequence
  Single strand oligonucleotide
ttatctgtgcttggactgaaggg

SEQ ID NO: 312 - DNA, 23 bp, Artificial sequence
  Single strand oligonucleotide
gatagagagcacgaataatgagg

SEQ ID NO: 313 - DNA, 23 bp, Artificial sequence
  Single strand oligonucleotide
aagccttgctgaagtgtttgggg

SEQ ID NO: 314 - DNA, 23 bp, Artificial sequence
  Single strand oligonucleotide
ttatctgtgcttggactgaaggg

SEQ ID NO: 315 - DNA, 23 bp, Artificial sequence
  Single strand oligonucleotide
ttatctgtgcttggactgaaggg

SEQ ID NO: 316 - DNA, 23 bp, Artificial sequence
  Single strand oligonucleotide
ctacgcaggagagatgatgctgg

SEQ ID NO: 317 - DNA, 23 bp, Artificial sequence
  Single strand oligonucleotide
agctcccttcagtccaagcaagg

SEQ ID NO: 318 - DNA, 23 bp, Artificial sequence
  Single strand oligonucleotide
ttatctgtgcttggactgaaggg

SEQ ID NO: 319 - DNA, 23 bp, Artificial sequence
  Single strand oligonucleotide
ttatctgtgcttggactgaaggg

SEQ ID NO: 320 - DNA, 23 bp, Artificial sequence
  Single strand oligonucleotide
gatagagagcacgaataatgagg

SEQ ID NO: 321 - DNA, 23 bp, Artificial sequence
  Single strand oligonucleotide
aagccttgctgaagtgtttgggg

SEQ ID NO: 322 - DNA, 23 bp, Artificial sequence
  Single strand oligonucleotide
ttatctgtgcttggactgaaggg

SEQ ID NO: 323 - DNA, 23 bp, Artificial sequence
  Single strand oligonucleotide
ggaagggagaatatccaggatgg

SEQ ID NO: 324 - DNA, 23 bp, Artificial sequence
  Single strand oligonucleotide
acaccctggattattcgaaaagg

SEQ ID NO: 325 - DNA, 23 bp, Artificial sequence
  Single strand oligonucleotide
gatatgggcatgggcggtgtagg

SEQ ID NO: 326 - DNA, 23 bp, Artificial sequence
  Single strand oligonucleotide
ggaagggagaatatccaggatgg

SEQ ID NO: 327 - DNA, 23 bp, Artificial sequence
  Single strand oligonucleotide
ggaagggagaatatccaggatgg

SEQ ID NO: 328 - DNA, 23 bp, Artificial sequence
  Single strand oligonucleotide
acaccctggattattcgaaaagg

SEQ ID NO: 329 - DNA, 23 bp, Artificial sequence
  Single strand oligonucleotide
gatatgggcatgggcggtgtagg

SEQ ID NO: 330 - DNA, 23 bp, Artificial sequence
  Single strand oligonucleotide
ggaagggagaatatccaggatgg

SEQ ID NO: 331 - DNA, 23 bp, Artificial sequence
  Single strand oligonucleotide
ggaagggagaatatccaggatgg

SEQ ID NO: 332 - DNA, 23 bp, Artificial sequence
  Single strand oligonucleotide
cgcaccgggcttgcctagaacgg

SEQ ID NO: 333 - DNA, 23 bp, Artificial sequence
  Single strand oligonucleotide
gagagacggaattgagaagaggg

SEQ ID NO: 334 - DNA, 23 bp, Artificial sequence
  Single strand oligonucleotide
ggaagggagaatatccaggatgg

SEQ ID NO: 335 - DNA, 23 bp, Artificial sequence
  Single strand oligonucleotide
gaggctatgtgctgcagccaagg

SEQ ID NO: 336 - DNA, 23 bp, Artificial sequence
  Single strand oligonucleotide
gaaggaagtttagatcatgctgg

SEQ ID NO: 337 - DNA, 23 bp, Artificial sequence
  Single strand oligonucleotide
ctgccagcatgatctatctttgg

SEQ ID NO: 338 - DNA, 23 bp, Artificial sequence
  Single strand oligonucleotide
gaggctatgtgctgcagccaagg

SEQ ID NO: 339 - DNA, 23 bp, Artificial sequence
  Single strand oligonucleotide
ttgaagctgccagcatgatctgg

SEQ ID NO: 340 - DNA, 23 bp, Artificial sequence
  Single strand oligonucleotide
taaaccatgctggagaagcaggg

SEQ ID NO: 341 - DNA, 23 bp, Artificial sequence
  Single strand oligonucleotide
ttgaagctgccagcatgatctgg

SEQ ID NO: 342 - DNA, 23 bp, Artificial sequence
  Single strand oligonucleotide
ttgaagctgccagcatgatctgg

SEQ ID NO: 343 - DNA, 23 bp, Artificial sequence
  Single strand oligonucleotide
ttgaagctgccagcatgatctgg

SEQ ID NO: 344 - DNA, 23 bp, Artificial sequence
  Single strand oligonucleotide
tagggaagttgagatcatgctgg

SEQ ID NO: 345 - DNA, 23 bp, Artificial sequence
  Single strand oligonucleotide
ttgaagctgccagcatgatctgg

SEQ ID NO: 346 - DNA, 23 bp, Artificial sequence
  Single strand oligonucleotide
ttgaagctgccagcatgatctgg

SEQ ID NO: 347 - DNA, 23 bp, Artificial sequence
  Single strand oligonucleotide
ttgaagctgccagcatgatctgg

SEQ ID NO: 348 - DNA, 23 bp, Artificial sequence
  Single strand oligonucleotide
aatctgaatgatctcggaccagg

SEQ ID NO: 349 - DNA, 23 bp, Artificial sequence
  Single strand oligonucleotide
ttgaagctgccagcatgatctgg

SEQ ID NO: 350 - DNA, 23 bp, Artificial sequence
  Single strand oligonucleotide
ttgaagctgccagcatgatctgg

SEQ ID NO: 351 - DNA, 23 bp, Artificial sequence
  Single strand oligonucleotide
ttgaagctgccagcatgatctgg

SEQ ID NO: 352 - DNA, 23 bp, Artificial sequence
  Single strand oligonucleotide
ataagtgaaggtgtcggaccagg

SEQ ID NO: 353 - DNA, 23 bp, Artificial sequence
  Single strand oligonucleotide
ttgaagctgccagcatgatctgg

SEQ ID NO: 354 - DNA, 23 bp, Artificial sequence
  Single strand oligonucleotide
ttgaagctgccagcatgatctgg

SEQ ID NO: 355 - DNA, 23 bp, Artificial sequence
  Single strand oligonucleotide
aggggaatgttgtctggctcggg

SEQ ID NO: 356 - DNA, 23 bp, Artificial sequence
  Single strand oligonucleotide
agggttgcctataagatggatgg

SEQ ID NO: 357 - DNA, 23 bp, Artificial sequence
  Single strand oligonucleotide
agaagagagtgagcacgcatcgg

SEQ ID NO: 358 - DNA, 23 bp, Artificial sequence
  Single strand oligonucleotide
aggggaatgttgtctggctcggg

SEQ ID NO: 359 - DNA, 23 bp, Artificial sequence
  Single strand oligonucleotide
aggggaatgttgtctggctcggg

SEQ ID NO: 360 - DNA, 23 bp, Artificial sequence
  Single strand oligonucleotide
cagccgtggctcgttcggaccgg

SEQ ID NO: 361 - DNA, 23 bp, Artificial sequence
  Single strand oligonucleotide
agaaggttgtgatattggcacgg

SEQ ID NO: 362 - DNA, 23 bp, Artificial sequence
  Single strand oligonucleotide
aggggaatgttgtctggctcggg

SEQ ID NO: 363 - DNA, 23 bp, Artificial sequence
  Single strand oligonucleotide
aggggaatgttgtctggctcggg

SEQ ID NO: 364 - DNA, 23 bp, Artificial sequence
  Single strand oligonucleotide
gctggggatgtgaatcttgatgg

SEQ ID NO: 365 - DNA, 23 bp, Artificial sequence
  Single strand oligonucleotide
aggggaatgttgtctggctcggg

SEQ ID NO: 366 - DNA, 23 bp, Artificial sequence
  Single strand oligonucleotide
aggggaatgttgtctggctcggg

SEQ ID NO: 367 - DNA, 22 bp, Artificial sequence
  Single strand oligonucleotide
gttgagagtgttggagaaggag

SEQ ID NO: 368 - DNA, 21 bp, Artificial sequence
  Single strand oligonucleotide
ctcggtgttgatcctgagaag

SEQ ID NO: 369 - DNA, 20 bp, Artificial sequence
  Single strand oligonucleotide
gtactgctggtcctttgcag

SEQ ID NO: 370 - DNA, 20 bp, Artificial sequence
  Single strand oligonucleotide
aggagcactacggaaggatg

SEQ ID NO: 371 - DNA, 19 bp, Artificial sequence
  Single strand oligonucleotide
acaccctgggaattggttt

SEQ ID NO: 372 - DNA, 20 bp, Artificial sequence
  Single strand oligonucleotide
gtatgcgccaataagaccac

SEQ ID NO: 373 - DNA, 95 bp, Artificial sequence
  Single strand oligonucleotide
accagaagcgaacatctctttttagtgttgttttgttacgacaaagtagagcttttgtaggcattgggttgctttagtttcttctcctgcccttc

SEQ ID NO: 374 - DNA, 22 bp, Artificial sequence
  Single strand oligonucleotide
ttcgcttgcagagagaaatcac

SEQ ID NO: 375 - DNA, 95 bp, Artificial sequence
  Single strand oligonucleotide
aacttcttcagcacgacgaagtacaccagccccatcgccgacttcgtgacgtgcggcatccagtcccaccagtgctcccacccggtcccgtgccc

SEQ ID NO: 376 - DNA, 21 bp, Artificial sequence
  Single strand oligonucleotide
aagtcgtgctgcttcatgtgg

SEQ ID NO: 377 - DNA, 95 bp, Artificial sequence
  Single strand oligonucleotide
acaacatcaacatgaggtcgaacacggggtcctacaacggcaggaggaacttcagctacgggaagtcgagctacgccaagtggtcccacagcggg

SEQ ID NO: 378 - DNA, 21 bp, Artificial sequence
  Single strand oligonucleotide
agttgtactccagcttgtgcc

SEQ ID NO: 379 - DNA, 95 bp, Artificial sequence
  Single strand oligonucleotide
aaccttataggtgtgtttgatggacgtttcctggtcgtcatgaggaggaggaacaagaacagaattcgcgaactcttcacccttgggatttcgat

SEQ ID NO: 380 - DNA, 21 bp, Artificial sequence
  Single strand oligonucleotide
tatccacacaaactacctgca

SEQ ID NO: 381 - DNA, 95 bp, Artificial sequence
  Single strand oligonucleotide
acgtcaactgttaggtcggttaggtcgtggtcgttaatgttgaaagtttccgaatcgtcctgctcctcgtgatgccttcctacgtctatttgatc

SEQ ID NO: 382 - DNA, 21 bp, Artificial sequence
  Single strand oligonucleotide
tgacaatccagccaatccagc

SEQ ID NO: 383 - DNA, 94 bp, Artificial sequence
  Single strand oligonucleotide
gaggccatttctagccgttgtgtactagaggaccgacttctagtcagtgaggaagaggttgtgagagttgttagggaggtcgaagtaccggctt

SEQ ID NO: 384 - DNA, 21 bp, Artificial sequence
  Single strand oligonucleotide
taaagatcggcaacacatgat

SEQ ID NO: 385 - DNA, 94 bp, Artificial sequence
  Single strand oligonucleotide
tgtgaaactggaaagaacccaaatcggtgtaagtttcaacgaggattgggtcatctgtttggtgttgactgttatgtctggaacagttctcctc

SEQ ID NO: 386 - DNA, 21 bp, Artificial sequence
  Single strand oligonucleotide
tgacctttcttgggtttagcc

SEQ ID NO: 387 - DNA, 87 bp, Artificial sequence
  Single strand oligonucleotide
ctgattttcgagtctatcctattgtggcgaaatagtaactttgaccttacggcttctttttgagttacagagtcgtgtcgcctaggt

SEQ ID NO: 388 - DNA, 21 bp, Artificial sequence
  Single strand oligonucleotide
aagctcaggagggatagcgcc

SEQ ID NO: 389 - DNA, 87 bp, Artificial sequence
  Single strand oligonucleotide
aacttcttcagcacgacgaagtacaccagccccatcgccgacttcgtgacgtgcggcatccagtcccaccagtgctcccacccggtc

SEQ ID NO: 390 - DNA, 21 bp, Artificial sequence
  Single strand oligonucleotide
aagtcgtgctgcttcatgtgg

SEQ ID NO: 391 - DNA, 87 bp, Artificial sequence
  Single strand oligonucleotide
acaacatcaacatgaggtcgaacacggggtcctacaacggcaggaggaacttcagctacgggaagtcgagctacgccaagtggtccc

SEQ ID NO: 392 - DNA, 21 bp, Artificial sequence
  Single strand oligonucleotide
agttgtactccagcttgtgcc

SEQ ID NO: 393 - DNA, 87 bp, Artificial sequence
  Single strand oligonucleotide
aaccttataggtgtgtttgatggacgtttcctggtcgtcatgaggaggaggaacaagaacagaattcgcgaactcttcacccttggg

SEQ ID NO: 394 - DNA, 21 bp, Artificial sequence
  Single strand oligonucleotide
tatccacacaaactacctgca

SEQ ID NO: 395 - DNA, 87 bp, Artificial sequence
  Single strand oligonucleotide
acgtcaactgttaggtcggttaggtcgtggtcgttaatgttgaaagtttccgaatcgtcctgctcctcgtgatgccttcctacgtct

SEQ ID NO: 396 - DNA, 21 bp, Artificial sequence
  Single strand oligonucleotide
tgacaatccagccaatccagc

SEQ ID NO: 397 - DNA, 87 bp, Artificial sequence
  Single strand oligonucleotide
gaggccatttctagccgttgtgtactagaggaccgacttctagtcagtgaggaagaggttgtgagagttgttagggaggtcgaagta

SEQ ID NO: 398 - DNA, 21 bp, Artificial sequence
  Single strand oligonucleotide
taaagatcggcaacacatgat

SEQ ID NO: 399 - DNA, 89 bp, Artificial sequence
  Single strand oligonucleotide
tgtgaaactggaaagaacccaaatcggtgtaagtttcaacgaggattgggtcatctgtttggtgttgactgttatgtctggaacagttc

SEQ ID NO: 400 - DNA, 21 bp, Artificial sequence
  Single strand oligonucleotide
tgacctttcttgggtttagcc

SEQ ID NO: 401 - DNA, 416 bp, Artificial sequence
  Single strand oligonucleotide
aaaacgtaataagttctttttgtgtgtgtctgcaggcaatatcaaaaacataaccatcatgatgtatagagactgtcgggtccattgtgaggagacattcagtttctctttaaaactccttcattgaaatagtccggtgttatccctacctgagcttagttttttttttttaattttttttctgtcctattgaattattctattctcttgtccatgttcgacccatccctttcaaagtatctcaaccttctatcgttttaaagactctctcctatctctttttggtgttgagtatgtgtgtatctctactcctagttcatttgaatcagtttttctaccttgtctatccctcctgagctaatgtttgcatcttcttgttggtcattgatgtatggttgatataaattccaaataaa

SEQ ID NO: 402 - DNA, 416 bp, Artificial sequence
  Single strand oligonucleotide
aaaacgtaataagttctttttgtgtgtgtctgcaggcaatatcaaaaacataaccatcatgatgtatagagactgtcgggtccattgtgaggagacattcagtttctctttaaaactccttcattgaaatagtccggtgttatccctacctgagcttagttttttttttttaattttttttctgtcctattgaattattctattggtcacttgaccgccatgacatccctttcaaagtatctcaaccttctatcgttttaaagactctctcctatctctttttggtgttgagtatgtgtgtatctctactcctagttcatttgaatcagtttttctaccttgtctatccctcctgagctaatgtttgcatcttcttgttggtcattgatgtatggttgatataaattccaaataaa

SEQ ID NO: 403 - DNA, 416 bp, Artificial sequence
  Single strand oligonucleotide
aaaacgtaataagttctttttgtgtgtgtctgcaggcaatatcaaaaacataaccatcatgatgtatagagactgtcgggtccattgtgaggagacattcagtttctctttaaaactccttcattgaaatagtccggtgttatccctacctgagcttagttttttttttttaattttttttctgtcctattgaattattctattttcttgaccttgtaagacccatccctttcaaagtatctcaaccttctatcgttttaaagactctctcctatctctttttggtgttgagtatgtgtgtatctctactcctagttcatttgaatcagtttttctaccttgtctatccctcctgagctaatgtttgcatcttcttgttggtcattgatgtatggttgatataaattccaaataaa

SEQ ID NO: 404 - DNA, 107 bp, Artificial sequence; identical to SEQ ID NO: 64
  Single strand oligonucleotide

SEQ ID NO: 405 - DNA, 107 bp, Artificial sequence; identical to SEQ ID NO: 65
  Single strand oligonucleotide

SEQ ID NO: 406 - DNA, 107 bp, Artificial sequence; identical to SEQ ID NO: 66
  Single strand oligonucleotide

SEQ ID NO: 407 - DNA, 107 bp, Artificial sequence; identical to SEQ ID NO: 67
  Single strand oligonucleotide

SEQ ID NO: 408 - DNA, 107 bp, Artificial sequence; identical to SEQ ID NO: 68
  Single strand oligonucleotide

SEQ ID NO: 409 - DNA, 107 bp, Artificial sequence; identical to SEQ ID NO: 69
  Single strand oligonucleotide

SEQ ID NO: 410 - DNA, 107 bp, Artificial sequence; identical to SEQ ID NO: 70
  Single strand oligonucleotide

SEQ ID NO: 411 - DNA, 102 bp, Artificial sequence; identical to SEQ ID NO: 57
  Single strand oligonucleotide

SEQ ID NO: 412 - DNA, 102 bp, Artificial sequence; identical to SEQ ID NO: 58
  Single strand oligonucleotide

SEQ ID NO: 413 - DNA, 102 bp, Artificial sequence; identical to SEQ ID NO: 59
  Single strand oligonucleotide

SEQ ID NO: 414 - DNA, 102 bp, Artificial sequence; identical to SEQ ID NO: 60
  Single strand oligonucleotide

SEQ ID NO: 415 - DNA, 102 bp, Artificial sequence; identical to SEQ ID NO: 61
  Single strand oligonucleotide

SEQ ID NO: 416 - DNA, 102 bp, Artificial sequence; identical to SEQ ID NO: 62
  Single strand oligonucleotide

SEQ ID NO: 417 - DNA, 102 bp, Artificial sequence; identical to SEQ ID NO: 63
  Single strand oligonucleotide